European Patent Application EP 4 803 622 A1, published September 9, 2026. Title: ENGINEERING AND OPTIMIZATION OF IMPROVED SYSTEMS, METHODS AND ENZYME COMPOSITIONS FOR SEQUENCE MANIPULATION. Applicant: THE BROAD INSTITUTE, INC. The sequence listing filed with the application follows.

SEQUENCE LISTING (228 sequences)

SEQ ID NO: 1 - DNA, 20 bp, Homo sapiens
  source 1..20: mol_type = genomic DNA
gagtccgagcagaagaagaa

SEQ ID NO: 2 - DNA, 20 bp, Homo sapiens
  source 1..20: mol_type = genomic DNA
gagtcctagcaggagaagaa

SEQ ID NO: 3 - DNA, 20 bp, Homo sapiens
  source 1..20: mol_type = genomic DNA
gagtctaagcagaagaagaa

SEQ ID NO: 4-57 - skipped (54 entries)

SEQ ID NO: 58 - RNA, 12 nt, synthetic construct
  misc_feature 1..12: note = source = /note="Description of Artificial Sequence: Synthetic oligonucleotide"
  source 1..12: mol_type = other RNA
gttttagagcta

SEQ ID NO: 59 - protein, 7 aa, unidentified
PKKKRKV

SEQ ID NO: 60 - protein, 16 aa, unidentified
  REGION 1..16: note = source = /note="Description of Unknown: Nucleoplasmin bipartite NLS sequence"
KRPAATKKAGQAKKKK

SEQ ID NO: 61 - protein, 9 aa, unidentified
  REGION 1..9: note = source = /note="Description of Unknown: C-myc NLS sequence"
PAAKRVKLD

SEQ ID NO: 62 - protein, 11 aa, unidentified
  REGION 1..11: note = source = /note="Description of Unknown: C-myc NLS sequence"
RQRRNELKRSP

SEQ ID NO: 63 - protein, 38 aa, Homo sapiens
NQSSNFGPMKGGNFGGRSSGPYGGGGQYFAKPRNQGGY

SEQ ID NO: 64 - protein, 42 aa, unidentified
  REGION 1..42: note = source = /note="Description of Unknown: IBB domain from importin-alpha sequence"
RMRIZFKNKGKDTAELRRRRVEVSVELRKAKKDEQILKRRNV

SEQ ID NO: 65 - protein, 8 aa, unidentified
  REGION 1..8: note = source = /note="Description of Unknown: Myoma T protein sequence"
VSRKRPRP

SEQ ID NO: 66 - protein, 8 aa, unidentified
  REGION 1..8: note = source = /note="Description of Unknown: Myoma T protein sequence"
PPKKARED

SEQ ID NO: 67 - protein, 8 aa, Homo sapiens
PQPKKKPL

SEQ ID NO: 68 - protein, 12 aa, Mus musculus
SALIKKKKKMAP

SEQ ID NO: 69 - protein, 5 aa, unidentified
DRLRR

SEQ ID NO: 70 - protein, 7 aa, unidentified
PKQKKRK

SEQ ID NO: 71 - protein, 10 aa, unidentified
RKLKKKIKKL

SEQ ID NO: 72 - protein, 10 aa, Mus musculus
REKKKFLKRR

SEQ ID NO: 73 - protein, 20 aa, Homo sapiens
KRKGDEVDGVDEVAKKKSKK

SEQ ID NO: 74 - protein, 17 aa, Homo sapiens
RKCLQAGMNLEARKTKK

SEQ ID NO: 75 - DNA, 137 bp, synthetic construct
  misc_feature 1..137: note = source = /note="Description of Artificial Sequence: Synthetic polynucleotide"
  source 1..137: mol_type = other DNA
nnnnnnnnnnnnnnnnnnnngtttttgtactctcaagatttagaaataaatcttgcagaagctacaaagataaggcttcatgccgaaatcaacaccctgtcattttatggcagggtgttttcgttatttaatttttt

SEQ ID NO: 76 - DNA, 123 bp, synthetic construct
  misc_feature 1..123: note = source = /note="Description of Artificial Sequence: Synthetic polynucleotide"
  source 1..123: mol_type = other DNA
nnnnnnnnnnnnnnnnnnnngtttttgtactctcagaaatgcagaagctacaaagataaggcttcatgccgaaatcaacaccctgtcattttatggcagggtgttttcgttatttaatttttt

SEQ ID NO: 77 - DNA, 110 bp, synthetic construct
  misc_feature 1..110: note = source = /note="Description of Artificial Sequence: Synthetic polynucleotide"
  source 1..110: mol_type = other DNA
nnnnnnnnnnnnnnnnnnnngtttttgtactctcagaaatgcagaagctacaaagataaggcttcatgccgaaatcaacaccctgtcattttatggcagggtgttttttt

SEQ ID NO: 78 - DNA, 102 bp, synthetic construct
  misc_feature 1..102: note = source = /note="Description of Artificial Sequence: Synthetic polynucleotide"
  source 1..102: mol_type = other DNA
nnnnnnnnnnnnnnnnnnnngttttagagctagaaatagcaagttaaaataaggctagtccgttatcaacttgaaaaagtggcaccgagtcggtgctttttt

SEQ ID NO: 79 - DNA, 88 bp, synthetic construct
  misc_feature 1..88: note = source = /note="Description of Artificial Sequence: Synthetic oligonucleotide"
  source 1..88: mol_type = other DNA
nnnnnnnnnnnnnnnnnnnngttttagagctagaaatagcaagttaaaataaggctagtccgttatcaacttgaaaaagtgttttttt

SEQ ID NO: 80 - DNA, 76 bp, synthetic construct
  misc_feature 1..76: note = source = /note="Description of Artificial Sequence: Synthetic oligonucleotide"
  source 1..76: mol_type = other DNA
nnnnnnnnnnnnnnnnnnnngttttagagctagaaatagcaagttaaaataaggctagtccgttatcatttttttt

SEQ ID NO: 81 - protein, 984 aa, Campylobacter jejuni
MARILAFDIGISSIGWAFSENDELKDCGVRIFTKVENPKTGESLALPRRLARSARKRLARRKARLNHLKHLIANEFKLNYEDYQSFDESLAKAYKGSLISPYELRFRALNELLSKQDFARVILHIAKRRGYDDIKNSDDKEKGAILKAIKQNEEKLANYQSVGEYLYKEYFQKFKENSKEFTNVRNKKESYERCIAQSFLKDELKLIFKKQREFGFSFSKKFEEEVLSVAFYKRALKDFSHLVGNCSFFTDEKRAPKNSPLAFMFVALTRIINLLNNLKNTEGILYTKDDLNALLNEVLKNGTLTYKQTKKLLGLSDDYEFKGEKGTYFIEFKKYKEFIKALGEHNLSQDDLNEIAKDITLIKDEIKLKKALAKYDLNQNQIDSLSKLEFKDHLNISFKALKLVTPLMLEGKKYDEACNELNLKVAINEDKKDFLPAFNETYYKDEVTNPVVLRAIKEYRKVLNALLKKYGKVHKINIELAREVGKNHSQRAKIEKEQNENYKAKKDAELECEKLGLKINSKNILKLRLFKEQKEFCAYSGEKIKISDLQDEKMLEIDHIYPYSRSFDDSYMNKVLVFTKQNQEKLNQTPFEAFGNDSAKWQKIEVLAKNLPTKKQKRILDKNYKDKEQKNFKDRNLNDTRYIARLVLNYTKDYLDFLPLSDDENTKLNDTQKGSKVHVEAKSGMLTSALRHTWGFSAKDRNNHLHHAIDAVIIAYANNSIVKAFSDFKKEQESNSAELYAKKISELDYKNKRKFFEPFSGFRQKVLDKIDEIFVSKPERKKPSGALHEETFRKEEEFYQSYGGKEGVLKALELGKIRKVNGKIVKNGDMFRVDIFKHKKTNKFYAVPIYTMDFALKVLPNKAVARSKKGEIKDWILMDENYEFCFSLYKDSLILIQTKDMQEPEFVYYNAFTSSTVSLIVSKHDNKFETLSKNQKILFKNANEKEVIAKSIGIQNLKVFEKYIVSALGEVTKAEFRQREDFKK

SEQ ID NO: 82 - DNA, 91 bp, synthetic construct
  misc_feature 1..91: note = source = /note="Description of Artificial Sequence: Synthetic oligonucleotide"
  source 1..91: mol_type = other DNA
tataatctcataagaaatttaaaaagggactaaaataaagagtttgcgggactctgcggggttacaatcccctaaaaccgcttttaaaatt

SEQ ID NO: 83 - DNA, 36 bp, synthetic construct
  misc_feature 1..36: note = source = /note="Description of Artificial Sequence: Synthetic oligonucleotide"
  source 1..36: mol_type = other DNA
gttttagtccctttttaaatttctttatggtaaaat

SEQ ID NO: 84 - RNA, 95 nt, synthetic construct
  misc_feature 1..95: note = source = /note="Description of Artificial Sequence: Synthetic oligonucleotide"
  source 1..95: mol_type = other RNA
nnnnnnnnnnnnnnnnnnnngttttagtcccgaaagggactaaaataaagagtttgcgggactctgcggggttacaatcccctaaaaccgctttt

SEQ ID NO: 85 - DNA, 3243 bp, synthetic construct
  misc_feature 1..3243: note = source = /note="Description of Artificial Sequence: Synthetic polynucleotide"
  source 1..3243: mol_type = other DNA
accggtgccaccatgtacccatacgatgttccagattacgcttcgccgaagaaaaagcgcaaggtcgaagcgtccatgaaaaggaactacattctggggctggacatcgggattacaagcgtggggtatgggattattgactatgaaacaagggacgtgatcgacgcaggcgtcagactgttcaaggaggccaacgtggaaaacaatgagggacggagaagcaagaggggagccaggcgcctgaaacgacggagaaggcacagaatccagagggtgaagaaactgctgttcgattacaacctgctgaccgaccattctgagctgagtggaattaatccttatgaagccagggtgaaaggcctgagtcagaagctgtcagaggaagagttttccgcagctctgctgcacctggctaagcgccgaggagtgcataacgtcaatgaggtggaagaggacaccggcaacgagctgtctacaaaggaacagatctcacgcaatagcaaagctctggaagagaagtatgtcgcagagctgcagctggaacggctgaagaaagatggcgaggtgagagggtcaattaataggttcaagacaagcgactacgtcaaagaagccaagcagctgctgaaagtgcagaaggcttaccaccagctggatcagagcttcatcgatacttatatcgacctgctggagactcggagaacctactatgagggaccaggagaagggagccccttcggatggaaagacatcaaggaatggtacgagatgctgatgggacattgcacctattttccagaagagctgagaagcgtcaagtacgcttataacgcagatctgtacaacgccctgaatgacctgaacaacctggtcatcaccagggatgaaaacgagaaactggaatactatgagaagttccagatcatcgaaaacgtgtttaagcagaagaaaaagcctacactgaaacagattgctaaggagatcctggtcaacgaagaggacatcaagggctaccgggtgacaagcactggaaaaccagagttcaccaatctgaaagtgtatcacgatattaaggacatcacagcacggaaagaaatcattgagaacgccgaactgctggatcagattgctaagatcctgactatctaccagagctccgaggacatccaggaagagctgactaacctgaacagcgagctgacccaggaagagatcgaacagattagtaatctgaaggggtacaccggaacacacaacctgtccctgaaagctatcaatctgattctggatgagctgtggcatacaaacgacaatcagattgcaatctttaaccggctgaagctggtcccaaaaaaggtggacctgagtcagcagaaagagatcccaaccacactggtggacgatttcattctgtcacccgtggtcaagcggagcttcatccagagcatcaaagtgatcaacgccatcatcaagaagtacggcctgcccaatgatatcattatcgagctggctagggagaagaacagcaaggacgcacagaagatgatcaatgagatgcagaaacgaaaccggcagaccaatgaacgcattgaagagattatccgaactaccgggaaagagaacgcaaagtacctgattgaaaaaatcaagctgcacgatatgcaggagggaaagtgtctgtattctctggaggccatccccctggaggacctgctgaacaatccattcaactacgaggtcgatcatattatccccagaagcgtgtccttcgacaattcctttaacaacaaggtgctggtcaagcaggaagagaactctaaaaagggcaataggactcctttccagtacctgtctagttcagattccaagatctcttacgaaacctttaaaaagcacattctgaatctggccaaaggaaagggccgcatcagcaagaccaaaaaggagtacctgctggaagagcgggacatcaacagattctccgtccagaaggattttattaaccggaatctggtggacacaagatacgctactcgcggcctgatgaatctgctgcgatcctatttccgggtgaacaatctggatgtgaaagtcaagtccatcaacggcgggttcacatcttttctgaggcgcaaatggaagtttaaaaaggagcgcaacaaagggtacaagcaccatgccgaagatgctctgattatcgcaaatgccgacttcatctttaaggagtggaaaaagctggacaaagccaagaaagtgatggagaaccagatgttcgaagagaagcaggccgaatctatgcccgaaatcgagacagaacaggagtacaaggagattttcatcactcctcaccagatcaagcatatcaaggatttcaaggactacaagtactctcaccgggtggataaaaagcccaacagagagctgatcaatgacaccctgtatagtacaagaaaagacgataaggggaataccctgattgtgaacaatctgaacggactgtacgacaaagataatgacaagctgaaaaagctgatcaacaaaagtcccgagaagctgctgatgtaccaccatgatcctcagacatatcagaaactgaagctgattatggagcagtacggcgacgagaagaacccactgtataagtactatgaagagactgggaactacctgaccaagtatagcaaaaaggataatggccccgtgatcaagaagatcaagtactatgggaacaagctgaatgcccatctggacatcacagacgattaccctaacagtcgcaacaaggtggtcaagctgtcactgaagccatacagattcgatgtctatctggacaacggcgtgtataaatttgtgactgtcaagaatctggatgtcatcaaaaaggagaactactatgaagtgaatagcaagtgctacgaagaggctaaaaagctgaaaaagattagcaaccaggcagagttcatcgcctccttttacaacaacgacctgattaagatcaatggcgaactgtatagggtcatcggggtgaacaatgatctgctgaaccgcattgaagtgaatatgattgacatcacttaccgagagtatctggaaaacatgaatgataagcgcccccctcgaattatcaaaacaattgcctctaagactcagagtatcaaaaagtactcaaccgacattctgggaaacctgtatgaggtgaagagcaaaaagcaccctcagattatcaaaaagggctaagaattc

SEQ ID NO: 86 - protein, 1115 aa, synthetic construct
  REGION 1..1115: note = source = /note="Description of Artificial Sequence: Synthetic polypeptide"
MSDLVLGLDIGIGSVGVGILNKVTGEIIHKNSRIFPAAQAENNLVRRTNRQGRRLARRKKHRRVRLNRLFEESGLITDFTKISINLNPYQLRVKGLTDELSNEELFIALKNMVKHRGISYLDDASDDGNSSVGDYAQIVKENSKQLETKTPGQIQLERYQTYGQLRGDFTVEKDGKKHRLINVFPTSAYRSEALRILQTQQEFNPQITDEFINRYLEILTGKRKYYHGPGNEKSRTDYGRYRTSGETLDNIFGILIGKCTFYPDEFRAAKASYTAQEFNLLNDLNNLTVPTETKKLSKEQKNQIINYVKNEKAMGPAKLFKYIAKLLSCDVADIKGYRIDKSGKAEIHTFEAYRKMKTLETLDIEQMDRETLDKLAYVLTLNTEREGIQEALEHEFADGSFSQKQVDELVQFRKANSSIFGKGWHNFSVKLMMELIPELYETSEEQMTILTRLGKQKTTSSSNKTKYIDEKLLTEEIYNPVVAKSVRQAIKIVNAAIKEYGDFDNIVIEMARENQTTQKGQKNSRERMKRIEEGIKELGSQILKEHPVENTQLQNEKLYLYYLQNGRDMYVDQELDINRLSDYDVDHIVPQSFLKDDSIDNKVLTRSDKNRGKSDNVPSEEVVKKMKNYWRQLLNAKLITQRKFDNLTKAERGGLSELDKAGFIKRQLVETRQITKHVAQILDSRMNTKYDENDKLIREVKVITLKSKLVSDFRKDFQFYKVREINNYHHAHDAYLNAVVGTALIKKYPKLESEFVYGDYKVYDVRKMIAKSEQEIGKATAKYFFYSNIMNFFKTEITLANGEIRKRPLIETNGETGEIVWDKGRDFATVRKVLSMPQVNIVKKTEVQTGGFSKESILPKRNSDKLIARKKDWDPKKYGGFDSPTVAYSVLVVAKVEKGKSKKLKSVKELLGITIMERSSFEKNPIDFLEAKGYKEVKKDLIIKLPKYSLFELENGRKRMLASAGELQKGNELALPSKYVNFLYLASHYEKLKGSPEDNEQKQLFVEQHKHYLDEIIEQISEFSKRVILADANLDKVLSAYNKHRDKPIREQAENIIHLFTLTNLGAPAAFKYFDTTIDRKRYTSTKEVLDATLIHQSITGLYETRIDLSQLGGD

SEQ ID NO: 87 - protein, 1374 aa, synthetic construct
  REGION 1..1374: note = source = /note="Description of Artificial Sequence: Synthetic polypeptide"
MDKKYSIGLDIGTNSVGWAVITDEYKVPSKKFKVLGNTDRHSIKKNLIGALLFDSGETAEATRLKRTARRRYTRRKNRICYLQEIFSNEMAKVDDSFFHRLEESFLVEEDKKHERHPIFGNIVDEVAYHEKYPTIYHLRKKLVDSTDKADLRLIYLALAHMIKFRGHFLIEGDLNPDNSDVDKLFIQLVQTYNQLFEENPINASGVDAKAILSARLSKSRRLENLIAQLPGEKKNGLFGNLIALSLGLTPNFKSNFDLAEDAKLQLSKDTYDDDLDNLLAQIGDQYADLFLAAKNLSDAILLSDILRVNTEITKAPLSASMIKRYDEHHQDLTLLKALVRQQLPEKYKEIFFDQSKNGYAGYIDGGASQEEFYKFIKPILEKMDGTEELLVKLNREDLLRKQRTFDNGSIPHQIHLGELHAILRRQEDFYPFLKDNREKIEKILTFRIPYYVGPLARGNSRFAWMTRKSEETITPWNFEEVVDKGASAQSFIERMTNFDKNLPNEKVLPKHSLLYEYFTVYNELTKVKYVTEGMRKPAFLSGEQKKAIVDLLFKTNRKVTVKQLKEDYFKKIECFDSVEISGVEDRFNASLGTYHDLLKIIKDKDFLDNEENEDILEDIVLTLTLFEDREMIEERLKTYAHLFDDKVMKQLKRRRYTGWGRLSRKLINGIRDKQSGKTILDFLKSDGFANRNFMQLIHDDSLTFKEDIQKAQVSGQGDSLHEHIANLAGSPAIKKGILQTVKVVDELVKVMGRHKPENIVIEMARETNEDDEKKAIQKIQKANKDEKDAAMLKAANQYNGKAELPHSVFHGHKQLATKIRLWHQQGERCLYTGKTISIHDLINNSNQFEVDHILPLSITFDDSLANKVLVYATANQEKGQRTPYQALDSMDDAWSFRELKAFVRESKTLSNKKKEYLLTEEDISKFDVRKKFIERNLVDTRYASRVVLNALQEHFRAHKIDTKVSVVRGQFTSQLRRHWGIEKTRDTYHHHAVDALIIAASSQLNLWKKQKNTLVSYSEDQLLDIETGELISDDEYKESVFKAPYQHFVDTLKSKEFEDSILFSYQVDSKFNRKISDATIYATRQAKVGKDKADETYVLGKIKDIYTQDGYDAFMKIYKKDKSKFLMYRHDPQTFEKVIEPILENYPNKQINEKGKEVPCNPFLKYKEEHGYIRKYSKKGNGPEIKSLKYYDSKLGNHIDITPKDSNNKVVLQSVSPWRADVYFNKTTGKYEILGLKYADLQFEKGTGTYKISQEKYNDIKKKEGVDSDSEFKFTLYKNDLLLVKDTETKEQQLFRFLSRTMPKQKHYVELKPYDKQKFEGGEALIKVLGNVANSGQCKKGLGKSNISIYKVRTDVLGNQHIIKNEGDKPKLDF

SEQ ID NO: 88 - DNA, 4677 bp, synthetic construct
  misc_feature 1..4677: note = source = /note="Description of Artificial Sequence: Synthetic polynucleotide"
  source 1..4677: mol_type = other DNA
tctttcttgcgctatgacacttccagcaaaaggtagggcgggctgcgagacggcttcccggcgctgcatgcaacaccgatgatgcttcgaccccccgaagctccttcggggctgcatgggcgctccgatgccgctccagggcgagcgctgtttaaatagccaggcccccgattgcaaagacattatagcgagctaccaaagccatattcaaacacctagatcactaccacttctacacaggccactcgagcttgtgatcgcactccgctaagggggcgcctcttcctcttcgtttcagtcacaacccgcaaacatgtacccatacgatgttccagattacgcttcgccgaagaaaaagcgcaaggtcgaagcgtccgacaagaagtacagcatcggcctggacatcggcaccaactctgtgggctgggccgtgatcaccgacgagtacaaggtgcccagcaagaaattcaaggtgctgggcaacaccgaccggcacagcatcaagaagaacctgatcggagccctgctgttcgacagcggcgaaacagccgaggccacccggctgaagagaaccgccagaagaagatacaccagacggaagaaccggatctgctatctgcaagagatcttcagcaacgagatggccaaggtggacgacagcttcttccacagactggaagagtccttcctggtggaagaggataagaagcacgagcggcaccccatcttcggcaacatcgtggacgaggtggcctaccacgagaagtaccccaccatctaccacctgagaaagaaactggtggacagcaccgacaaggccgacctgcggctgatctatctggccctggcccacatgatcaagttccggggccacttcctgatcgagggcgacctgaaccccgacaacagcgacgtggacaagctgttcatccagctggtgcagacctacaaccagctgttcgaggaaaaccccatcaacgccagcggcgtggacgccaaggccatcctgtctgccagactgagcaagagcagacggctggaaaatctgatcgcccagctgcccggcgagaagaagaatggcctgttcggcaacctgattgccctgagcctgggcctgacccccaacttcaagagcaacttcgacctggccgaggatgccaaactgcagctgagcaaggacacctacgacgacgacctggacaacctgctggcccagatcggcgaccagtacgccgacctgtttctggccgccaagaacctgtccgacgccatcctgctgagcgacatcctgagagtgaacaccgagatcaccaaggcccccctgagcgcctctatgatcaagagatacgacgagcaccaccaggacctgaccctgctgaaagctctcgtgcggcagcagctgcctgagaagtacaaagagattttcttcgaccagagcaagaacggctacgccggctacattgacggcggagccagccaggaagagttctacaagttcatcaagcccatcctggaaaagatggacggcaccgaggaactgctcgtgaagctgaacagagaggacctgctgcggaagcagcggaccttcgacaacggcagcatcccccaccagatccacctgggagagctgcacgccattctgcggcggcaggaagatttttacccattcctgaaggacaaccgggaaaagatcgagaagatcctgaccttccgcatcccctactacgtgggccctctggccaggggaaacagcagattcgcctggatgaccagaaagagcgaggaaaccatcaccccctggaacttcgaggaagtggtggacaagggcgcttccgcccagagcttcatcgagcggatgaccaacttcgataagaacctgcccaacgagaaggtgctgcccaagcacagcctgctgtacgagtacttcaccgtgtataacgagctgaccaaagtgaaatacgtgaccgagggaatgagaaagcccgccttcctgagcggcgagcagaaaaaggccatcgtggacctgctgttcaagaccaaccggaaagtgaccgtgaagcagctgaaagaggactacttcaagaaaatcgagtgcttcgactccgtggaaatctccggcgtggaagatcggttcaacgcctccctgggcacataccacgatctgctgaaaattatcaaggacaaggacttcctggacaatgaggaaaacgaggacattctggaagatatcgtgctgaccctgacactgtttgaggacagagagatgatcgaggaacggctgaaaacctatgcccacctgttcgacgacaaagtgatgaagcagctgaagcggcggagatacaccggctggggcaggctgagccggaagctgatcaacggcatccgggacaagcagtccggcaagacaatcctggatttcctgaagtccgacggcttcgccaacagaaacttcatgcagctgatccacgacgacagcctgacctttaaagaggacatccagaaagcccaggtgtccggccagggcgatagcctgcacgagcacattgccaatctggccggcagccccgccattaagaagggcatcctgcagacagtgaaggtggtggacgagctcgtgaaagtgatgggccggcacaagcccgagaacatcgtgatcgaaatggccagagagaaccagaccacccagaagggacagaagaacagccgcgagagaatgaagcggatcgaagagggcatcaaagagctgggcagccagatcctgaaagaacaccccgtggaaaacacccagctgcagaacgagaagctgtacctgtactacctgcagaatgggcgggatatgtacgtggaccaggaactggacatcaaccggctgtccgactacgatgtggaccatatcgtgcctcagagctttctgaaggacgactccatcgacaacaaggtgctgaccagaagcgacaagaaccggggcaagagcgacaacgtgccctccgaagaggtcgtgaagaagatgaagaactactggcggcagctgctgaacgccaagctgattacccagagaaagttcgacaatctgaccaaggccgagagaggcggcctgagcgaactggataaggccggcttcatcaagagacagctggtggaaacccggcagatcacaaagcacgtggcacagatcctggactcccggatgaacactaagtacgacgagaatgacaagctgatccgggaagtgaaagtgatcaccctgaagtccaagctggtgtccgatttccggaaggatttccagttttacaaagtgcgcgagatcaacaactaccaccacgcccacgacgcctacctgaacgccgtcgtgggaaccgccctgatcaaaaagtaccctaagctggaaagcgagttcgtgtacggcgactacaaggtgtacgacgtgcggaagatgatcgccaagagcgagcaggaaatcggcaaggctaccgccaagtacttcttctacagcaacatcatgaactttttcaagaccgagattaccctggccaacggcgagatccggaagcggcctctgatcgagacaaacggcgaaaccggggagatcgtgtgggataagggccgggattttgccaccgtgcggaaagtgctgagcatgccccaagtgaatatcgtgaaaaagaccgaggtgcagacaggcggcttcagcaaagagtctatcctgcccaagaggaacagcgataagctgatcgccagaaagaaggactgggaccctaagaagtacggcggcttcgacagccccaccgtggcctattctgtgctggtggtggccaaagtggaaaagggcaagtccaagaaactgaagagtgtgaaagagctgctggggatcaccatcatggaaagaagcagcttcgagaagaatcccatcgactttctggaagccaagggctacaaagaagtgaaaaaggacctgatcatcaagctgcctaagtactccctgttcgagctggaaaacggccggaagagaatgctggcctctgccggcgaactgcagaagggaaacgaactggccctgccctccaaatatgtgaacttcctgtacctggccagccactatgagaagctgaagggctcccccgaggataatgagcagaaacagctgtttgtggaacagcacaagcactacctggacgagatcatcgagcagatcagcgagttctccaagagagtgatcctggccgacgctaatctggacaaagtgctgtccgcctacaacaagcaccgggataagcccatcagagagcaggccgagaatatcatccacctgtttaccctgaccaatctgggagcccctgccgccttcaagtactttgacaccaccatcgaccggaagaggtacaccagcaccaaagaggtgctggacgccaccctgatccaccagagcatcaccggcctgtacgagacacggatcgacctgtctcagctgggaggcgacagccccaagaagaagagaaaggtggaggccagctaaggatccggcaagactggccccgcttggcaacgcaacagtgagcccctccctagtgtgtttggggatgtgactatgtattcgtgtgttggccaacgggtcaacccgaacagattgatacccgccttggcatttcctgtcagaatgtaacgtcagttgatggtact

SEQ ID NO: 89 - DNA, 3150 bp, synthetic construct
  misc_feature 1..3150: note = source = /note="Description of Artificial Sequence: Synthetic polynucleotide"
  source 1..3150: mol_type = other DNA
tctttcttgcgctatgacacttccagcaaaaggtagggcgggctgcgagacggcttcccggcgctgcatgcaacaccgatgatgcttcgaccccccgaagctccttcggggctgcatgggcgctccgatgccgctccagggcgagcgctgtttaaatagccaggcccccgattgcaaagacattatagcgagctaccaaagccatattcaaacacctagatcactaccacttctacacaggccactcgagcttgtgatcgcactccgctaagggggcgcctcttcctcttcgtttcagtcacaacccgcaaacatgcctaagaagaagaggaaggttaacacgattaacatcgctaagaacgacttctctgacatcgaactggctgctatcccgttcaacactctggctgaccattacggtgagcgtttagctcgcgaacagttggcccttgagcatgagtcttacgagatgggtgaagcacgcttccgcaagatgtttgagcgtcaacttaaagctggtgaggttgcggataacgctgccgccaagcctctcatcactaccctactccctaagatgattgcacgcatcaacgactggtttgaggaagtgaaagctaagcgcggcaagcgcccgacagccttccagttcctgcaagaaatcaagccggaagccgtagcgtacatcaccattaagaccactctggcttgcctaaccagtgctgacaatacaaccgttcaggctgtagcaagcgcaatcggtcgggccattgaggacgaggctcgcttcggtcgtatccgtgaccttgaagctaagcacttcaagaaaaacgttgaggaacaactcaacaagcgcgtagggcacgtctacaagaaagcatttatgcaagttgtcgaggctgacatgctctctaagggtctactcggtggcgaggcgtggtcttcgtggcataaggaagactctattcatgtaggagtacgctgcatcgagatgctcattgagtcaaccggaatggttagcttacaccgccaaaatgctggcgtagtaggtcaagactctgagactatcgaactcgcacctgaatacgctgaggctatcgcaacccgtgcaggtgcgctggctggcatctctccgatgttccaaccttgcgtagttcctcctaagccgtggactggcattactggtggtggctattgggctaacggtcgtcgtcctctggcgctggtgcgtactcacagtaagaaagcactgatgcgctacgaagacgtttacatgcctgaggtgtacaaagcgattaacattgcgcaaaacaccgcatggaaaatcaacaagaaagtcctagcggtcgccaacgtaatcaccaagtggaagcattgtccggtcgaggacatccctgcgattgagcgtgaagaactcccgatgaaaccggaagacatcgacatgaatcctgaggctctcaccgcgtggaaacgtgctgccgctgctgtgtaccgcaaggacaaggctcgcaagtctcgccgtatcagccttgagttcatgcttgagcaagccaataagtttgctaaccataaggccatctggttcccttacaacatggactggcgcggtcgtgtttacgctgtgtcaatgttcaacccgcaaggtaacgatatgaccaaaggactgcttacgctggcgaaaggtaaaccaatcggtaaggaaggttactactggctgaaaatccacggtgcaaactgtgcgggtgtcgacaaggttccgttccctgagcgcatcaagttcattgaggaaaaccacgagaacatcatggcttgcgctaagtctccactggagaacacttggtgggctgagcaagattctccgttctgcttccttgcgttctgctttgagtacgctggggtacagcaccacggcctgagctataactgctcccttccgctggcgtttgacgggtcttgctctggcatccagcacttctccgcgatgctccgagatgaggtaggtggtcgcgcggttaacttgcttcctagtgaaaccgttcaggacatctacgggattgttgctaagaaagtcaacgagattctacaagcagacgcaatcaatgggaccgataacgaagtagttaccgtgaccgatgagaacactggtgaaatctctgagaaagtcaagctgggcactaaggcactggctggtcaatggctggcttacggtgttactcgcagtgtgactaagcgttcagtcatgacgctggcttacgggtccaaagagttcggcttccgtcaacaagtgctggaagataccattcagccagctattgattccggcaagggtctgatgttcactcagccgaatcaggctgctggatacatggctaagctgatttgggaatctgtgagcgtgacggtggtagctgcggttgaagcaatgaactggcttaagtctgctgctaagctgctggctgctgaggtcaaagataagaagactggagagattcttcgcaagcgttgcgctgtgcattgggtaactcctgatggtttccctgtgtggcaggaatacaagaagcctattcagacgcgcttgaacctgatgttcctcggtcagttccgcttacagcctaccattaacaccaacaaagatagcgagattgatgcacacaaacaggagtctggtatcgctcctaactttgtacacagccaagacggtagccaccttcgtaagactgtagtgtgggcacacgagaagtacggaatcgaatcttttgcactgattcacgactccttcggtacgattccggctgacgctgcgaacctgttcaaagcagtgcgcgaaactatggttgacacatatgagtcttgtgatgtactggctgatttctacgaccagttcgctgaccagttgcacgagtctcaattggacaaaatgccagcacttccggctaaaggtaacttgaacctccgtgacatcttagagtcggacttcgcgttcgcgtaaggatccggcaagactggccccgcttggcaacgcaacagtgagcccctccctagtgtgtttggggatgtgactatgtattcgtgtgttggccaacgggtcaacccgaacagattgatacccgccttggcatttcctgtcagaatgtaacgtcagttgatggtact

SEQ ID NO: 90 - DNA, 125 bp, synthetic construct
  misc_feature 1..125: note = source = /note="Description of Artificial Sequence: Synthetic polynucleotide"
  source 1..125: mol_type = other DNA
gaaattaatacgactcactatannnnnnnnnnnnnnnnnnnngttttagagctagaaatagcaagttaaaataaggctagtccgttatcaacttgaaaaagtggcaccgagtcggtgcttttttt

SEQ ID NO: 91 - DNA, 8452 bp, synthetic construct
  misc_feature 1..8452: note = source = /note="Description of Artificial Sequence: Synthetic polynucleotide"
  source 1..8452: mol_type = other DNA
tgcggtatttcacaccgcatcaggtggcacttttcggggaaatgtgcgcggaacccctatttgtttatttttctaaatacattcaaatatgtatccgctcatgagattatcaaaaaggatcttcacctagatccttttaaattaaaaatgaagttttaaatcaatctaaagtatatatgagtaaacttggtctgacagttaccaatgcttaatcagtgaggcacctatctcagcgatctgtctatttcgttcatccatagttgcctgactccccgtcgtgtagataactacgatacgggagggcttaccatctggccccagtgctgcaatgataccgcgagacccacgctcaccggctccagatttatcagcaataaaccagccagccggaagggccgagcgcagaagtggtcctgcaactttatccgcctccatccagtctattaattgttgccgggaagctagagtaagtagttcgccagttaatagtttgcgcaacgttgttgccattgctacaggcatcgtggtgtcacgctcgtcgtttggtatggcttcattcagctccggttcccaacgatcaaggcgagttacatgatcccccatgttgtgcaaaaaagcggttagctccttcggtcctccgatcgttgtcagaagtaagttggccgcagtgttatcactcatggttatggcagcactgcataattctcttactgtcatgccatccgtaagatgcttttctgtgactggtgagtactcaaccaagtcattctgagaatagtgtatgcggcgaccgagttgctcttgcccggcgtcaatacgggataataccgcgccacatagcagaactttaaaagtgctcatcattggaaaacgttcttcggggcgaaaactctcaaggatcttaccgctgttgagatccagttcgatgtaacccactcgtgcacccaactgatcttcagcatcttttactttcaccagcgtttctgggtgagcaaaaacaggaaggcaaaatgccgcaaaaaagggaataagggcgacacggaaatgttgaatactcatactcttcctttttcaatattattgaagcatttatcagggttattgtctcatgaccaaaatcccttaacgtgagttttcgttccactgagcgtcagaccccgtagaaaagatcaaaggatcttcttgagatcctttttttctgcgcgtaatctgctgcttgcaaacaaaaaaaccaccgctaccagcggtggtttgtttgccggatcaagagctaccaactctttttccgaaggtaactggcttcagcagagcgcagataccaaatactgttcttctagtgtagccgtagttaggccaccacttcaagaactctgtagcaccgcctacatacctcgctctgctaatcctgttaccagtggctgttgccagtggcgataagtcgtgtcttaccgggttggactcaagacgatagttaccggataaggcgcagcggtcgggctgaacggggggttcgtgcacacagcccagcttggagcgaacgacctacaccgaactgagatacctacagcgtgagctatgagaaagcgccacgcttcccgaagggagaaaggcggacaggtatccggtaagcggcagggtcggaacaggagagcgcacgagggagcttccagggggaaacgcctggtatctttatagtcctgtcgggtttcgccacctctgacttgagcgtcgatttttgtgatgctcgtcaggggggcggagcctatggaaaaacgccagcaacgcggcctttttacggttcctggccttttgctggccttttgctcacatgttctttcctgcgttatcccctgattctgtggataaccgtattaccgcctttgagtgagctgataccgctcgccgcagccgaacgaccgagcgcagcgagtcagtgagcgaggaagcggtcgctgaggcttgacatgattggtgcgtatgtttgtatgaagctacaggactgatttggcgggctatgagggcgggggaagctctggaagggccgcgatggggcgcgcggcgtccagaaggcgccatacggcccgctggcggcacccatccggtataaaagcccgcgaccccgaacggtgacctccactttcagcgacaaacgagcacttatacatacgcgactattctgccgctatacataaccactcagctagcttaagatcccatcaagcttgcatgccgggcgcgccagaaggagcgcagccaaaccaggatgatgtttgatggggtatttgagcacttgcaacccttatccggaagccccctggcccacaaaggctaggcgccaatgcaagcagttcgcatgcagcccctggagcggtgccctcctgataaaccggccagggggcctatgttctttacttttttacaagagaagtcactcaacatcttaaaatggccaggtgagtcgacgagcaagcccggcggatcaggcagcgtgcttgcagatttgacttgcaacgcccgcattgtgtcgacgaaggcttttggctcctctgtcgctgtctcaagcagcatctaaccctgcgtcgccgtttccatttgcaggagattcgaggtaccatgtacccatacgatgttccagattacgcttcgccgaagaaaaagcgcaaggtcgaagcgtccgacaagaagtacagcatcggcctggacatcggcaccaactctgtgggctgggccgtgatcaccgacgagtacaaggtgcccagcaagaaattcaaggtgctgggcaacaccgaccggcacagcatcaagaagaacctgatcggagccctgctgttcgacagcggcgaaacagccgaggccacccggctgaagagaaccgccagaagaagatacaccagacggaagaaccggatctgctatctgcaagagatcttcagcaacgagatggccaaggtggacgacagcttcttccacagactggaagagtccttcctggtggaagaggataagaagcacgagcggcaccccatcttcggcaacatcgtggacgaggtggcctaccacgagaagtaccccaccatctaccacctgagaaagaaactggtggacagcaccgacaaggccgacctgcggctgatctatctggccctggcccacatgatcaagttccggggccacttcctgatcgagggcgacctgaaccccgacaacagcgacgtggacaagctgttcatccagctggtgcagacctacaaccagctgttcgaggaaaaccccatcaacgccagcggcgtggacgccaaggccatcctgtctgccagactgagcaagagcagacggctggaaaatctgatcgcccagctgcccggcgagaagaagaatggcctgttcggcaacctgattgccctgagcctgggcctgacccccaacttcaagagcaacttcgacctggccgaggatgccaaactgcagctgagcaaggacacctacgacgacgacctggacaacctgctggcccagatcggcgaccagtacgccgacctgtttctggccgccaagaacctgtccgacgccatcctgctgagcgacatcctgagagtgaacaccgagatcaccaaggcccccctgagcgcctctatgatcaagagatacgacgagcaccaccaggacctgaccctgctgaaagctctcgtgcggcagcagctgcctgagaagtacaaagagattttcttcgaccagagcaagaacggctacgccggctacattgacggcggagccagccaggaagagttctacaagttcatcaagcccatcctggaaaagatggacggcaccgaggaactgctcgtgaagctgaacagagaggacctgctgcggaagcagcggaccttcgacaacggcagcatcccccaccagatccacctgggagagctgcacgccattctgcggcggcaggaagatttttacccattcctgaaggacaaccgggaaaagatcgagaagatcctgaccttccgcatcccctactacgtgggccctctggccaggggaaacagcagattcgcctggatgaccagaaagagcgaggaaaccatcaccccctggaacttcgaggaagtggtggacaagggcgcttccgcccagagcttcatcgagcggatgaccaacttcgataagaacctgcccaacgagaaggtgctgcccaagcacagcctgctgtacgagtacttcaccgtgtataacgagctgaccaaagtgaaatacgtgaccgagggaatgagaaagcccgccttcctgagcggcgagcagaaaaaggccatcgtggacctgctgttcaagaccaaccggaaagtgaccgtgaagcagctgaaagaggactacttcaagaaaatcgagtgcttcgactccgtggaaatctccggcgtggaagatcggttcaacgcctccctgggcacataccacgatctgctgaaaattatcaaggacaaggacttcctggacaatgaggaaaacgaggacattctggaagatatcgtgctgaccctgacactgtttgaggacagagagatgatcgaggaacggctgaaaacctatgcccacctgttcgacgacaaagtgatgaagcagctgaagcggcggagatacaccggctggggcaggctgagccggaagctgatcaacggcatccgggacaagcagtccggcaagacaatcctggatttcctgaagtccgacggcttcgccaacagaaacttcatgcagctgatccacgacgacagcctgacctttaaagaggacatccagaaagcccaggtgtccggccagggcgatagcctgcacgagcacattgccaatctggccggcagccccgccattaagaagggcatcctgcagacagtgaaggtggtggacgagctcgtgaaagtgatgggccggcacaagcccgagaacatcgtgatcgaaatggccagagagaaccagaccacccagaagggacagaagaacagccgcgagagaatgaagcggatcgaagagggcatcaaagagctgggcagccagatcctgaaagaacaccccgtggaaaacacccagctgcagaacgagaagctgtacctgtactacctgcagaatgggcgggatatgtacgtggaccaggaactggacatcaaccggctgtccgactacgatgtggaccatatcgtgcctcagagctttctgaaggacgactccatcgacaacaaggtgctgaccagaagcgacaagaaccggggcaagagcgacaacgtgccctccgaagaggtcgtgaagaagatgaagaactactggcggcagctgctgaacgccaagctgattacccagagaaagttcgacaatctgaccaaggccgagagaggcggcctgagcgaactggataaggccggcttcatcaagagacagctggtggaaacccggcagatcacaaagcacgtggcacagatcctggactcccggatgaacactaagtacgacgagaatgacaagctgatccgggaagtgaaagtgatcaccctgaagtccaagctggtgtccgatttccggaaggatttccagttttacaaagtgcgcgagatcaacaactaccaccacgcccacgacgcctacctgaacgccgtcgtgggaaccgccctgatcaaaaagtaccctaagctggaaagcgagttcgtgtacggcgactacaaggtgtacgacgtgcggaagatgatcgccaagagcgagcaggaaatcggcaaggctaccgccaagtacttcttctacagcaacatcatgaactttttcaagaccgagattaccctggccaacggcgagatccggaagcggcctctgatcgagacaaacggcgaaaccggggagatcgtgtgggataagggccgggattttgccaccgtgcggaaagtgctgagcatgccccaagtgaatatcgtgaaaaagaccgaggtgcagacaggcggcttcagcaaagagtctatcctgcccaagaggaacagcgataagctgatcgccagaaagaaggactgggaccctaagaagtacggcggcttcgacagccccaccgtggcctattctgtgctggtggtggccaaagtggaaaagggcaagtccaagaaactgaagagtgtgaaagagctgctggggatcaccatcatggaaagaagcagcttcgagaagaatcccatcgactttctggaagccaagggctacaaagaagtgaaaaaggacctgatcatcaagctgcctaagtactccctgttcgagctggaaaacggccggaagagaatgctggcctctgccggcgaactgcagaagggaaacgaactggccctgccctccaaatatgtgaacttcctgtacctggccagccactatgagaagctgaagggctcccccgaggataatgagcagaaacagctgtttgtggaacagcacaagcactacctggacgagatcatcgagcagatcagcgagttctccaagagagtgatcctggccgacgctaatctggacaaagtgctgtccgcctacaacaagcaccgggataagcccatcagagagcaggccgagaatatcatccacctgtttaccctgaccaatctgggagcccctgccgccttcaagtactttgacaccaccatcgaccggaagaggtacaccagcaccaaagaggtgctggacgccaccctgatccaccagagcatcaccggcctgtacgagacacggatcgacctgtctcagctgggaggcgacagccccaagaagaagagaaaggtggaggccagctaacatatgattcgaatgtctttcttgcgctatgacacttccagcaaaaggtagggcgggctgcgagacggcttcccggcgctgcatgcaacaccgatgatgcttcgaccccccgaagctccttcggggctgcatgggcgctccgatgccgctccagggcgagcgctgtttaaatagccaggcccccgattgcaaagacattatagcgagctaccaaagccatattcaaacacctagatcactaccacttctacacaggccactcgagcttgtgatcgcactccgctaagggggcgcctcttcctcttcgtttcagtcacaacccgcaaacatgacacaagaatccctgttacttctcgaccgtattgattcggatgattcctacgcgagcctgcggaacgaccaggaattctgggaggtgagtcgacgagcaagcccggcggatcaggcagcgtgcttgcagatttgacttgcaacgcccgcattgtgtcgacgaaggcttttggctcctctgtcgctgtctcaagcagcatctaaccctgcgtcgccgtttccatttgcagccgctggcccgccgagccctggaggagctcgggctgccggtgccgccggtgctgcgggtgcccggcgagagcaccaaccccgtactggtcggcgagcccggcccggtgatcaagctgttcggcgagcactggtgcggtccggagagcctcgcgtcggagtcggaggcgtacgcggtcctggcggacgccccggtgccggtgccccgcctcctcggccgcggcgagctgcggcccggcaccggagcctggccgtggccctacctggtgatgagccggatgaccggcaccacctggcggtccgcgatggacggcacgaccgaccggaacgcgctgctcgccctggcccgcgaactcggccgggtgctcggccggctgcacagggtgccgctgaccgggaacaccgtgctcaccccccattccgaggtcttcccggaactgctgcgggaacgccgcgcggcgaccgtcgaggaccaccgcgggtggggctacctctcgccccggctgctggaccgcctggaggactggctgccggacgtggacacgctgctggccggccgcgaaccccggttcgtccacggcgacctgcacgggaccaacatcttcgtggacctggccgcgaccgaggtcaccgggatcgtcgacttcaccgacgtctatgcgggagactcccgctacagcctggtgcaactgcatctcaacgccttccggggcgaccgcgagatcctggccgcgctgctcgacggggcgcagtggaagcggaccgaggacttcgcccgcgaactgctcgccttcaccttcctgcacgacttcgaggtgttcgaggagaccccgctggatctctccggcttcaccgatccggaggaactggcgcagttcctctgggggccgccggacaccgcccccggcgcctgataaggatccggcaagactggccccgcttggcaacgcaacagtgagcccctccctagtgtgtttggggatgtgactatgtattcgtgtgttggccaacgggtcaacccgaacagattgatacccgccttggcatttcctgtcagaatgtaacgtcagttgatggtact

SEQ ID NO: 92 - DNA, 102 bp, synthetic construct
  misc_feature 1..102: note = source = /note="Description of Artificial Sequence: Synthetic polynucleotide"
  source 1..102: mol_type = other DNA
gttttagagctatgctgttttgaatggtcccaaaacggaagggcctgagtccgagcagaagaagaagttttagagctatgctgttttgaatggtcccaaaac

SEQ ID NO: 93 - DNA, 100 bp, Homo sapiens
  source 1..100: mol_type = unassigned DNA
cggaggacaaagtacaaacggcagaagctggaggaggaagggcctgagtccgagcagaagaagaagggctcccatcacatcaaccggtggcgcattgcca

SEQ ID NO: 94 - DNA, 50 bp, Homo sapiens
  source 1..50: mol_type = unassigned DNA
agctggaggaggaagggcctgagtccgagcagaagaagaagggctcccac

SEQ ID NO: 95 - RNA, 30 nt, synthetic construct
  misc_feature 1..30: note = source = /note="Description of Artificial Sequence: Synthetic oligonucleotide"
  source 1..30: mol_type = other RNA
gagtccgagcagaagaagaagttttagagc

SEQ ID NO: 96 - DNA, 49 bp, synthetic construct
  misc_feature 1..49: note = source = /note="Description of Artificial Sequence: Synthetic oligonucleotide"
  source 1..49: mol_type = other DNA
agctggaggaggaagggcctgagtccgagcagaagagaagggctcccat

SEQ ID NO: 97 - DNA, 53 bp, Homo sapiens
  source 1..53: mol_type = unassigned DNA
ctggaggaggaagggcctgagtccgagcagaagaagaagggctcccatcacat

SEQ ID NO: 98 - DNA, 52 bp, Homo sapiens
  source 1..52: mol_type = unassigned DNA
ctggaggaggaagggcctgagtccgagcagaagagaagggctcccatcacat

SEQ ID NO: 99 - DNA, 54 bp, Homo sapiens
  source 1..54: mol_type = unassigned DNA
ctggaggaggaagggcctgagtccgagcagaagaaagaagggctcccatcacat

SEQ ID NO: 100 - DNA, 50 bp, Homo sapiens
  source 1..50: mol_type = unassigned DNA
ctggaggaggaagggcctgagtccgagcagaagaagggctcccatcacat

SEQ ID NO: 101 - DNA, 47 bp, Homo sapiens
  source 1..47: mol_type = unassigned DNA
ctggaggaggaagggcctgagcccgagcagaagggctcccatcacat

SEQ ID NO: 102 - RNA, 155 nt, synthetic construct
  misc_feature 1..155: note = source = /note="Description of Artificial Sequence: Synthetic polynucleotide"
  source 1..155: mol_type = other RNA
gtttcagtgctataggaaactataggaaatcaccttcgggtgagctgaaatcccctaaagctaagattgaatccggccactatctattagtagatatccggatattctgatataaaacctcattctttgattagaccaaaggatgaggttttttt

SEQ ID NO: 103 - RNA, 107 nt, synthetic construct
  misc_feature 1..107: note = source = /note="Description of Artificial Sequence: Synthetic polynucleotide"
  source 1..107: mol_type = other RNA
gtttgagagttggaaacaacgagttcaaataagaattcatcaaaatcgtcccttttgggaccgctcattgtggagcatcaaggcttaacatggttaagccttttttt

SEQ ID NO: 104 - RNA, 99 nt, synthetic construct
  misc_feature 1..99: note = source = /note="Description of Artificial Sequence: Synthetic oligonucleotide"
  source 1..99: mol_type = other RNA
gtttgagagtaggaaactacacggttcaaataaagaatttttctaatcgcccaatgggcccatattgatatggatgaaactcgcttagcgagttttttt

SEQ ID NO: 105 - RNA, 91 nt, synthetic construct
  misc_feature 1..91: note = source = /note="Description of Artificial Sequence: Synthetic oligonucleotide"
  source 1..91: mol_type = other RNA
gttttagcactagaaatagttaagttaaaacaagcttaaagcgtcaatgtaatattttattaacaccctactgtgtcagtggggttttttt

SEQ ID NO: 106 - RNA, 94 nt, synthetic construct
  misc_feature 1..94: note = source = /note="Description of Artificial Sequence: Synthetic oligonucleotide"
  source 1..94: mol_type = other RNA
gttttagatggtgaaaaccagatttaaaatcaagcaatgcatcttttgatgcaaagtttcaatatttgtcccacgttatcgagggacttttttt

SEQ ID NO: 107 - RNA, 78 nt, synthetic construct
  misc_feature 1..78: note = source = /note="Description of Artificial Sequence: Synthetic oligonucleotide"
  source 1..78: mol_type = other RNA
attttagtacctggaaacagatctactaaaacaaggctttatgccgaaatcaagagcaccgacgggtgctcttttttt

SEQ ID NO: 108 - RNA, 84 nt, synthetic construct
  misc_feature 1..84: note = source = /note="Description of Artificial Sequence: Synthetic oligonucleotide"
  source 1..84: mol_type = other RNA
gtttttgtactcgaaagagcctacaaagataaggctttatgccgaattcaagcaccccatgttttgacatgaggtgcttttttt

SEQ ID NO: 109 - RNA, 85 nt, synthetic construct
  misc_feature 1..85: note = source = /note="Description of Artificial Sequence: Synthetic oligonucleotide"
  source 1..85: mol_type = other RNA
gtttttgtaccttagaaataagatctacaaaaataaggatttattccgaatttaccacctattttaattaataggtggttttttt

SEQ ID NO: 110 - RNA, 100 nt, synthetic construct
  misc_feature 1..100: note = source = /note="Description of Artificial Sequence: Synthetic polynucleotide"
  source 1..100: mol_type = other RNA
gttgtgatttgctttcatttgaaaaattgaagcaaatcacaataaggattattccgttgtgaaaacaattaaagcggtcttgcaaaaggtcgcttttttt

SEQ ID NO: 111 - RNA, 102 nt, synthetic construct
  misc_feature 1..102: note = source = /note="Description of Artificial Sequence: Synthetic polynucleotide"
  source 1..102: mol_type = other RNA
gttgtgattcgctttcaatgaaaattgaagcgaatcacaataaggattattccgttgtgaaaacatttactacggggcatcgaaagactgcctcgttttttt

SEQ ID NO: 112 - RNA, 90 nt, synthetic construct
  misc_feature 1..90: note = source = /note="Description of Artificial Sequence: Synthetic oligonucleotide"
  source 1..90: mol_type = other RNA
gttgtggtttgattagaaataatcttatcacaataaggctatatgccgtagacgaaagtctttagtcccgcttcggtgggactttttttt

SEQ ID NO: 113 - RNA, 78 nt, synthetic construct
  misc_feature 1..78: note = source = /note="Description of Artificial Sequence: Synthetic oligonucleotide"
  source 1..78: mol_type = other RNA
gttggggatgaccgcgaaagcgattatctctaataagacttaagtcgcaaaatgctccctattttgggagcttttttt

SEQ ID NO: 114 - RNA, 85 nt, synthetic construct
  misc_feature 1..85: note = source = /note="Description of Artificial Sequence: Synthetic oligonucleotide"
  source 1..85: mol_type = other RNA
gttgcggctggagaaatccagccgttaacatgttcccttcggggagcacgaaatgcggggcgggccacggtccgccccttttttt

SEQ ID NO: 115 - RNA, 126 nt, synthetic construct
  misc_feature 1..126: note = source = /note="Description of Artificial Sequence: Synthetic polynucleotide"
  source 1..126: mol_type = other RNA
gccgtggtttccgaaaggaaaccacggtaacagaattaccgtaaggttttttctgtgaaggatcatccctcgcttgggcaaccaggcgggggaaattcctcgttcgggccaatcagcccttttttt

SEQ ID NO: 116 - RNA, 82 nt, synthetic construct
  misc_feature 1..82: note = source = /note="Description of Artificial Sequence: Synthetic oligonucleotide"
  source 1..82: mol_type = other RNA
gttgtaattccctgaaaaggttattacaataaggtaagaaacctaaaagctctaatcccattcttcggaatgggattttttt

SEQ ID NO: 117 - RNA, 83 nt, synthetic construct
  misc_feature 1..83: note = source = /note="Description of Artificial Sequence: Synthetic oligonucleotide"
  source 1..83: mol_type = other RNA
gttttagtactctggaaacagaatctactaaaacaaggcaaaatgccgtgtttatctcgtcaacttgttggcgagattttttt

SEQ ID NO: 118 - RNA, 94 nt, synthetic construct
  misc_feature 1..94: note = source = /note="Description of Artificial Sequence: Synthetic oligonucleotide"
  source 1..94: mol_type = other RNA
gttttagcactgtacaagaaattgtcgtgctaaaataaggcgctgttaatgcagctgccgcatccgccagagcatttatgctctggcttttttt

SEQ ID NO: 119 - DNA, 4350 bp, synthetic construct
  misc_feature 1..4350: note = source = /note="Description of Artificial Sequence: Synthetic polynucleotide"
  source 1..4350: mol_type = other DNA
accggtgccaccatgtacccatacgatgttccagattacgcttcgccgaagaaaaagcgcaaggtcgaagcgtccatgactcagagcgagcgacgattttcttgcagcattggcattgacatgggggctaagtacactggggtgttctacgcactgttcgaccgggaggaactgcccacaaacctgaacagcaaggccatgaccctggtcatgcctgagacagggccaagatacgtgcaggcacagagaactgccgtcagacacaggctgcgcggacagaagagatataccctggctaggaaactggcatttctggtggtcgacgatatgatcaagaaacaggaaaagaggctgactgatgaggaatggaaacgaggacgggaggccctgtccggcctgctgaagcggagagggtactctcggcccaacgctgacggcgaagatctgacccctctggagaatgtgagagcagacgtgttcgccgctcatcctgccttcagcacatatttttccgaagtgcgctctctggctgagcagtgggaggagttcaccgcaaacatcagcaatgtcgagaagtttctgggcgacccaaacatccccgccgataaagagttcattgaatttgccgtggctgaagggctgattgacaagaccgagaagaaagcctaccagtcagctctgagcaccctgagggcaaacgccaatgtgctgacaggactgcggcagatgggccacaagcctagatcagaatattttaaagcaatcgaggccgacctgaagaaagatagccgcctggccaagattaacgaagcattcggaggagcagagcgcctggctcgactgctgggaaacctgtccaatctgcagctgcgggcagaaagatggtacttcaatgcccccgacatcatgaaggataggggctgggagcctgatcgcttcaagaaaacactggtgcgggcttttaagttctttcacccagcaaaggaccagaacaaacagcatctggaactgatcaaacagattgagaacagcgaagatatcattgagactctgtgcaccctggacccaaacagaaccatccccccttacgaggatcagaacaataggcgcccacccctggaccagactctgctgctgagtcccgaaaagctgacccggcagtatggcgagatctggaaaacatggagcgccagactgacctccgctgaacccacactggcacctgcagccgagattctggaaagatctaccgacaggaagagtcgcgtggcagtcaacggacacgagccactgcctacactggcttaccagctgagttatgcactgcagagagccttcgacaggtcaaaagccctggatccatatgctctgagggcactggctgcaggctcaaaaagcaataagctgacatccgcccgcactgctctggagaactgcatcggaggccagaatgtgaaaaccttcctggactgtgcccgacggtactatcgggaagcagacgatgccaaagtcgggctgtggttcgacaacgccgatggactgctggagagatctgacctgcatcctccaatgaagaaaaagatcctgcccctgctggtggccaatattctgcagacagatgaaaccacaggccagaagtttctggacgagatctggcgaaaacagattaaggggcgggaaactgtggctagccgatgtgcacggatcgagacagtgcggaaatccttcgggggaggctttaacattgcctacaataccgctcagtatagggaggtgaacaagctgccccgcaatgcccaggataaagaactgctgacaatcagagatagggtggctgagactgcagacttcattgccgctaacctggggctgtctgacgagcagaaaagaaagttcgccaatccttttagtctggctcagttctacaccctgatcgagacagaagtgtccggattttctgcaactaccctggccgtccacctggagaacgcctggaggatgacaatcaaggatgctgtgattaatggggaaactgtcagagcagcacagtgcagcaggctgcctgcagagacagctcgcccattcgatggactggtgagaaggctggtcgacagacaggcttgggagatcgcaaagagggtgtcaactgacattcagagcaaagtcgatttctccaacggcatcgtggacgtcagcatttttgtggaggaaaataagttcgagttttccgcatctgtggccgatctgaaaaagaacaaacgggtcaaagacaagatgctgtccgaggccgaaaagctggaaaccagatggctgatcaaaaatgagcggatcaagaaggccagccggggaacttgtccctacaccggcgataggctggctgaggggggagaaatcgaccacattctgccccgaagcctgatcaaggatgcccggggaattgtgtttaacgctgagcctaatctgatctatgcaagctcccgcggcaaccagctgaaaaagaatcagcgatacagtctgtcagatctgaaggccaactatcggaatgagatcttcaaaactagcaacatcgctgcaattaccgccgagattgaggacgtggtcactaagctgcagcagacccatagactgaaattctttgatctgctgaatgagcacgaacaggactgcgtgcggcacgccctgttcctggacgatggcagcgaagctcgcgacgcagtgctggagctgctggcaacacagcgccgaactcgcgtcaacgggacacagatctggatgattaagaacctggccaacaagatccgagaggaactgcagaattggtgtaagacaactaacaatagactgcactttcaggccgctgcaactaacgtgtccgatgcaaagaatctgaggctgaaactggcccagaaccagcccgacttcgagaagccagatatccagcccattgccagccattccatcgacgccctgtgctctttcgctgtggggagtgctgacgcagaacgcgatcagaatggatttgactacctggatggcaagaccgtgctgggactgtatccacagagctgtgaggtcattcacctgcaggccaagccccaggaggaaaaaagtcatttcgattcagtggctatctttaaggaaggcatctacgcagagcagttcctgcctatctttaccctgaacgaaaagatctggattggatatgagacactgaatgccaaaggcgaaagatgcggggctattgaggtgagtggcaaacagccaaaggagctgctggaaatgctggcccccttctttaacaagcctgtgggcgacctgtcagcccacgctacttaccggatcctgaaaaagcctgcatatgagtttctggcaaaggcagctctgcagccactgagcgcagaggaaaaaagactggcagccctgctggatgctctgcgctactgtaccagtcgaaagtcactgatgagcctgttcatggctgcaaacgggaaatccctgaaaaagcgggaggacgtgctgaaacccaagctgttccagctgaaggtcgagctgaaaggcgaaaagagcttcaagctgaacgggagcctgaccctgcctgtgaagcaggactggctgagaatctgcgatagcccagaactggcagacgcctttggcaaaccctgttccgccgatgagctgacatctaagctggctcgcatttggaaacgacctgtgatgcgggatctggctcatgcaccagtccggagagagttcagcctgcccgcaatcgacaacccaagtggagggttcaggattaggcgcaccaacctgtttggcaatgagctgtaccaggtgcacgccatcaacgctaaaaagtatcgcggcttcgcctccgctgggtctaatgtcgactggtccaaggggatcctgtttaacgagctgcagcatgaaaatctgaccgagtgcggaggcaggttcattacaagcgccgatgtgactcctatgtccgaatggcgcaaggtggtcgcagaggacaacctgtctatctggattgctccagggacagaaggacgacggtacgtgagggtcgagacaacattcatccaggccagtcactggtttgaacagtcagtggagaattgggccattactagtcctctgtcactgccagcttccttcaaggtggacaaaccagctgagtttcagaaggcagtcggaaccgagctgtcagaactgctgggccagcccaggagcgaaatcttcattgagaacgtgggcaatgccaagcatatccgcttttggtacattgtggtgagcagcaacaaaaagatgaacgagtcttacaacaatgtgtctaagagttaagaattc

SEQ ID NO: 120 - DNA, 4269 bp, synthetic construct
  misc_feature 1..4269: note = source = /note="Description of Artificial Sequence: Synthetic polynucleotide"
  source 1..4269: mol_type = other DNA
accggtgccaccatgtacccatacgatgttccagattacgcttcgccgaagaaaaagcgcaaggtcgaagcgtccatgaaaaaagaaatcaaagactacttcctggggctggatgtggggactgggagcgtggggtgggctgtgaccgatactgactacaaactgctgaaggctaaccgaaaagacctgtggggcatgagatgcttcgagacagccgaaactgctgaggtgcggagactgcacaggggagccaggcgccgaatcgagcggagaaagaaacgcattaagctgctgcaggagctgttctctcaggaaatcgccaaaaccgatgagggcttctttcagagaatgaaggaaagccccttttacgctgaggacaaaacaatcctgcaggaaaacactctgttcaatgacaaggattttgctgataagacttaccacaaagcatatcctaccattaatcatctgatcaaggcttggattgagaacaaggtgaaaccagacccccgactgctgtacctggcatgtcacaacatcattaagaaaaggggacatttcctgtttgaaggcgacttcgattcagagaatcagtttgataccagcatccaggcactgttcgagtatctgcgcgaggacatggaggtggacatcgatgccgacagccagaaggtcaaagagattctgaaggatagctccctgaagaactctgaaaaacagagtcggctgaataagatcctggggctgaagccttccgacaaacagaagaaagccatcacaaacctgatttctggaaacaagatcaatttcgccgatctgtacgacaatccagatctgaaggacgctgagaaaaactcaatcagcttctccaaggacgattttgatgcactgagtgacgatctggcctcaattctgggcgacagctttgaactgctgctgaaggccaaagctgtctataactgctctgtgctgagtaaggtcatcggggacgagcagtacctgagcttcgccaaggtgaaaatctacgaaaagcacaaaaccgatctgacaaagctgaaaaacgtgatcaagaaacatttccccaaggactacaagaaggtctttggatacaacaagaacgagaaaaacaacaacaattactccggctatgtgggagtctgtaagaccaagagtaagaaactgatcattaacaactcagtcaaccaggaagatttctacaagtttctgaaaactatcctgtcagccaagagcgagatcaaggaagtgaatgacatcctgaccgagattgaaactggcacctttctgccaaagcagatctctaaaagtaacgcagagattccctatcagctgaggaaaatggagctggaaaagatcctgtccaatgccgaaaagcacttctcttttctgaagcagaaagacgaaaaaggactgtcacatagcgagaagatcattatgctgctgaccttcaagatcccttactatattggcccaatcaacgataatcacaagaaattctttcccgacagatgctgggtggtcaagaaagagaaatccccttctggcaagaccacaccatggaacttctttgatcatatcgacaaggaaaaaacagcagaggccttcattacttctaggaccaatttttgcacttacctggtgggagagagcgtcctgcctaagtctagtctgctgtactccgaatataccgtgctgaacgagatcaacaatctgcagatcattatcgatggcaagaatatttgtgacatcaagctgaaacagaagatctacgaggacctgttcaagaagtacaagaaaattacccagaagcagatcagcaccttcatcaagcacgaaggcatctgcaacaaaaccgatgaagtgatcatcctggggattgacaaggaatgtacatcaagcctgaaaagctacatcgagctgaaaaacattttcggcaagcaggtggatgagatctccactaagaatatgctggaggaaattatcagatgggctaccatctacgacgagggggaaggaaagaccatcctgaaaacaaagatcaaggcagaatacggaaagtattgctccgacgagcagattaagaaaatcctgaacctgaagttctccggctgggggcgactgtctcggaaatttctggagacagtgactagtgaaatgcccggcttctcagaacctgtcaatattatcaccgccatgagggagacacagaacaatctgatggagctgctgtcctctgagttcaccttcaccgagaacattaagaaaatcaattctggattcgaagatgccgagaagcagtttagttacgacggcctggtgaaaccactgtttctgagtccctcagtcaagaaaatgctgtggcagaccctgaagctggtgaaagagattagccatatcacacaggccccccctaagaaaattttcatcgaaatggcaaagggggccgagctggaacctgctcggactaagaccagactgaaaatcctgcaggatctgtataacaattgtaagaacgatgctgacgccttcagctcagagatcaaagacctgagcggaaagattgagaacgaagataatctgaggctgcgctccgacaagctgtacctgtactatactcagctggggaaatgcatgtattgtggaaagccaattgagatcggccacgtgttcgatacctcaaactacgatattgaccatatctatccccagagcaagatcaaagacgatagcatttccaatcgggtgctggtctgcagctcctgtaacaagaacaaggaggacaagtacccactgaaatcagagatccagagcaagcagcgcggcttctggaactttctgcagcgaaacaatttcatttctctggagaagctgaatagactgacaagggccactccaatcagtgacgatgagacagccaagtttattgctaggcagctggtggaaactcgccaggctaccaaggtggccgctaaagtcctggaaaagatgttccccgagacaaaaatcgtgtacagcaaggccgagactgtctccatgttccggaacaagtttgatatcgtgaagtgcagagaaattaacgattttcaccatgctcacgacgcatacctgaatatcgtggtcggcaacgtgtataataccaagttcacaaacaatccttggaactttatcaaggagaaaagagataatccaaagattgctgacacctacaactactataaggtgttcgattatgacgtcaaaaggaacaatatcacagcatgggagaaggggaaaactattatcaccgtgaaagacatgctgaagagaaacacaccaatctacactaggcaggcagcctgtaagaaaggggagctgttcaatcagaccattatgaagaaaggactgggccagcaccccctgaagaaagaaggacctttttccaatatctctaaatacggcgggtataacaaggtgagcgctgcatactatacactgattgagtatgaggaaaagggcaacaaaatccgctccctggaaactattcccctgtacctggtgaaagatatccagaaggatcaggacgtcctgaagtcttatctgacagacctgctggggaagaaagagttcaagatcctggtgcccaagatcaagatcaacagcctgctgaagatcaatgggtttccttgccatattacaggaaaaactaacgatagtttcctgctgcgccctgccgtgcagttttgctgttcaaacaatgaggtcctgtacttcaagaaaattatccggttttccgaaatccgctctcagcgagagaagatcgggaaaacaattagcccatacgaggacctgagcttccggtcatatatcaaggagaacctgtggaagaaaactaagaacgatgaaatcggagagaaggaattttacgacctgctgcagaagaaaaacctggagatctatgatatgctgctgactaagcacaaagacaccatctacaagaaacgccctaattctgccaccattgatatcctggtgaaggggaaagagaagttcaaaagcctgattatcgaaaaccagtttgaagtgatcctggagatcctgaagctgttttctgcaacacggaatgtcagtgacctgcagcatatcggaggcagcaagtactccggcgtggccaaaatcgggaacaagatctctagtctggataactgtatcctgatctatcagtccatcaccggcatcttcgagaaacggatcgacctgctgaaggtgtaagaattc

SEQ ID NO: 121 - DNA, 4179 bp, synthetic construct
  misc_feature 1..4179: note = source = /note="Description of Artificial Sequence: Synthetic polynucleotide"
  source 1..4179: mol_type = other DNA
accggtgccaccatgtacccatacgatgttccagattacgcttcgccgaagaaaaagcgcaaggtcgaagcgtccatgaccaaggagtattacctggggctggatgtggggaccaattccgtgggatgggcagtgaccgattctcagtacaacctgtgcaagtttaagaaaaaggatatgtggggcatccggctgttcgaaagcgccaacacagcaaaggaccggagactgcagagagggaataggcgccgactggagcggaaaaagcagagaattgatctgctgcaggaaatcttctccccagagatctgcaagattgaccccactttctttatccgactgaacgaatcccggctgcacctggaggacaagtctaacgatttcaaatacccactgtttattgagaaggactattctgatatcgagtactataaagagttccccaccatttttcacctgaggaagcatctgatcgagagtgaggaaaaacaggatatccggctgatctacctggccctgcacaacatcattaagacccgaggacattttctgattgacggcgatctgcagagcgccaagcagctgaggcccatcctggatacattcctgctgtccctgcaggaggaacagaacctgtcagtgagcctgtccgaaaatcagaaggacgagtatgaggaaattctgaaaaaccgcagcatcgccaagtccgaaaaagtgaaaaagctgaagaatctgtttgagatctcagacgagctggaaaaagaggagaagaaggcccagagcgccgtgatcgagaacttctgcaagtttatcgtgggaaataagggcgatgtctgtaaattcctgcgggtgtctaaggaggaactggagattgactctttcagtttttcagagggcaagtacgaggacgacatcgtgaaaaacctggaggaaaaagtgcctgaaaaggtctacctgtttgagcagatgaaggcaatgtatgattggaatattctggtcgacatcctggaaaccgaggaatacatcagcttcgccaaagtgaagcagtatgagaaacacaagactaacctgcggctgctgagagacatcattctgaaatactgcaccaaggatgagtataatcggatgtttaacgacgagaaggaagctggcagctacaccgcatatgtggggaaactgaaaaagaacaacaagaagtactggatcgagaaaaagagaaatcccgaggagttctacaaatccctgggcaagctgctggataaaattgagcctctgaaggaggacctggaagtgctgactatgatgatcgaggagtgtaagaaccacaccctgctgccaattcagaaaaataaggacaacggcgtgatcccccaccaggtgcatgaggtcgaactgaaaaagatcctggaaaatgccaaaaagtactattccttcctgaccgagacagacaaggatgggtactcagtggtccagaaaatcgagagcattttcaggtttcgcatcccctactatgtggggcctctgagtacccggcaccaggaaaagggatcaaacgtgtggatggtcagaaaacctggcagggaggatcgcatctacccatggaatatggaggaaatcattgactttgagaagagcaacgaaaatttcattacacggatgactaacaaatgtacatatctgatcggggaagatgtcctgcccaagcattctctgctgtacagtaaatatatggtgctgaatgagctgaacaatgtgaaggtcagaggaaaaaagctgcctacatctctgaaacagaaggtgttcgaggacctgtttgaaaacaaatccaaagtgactggaaagaatctgctggagtacctgcagatccaggacaaagatatccagattgacgatctgtctggcttcgacaaggacttcaagaccagcctgaagagctatctggacttcaaaaagcagatttttggggaggaaatcgagaaggaaagcattcagaacatgatcgaagatatcattaagtggatcaccatctacggcaatgacaaggagatgctgaaacgagtgattcgggctaattatagcaaccagctgacagaggaacagatgaaaaagatcactggatttcagtacagtggctgggggaacttctcaaagatgtttctgaaagggatcagcggatccgacgtgagcaccggcgaaacattcgacatcattaccgcaatgtgggagacagacaacaatctgatgcagatcctgtcaaaaaagttcacctttatggacaacgtcgaggacttcaacagcggcaaggtcgggaaaatcgacaagattacttacgatagcaccgtgaaggaaatgttcctgtcccctgagaacaaaagggccgtctggcagaccattcaggtggctgaggagatcaagaaagtgatgggctgcgagccaaaaaagatctttattgaaatggcacggggcggggagaaggtgaaaaagaggacaaaatctcgcaaggcccagctgctggagctgtacgccgcttgcgaggaagattgtagagaactgatcaaggagattgaggaccgggacgagagggacttcaatagcatgaagctgtttctgtactatacccagttcgggaaatgtatgtattccggcgacgacatcgatattaacgagctgattcgcggcaattctaagtgggaccgagatcacatctacccccagagcaaaattaaggacgattccatcgataacctggtgctggtcaataagacatataatgccaaaaagtccaatgagctgctgtctgaggacatccagaaaaagatgcattcattctggctgagcctgctgaacaaaaagctgatcactaaaagcaagtacgaccgcctgactcgaaagggcgactttaccgatgaggaactgagtgggttcatcgctagacagctggtggaaacaaggcagtcaactaaggcaatcgccgatatcttcaagcagatctacagctccgaggtggtctatgtgaagagcagcctggtgagcgacttcaggaaaaagccactgaactacctgaagtctcggagagtcaatgattaccaccatgcaaaagacgcctatctgaacattgtggtcgggaacgtgtacaacaaaaagtttaccagtaatcccatccagtggatgaaaaagaatcgcgatacaaactatagcctgaacaaggtgttcgaacacgacgtggtcattaacggagaagtgatctgggaaaagtgcacataccatgaggacactaatacctatgatggaggcactctggaccgaatccggaagattgtggaacgcgataacattctgtacaccgagtacgcttattgtgagaagggcgaactgtttaatgcaaccatccagaacaaaaatggaaactccacagtctctctgaaaaagggcctggacgtgaaaaagtacgggggatacttcagcgccaacacaagttacttctcactgatcgagtttgaggacaagaagggggatagagcaaggcacatcattggagtgcctatctatattgcaaacatgctggagcattctccaagtgccttcctggagtactgcgaacagaaggggtatcagaatgtgcggattctggtcgagaaaatcaaaaagaacagcctgctgatcattaatggataccctctgcgcattcgaggcgagaacgaagtggatacttcctttaagagggccatccagctgaagctggaccagaaaaactatgagctggtccgcaatatcgagaagttcctggaaaaatacgtggagaaaaagggaaactatccaattgacgagaatagagatcacatcacacatgaaaagatgaaccagctgtacgaggtgctgctgtccaaaatgaaaaagttcaacaagaagggcatggccgacccctctgataggatcgaaaagagtaagcctaaattcatcaagctggaggacctgatcgataagattaatgtgatcaacaaaatgctgaacctgctgcgctgtgacaatgatactaaggccgacctgtctctgattgagctgcccaaaaacgctgggagtttcgtggtcaaaaagaataccatcggaaagtcaaaaatcatcctggtgaatcagagcgtgactggactgtacgagaatagacgggaactgtaagaattc

SEQ ID NO: 122 - DNA, 4086 bp, synthetic construct
  misc_feature 1..4086: note = source = /note="Description of Artificial Sequence: Synthetic polynucleotide"
  source 1..4086: mol_type = other DNA
accggtgccaccatgtacccatacgatgttccagattacgcttcgccgaagaaaaagcgcaaggtcgaagcgtccatggggaggaaaccttacattctgtctctggatattggaactgggtccgtcggctacgcttgcatggataaaggattcaacgtgctgaagtaccacgacaaagatgccctgggagtgtatctgttcgacggcgctctgactgcacaggagcggagacagtttaggacctccaggcgccgaaagaaccggagaatcaaacgcctgggcctgctgcaggaactgctggcacccctggtgcagaaccctaatttctaccagtttcagcggcagttcgcctggaagaacgacaatatggattttaagaacaagagcctgtctgaggtgctgagcttcctgggatatgaatccaagaaataccctaccatctaccacctgcaggaggctctgctgctgaaagacgagaagtttgatccagaactgatctacatggcactgtatcatctggtgaaatacagaggccactttctgttcgatcatctgaagatcgagaacctgactaacaatgacaatatgcacgatttcgtggagctgattgaaacctatgagaacctgaacaatatcaagctgaatctggactacgagaaaaccaaagtgatctatgagattctgaaagacaacgaaatgactaagaatgatagagccaaaagggtcaagaacatggagaagaaactggaacagttctctatcatgctgctggggctgaagttcaatgagggaaaactgtttaaccacgccgataatgctgaggaactgaagggggctaaccagagccatacatttgcagacaactacgaggaaaatctgactcccttcctgaccgtggaacagtcagagtttattgaaagggccaacaaaatctatctgagcctgactctgcaggatatcctgaagggcaagaaatcaatggctatgagcaaagtggccgcttacgacaagttcagaaatgagctgaaacaggtgaaggacattgtctataaggctgattctaccaggacacagttcaagaaaatctttgtgagctccaagaaaagtctgaagcagtacgacgcaactcccaacgatcagaccttctctagtctgtgcctgtttgaccagtacctgattcgcccaaagaaacagtatagcctgctgatcaaggagctgaagaaaatcattccccaggactccgaactgtactttgaggcagaaaatgataccctgctgaaggtgctgaacaccacagacaatgctagcatccctatgcagattaacctgtacgaggcagaaaccatcctgcgaaatcagcagaaatatcacgccgagatcacagatgagatgattgaaaaggtgctgtctctgatccagttccgcattccatactatgtggggcccctggtcaacgaccatacagccagtaagtttggatggatggagcgcaaaagtaacgaatcaatcaagccttggaatttcgacgaggtggtcgatcgaagtaaatcagccactcagtttattaggcgcatgaccaacaagtgttcctacctgatcaatgaggatgtgctgccaaaaaactctctgctgtatcaggagatggaagtcctgaacgaactgaatgccacacagatcaggctgcagactgacccaaaaaaccgcaagtaccgaatgatgccccagattaagctgttcgctgtggagcacatctttaagaaatataaaaccgtcagccattccaagttcctggaaattatgctgaacagcaatcacagggagaactttatgaatcatggagaaaagctgagtatcttcggcacacaggacgataagaaatttgcatcaaagctgtcaagctaccaggacatgactaaaatcttcggggatattgagggaaagcgcgcccagattgaggaaatcattcagtggatcaccatttttgaggacaagaaaatcctggtgcagaagctgaaagagtgctatcctgaactgacatccaagcagatcaaccagctgaagaaactgaattactctggctgggggaggctgagtgagaagctgctgactcacgcctatcagggccatagcatcattgaactgctgcgccactccgatgagaatttcatggaaattctgaccaacgacgtgtacgggttccagaattttatcaaagaggaaaaccaggtccagagcaataagatccagcatcaggatattgccaacctgactacctctcccgctctgaagaaaggcatctggagtacaattaagctggtgcgggagctgacttccattttcggggagcctgaaaagatcattatggagtttgctaccgaggaccagcagaaaggcaagaaacagaaatcaagaaagcagctgtgggacgataacatcaagaaaaataagctgaaaagcgtggacgagtacaaatatatcattgatgtcgccaataagctgaacaatgagcagctgcagcaggaaaaactgtggctgtacctgagccagaacggcaagtgtatgtatagcgggcagtccatcgacctggatgccctgctgtcccccaatgctaccaagcactacgaggtggatcatattttccctcggagcttcatcaaggacgatagcattgacaacaaggtgctggtcatcaagaaaatgaatcagacaaagggcgatcaggtgcccctgcagttcattcagcagccttacgagagaatcgcatattggaagagcctgaacaaagccgggctgatctctgatagtaaactgcacaagctgatgaaaccagagttcacagctatggacaaggaaggcttcatccagcggcagctggtggagactagacagatcagcgtgcatgtccgggattttctgaaagaggaataccctaataccaaagtgatcccaatgaaggccaaaatggtgagcgagttccggaagaaatttgacatcccaaagattagacagatgaacgacgcacaccatgccatcgatgcttacctgaatggcgtggtctatcacggggcacagctggcctaccccaacgtggacctgtttgatttcaattttaagtgggagaaagtccgagaaaagtggaaagccctgggagagttcaacacaaagcagaaatctcgggaactgttctttttcaagaaactggagaagatggaagtgtcccagggcgagcggctgatctctaagatcaagctggacatgaaccacttcaagatcaactactccagaaagctggccaacatccctcagcagttttataatcagaccgcagtgtctccaaagacagccgagctgaaatacgaatctaacaagagtaatgaggtggtctataagggactgacaccataccagacttatgtggtcgccatcaagagcgtgaacaagaaaggcaaggagaaaatggaataccagatgatcgaccactacgtgttcgatttttataaattccagaacggcaatgagaaggaactggctctgtacctggcacagagggagaacaaggacgaagtgctggatgctcagattgtctatagtctgaataagggggatctgctgtacatcaacaatcatccctgctatttcgtgtcacgcaaagaggtcatcaacgcaaagcagtttgagctgaccgtggaacagcagctgtctctgtacaacgtgatgaacaacaaggagacaaatgtcgaaaagctgctgatcgagtatgacttcattgccgagaaagtgatcaacgaataccaccattatctgaatagcaagctgaaagaaaagcgagtccggacctttttctcagagagcaaccagacacacgaggacttcatcaaggccctggacgagctgtttaaggtggtcaccgcatccgccacaaggtctgataaaatcgggagtcgcaagaacagcatgactcatcgagccttcctgggaaaaggcaaggacgtgaagattgcttacacctccatctctggactgaaaacaactaaacctaagagtctgtttaagctggccgagtcaagaaacgaactgtaagaattc

SEQ ID NO: 123 - DNA, 4209 bp, synthetic construct
  misc_feature 1..4209: note = source = /note="Description of Artificial Sequence: Synthetic polynucleotide"
  source 1..4209: mol_type = other DNA
accggtgccaccatgtacccatacgatgttccagattacgcttcgccgaagaaaaagcgcaaggtcgaagcgtccatgacaaaaatcaaagacgactacatcgtgggactggacatcggcacagactcctgcgggtgggtggctatgaacagcaataatgacattctgaaactgcagggcaagaccgcaatcgggtcacgcctgttcgagggagggaagagcgcagctgaacggagactgtttcgcaccacacacaggcgcatcaaacgacggagatggcgactgaagctgctggaggagttcttcgacccctacatggcagaggtggatccttatttctttgcccggctgaaggaatctggcctgagtccactggacaaaagaaagaccgtgagctccattgtgttccccacatccgccgaggataagaagttctacgacgattaccctacaatctaccatctgaggtataaactgatgactgaggacgaaaagttcgatctgcgcgaagtgtacctggctatccaccatatcattaagtaccgaggaaacttcctgtataataccagtgtgaaagacttcaaggcatcaaagatcgatgtcaaatctagtatcgagaagctgaacgagctgtatgaaaatctgggcctggacctgaacgtggagttcaacattagcaatactgccgagatcgaaaaggtgctgaaagacaagcagatcttcaagcgggataaagtcaagaaaattgccgagctgtttgctatcaaaaccgacaacaaggaacagagcaagagaatcaaagatatttccaaacaggtggccaatgctgtcctggggtacaagaccaggttcgacacaatcgctctgaaagagatttccaaggacgaactgtctgattggaacttcaaactgtcagacatcgatgcagacagcaagtttgaggccctgatgggaaacctggatgagaatgaacaggccatcctgctgactattaaggagctgtttaacgaagtgaccctgaatggaattgtcgaggacggcaacaccctgagcgaatccatgatcaacaagtacaatgatcaccgggacgatctgaagctgctgaaagaagtgatcgaaaatcatattgacagaaagaaagccaaggagctggcactggcctacgatctgtatgtcaacaataggcacggacagctgctgcaggctaagaaaaagctgggcaaaatcaagccccgctctaaggaggacttctacaaagtggtcaacaagaatctggacgattcacgggcaagcaaggagatcaaaaagaaaattgaactggacagctttatgcctaagcagagaaccaacgccaatggcgtgatcccataccagctgcagcagctggagctggataagatcatcgaaaaccagtctaagtactatccattcctgaaggagattaatcccgtgtcaagccacctgaaagaggccccctataagctggacgaactgatccgatttcgggtgccttactatgtcggccccctgatttctcctaacgagagtaccaaggatatccagacaaagaaaaaccagaatttcgcctggatgattcgcaaagaggaagggcgaatcacaccttggaactttgaccagaaggtggatcgaattgagagcgccaataagttcatcaaacggatgactaccaaggacacttacctgtttggggaggatgtgctgccagctaacagcctgctgtatcagaagttcaccgtcctgaacgaactgaacaacatccggattaatggaaaaagaatctccgtggacctgaagcaggagatctacgaaaacctgtttaagaaacacacaactgtgaccgtcaagaaactggagaattatctgaaggaaaaccataatctggtgaaagtcgagatcaaggggctggccgatgaaaagaaattcaacagcggactgaccacatacaatagattcaagaacctgaacatctttgacaaccagattgacgatctgaagtacaggaacgatttcgagaagatcatcgaatggtctacaatttttgaggacaagagtatctacaaagaaaagctgaggagcatcgattggctgaacgagaagcagattaacgctctgtctaatatcagactgcaggggtggggaaggctgagtaagaaactgctggcacagctgcacgaccataatggccagaccatcattgagcagctgtgggattcccagaacaatttcatgcagattgtgacacaggccgactttaaagatgctatcgcaaaggccaaccagaatctgctggtggctacctcagtcgaggacattctgaacaatgcatacacaagccccgcaaacaagaaagccatcagacaggtcatcaaggtggtcgacgatatcgtgaaggcagcctccggaaaggtcccaaaacagatcgccattgagttcactagggatgctgacgaaaatcccaagagaagtcagaccaggggctcaaagctgcagaaagtgtacaaggacctgagcactgagctggcctccaagaccattgctgaggaactgaacgaagcaatcaaagacaagaaactggtgcaggataagtactatctgtactttatgcagctggggcgggacgcctatacaggagagcctatcaatatcgatgaaatccagaagtacgatatcgaccacattctgccacagtctttcatcaaggacgatgccctggacaacagggtgctggtgagccgggctgtgaacaatggcaaatctgataatgtgcctgtcaagctgtttggcaacgagatggctgcaaatctggggatgactatcaggaaaatgtgggaggaatggaagaacatcggcctgattagcaaaacaaagtacaacaatctgctgactgatcccgaccacattaacaagtataagagtgccgggttcatcaggcgccagctggtggagacatcacagatcatcaagctggtgagcactatcctgcagagtcgctaccctaacactgaaatcattaccgtgaaggctaagtacaatcattatctgcgggagaaatttgacctgtataagagcagagaagtcaacgactaccaccatgctattgatgcatatctgtccgccatctgcggaaatctgctgtaccagaactatccaaatctgcggcccttctttgtgtacggccagtataagaaattctcctctgatcctgacaaagagaaggccatttttaacaaaacccgcaagttctcctttatctctcagctgctgaaaaacaagagtgagaacagcaaggaaatcgctaagaaactgaaacgggcataccagttcaagtatatgctggtgtctcgagagactgaaacccgggaccaggagatgttcaaaatgaccgtgtacccccggttcagccacgatacagtcaaggctcctaggaacctgattccaaagaaaatgggcatgtcccctgacatctacggaggctatacaaacaattctgacgcatacatggtcatcgtccgcattgataagaaaaagggaactgagtataagatcctgggcattccaacccgggaactggtgaatctgaaaaaggccgagaaggaggaccattacaaaagctatctgaaggagatcctgacaccaaggattctgtacaacaaaaatgggaagcgcgataaaaagatcacttccttcgaaattgtgaaatctaagatcccctataagcaggtcatccaggatggggacaaaaagtttatgctgggaagttcaacatacgtgtataacgcaaagcagctgacactgagcactgagtccatgaaagccatcactaacaatttcgataaggacagcgatgagaacgacgctctgattaaggcatacgatgaaatcctggacaaagtggataagtatctgccactgttcgacatcaacaagttccgggagaagctgcacagtgggcgagaaaagttcatcaagctgagcctggaggacaaaaaggataccatcctgaaagtgctggaaggactgcatgataacgctgtcatgacaaagatccctactattggcctgtccacaccactggggttcatgcagtttcccaacggcgtgattctgagcgagaatgccaaactgatctaccagtcccccaccgggctgttcaaaaagtcagtgaagatcagcgacctgtaagaattc

SEQ ID NO: 124 - DNA, 3405 bp, synthetic construct
  misc_feature 1..3405: note = source = /note="Description of Artificial Sequence: Synthetic polynucleotide"
  source 1..3405: mol_type = other DNA
accggtgccaccatgtacccatacgatgttccagattacgcttcgccgaagaaaaagcgcaaggtcgaagcgtccatgggctacactgtgggactggatattggggtggcttccgtcggggtggctgtgctggatgagaatgacaacatcgtggaggctgtgtcaaacatctttgatgaagccgacacaagcaacaataaggtgcggagaactctgagggagggcaggcgcacaaagcggcggcagaaaacccgcattgaggacttcaagcagctgtgggagacttcaggctacatcattcctcacaagctgcatctgaatatcattgagctgcgcaacaaagggctgaccgaactgctgagcctggatgagctgtattgcgtgctgctgtccatgctgaagcaccgggggatctcctacctggaggacgccgacgatggcgagaaggggaatgcctataagaaaggactggcttttaacgaaaaacagctgaaggagaaaatgccatgtgagatccagctggaacgcatgaagaaatacgggaagtaccatggagagttcatcatcgaaattaatgatgagaaggaataccagagcaacgtgttcaccacaaaggcttataagaaggagctggaaaagatcttcgagacacagcggtgcaacggcaacaagatcaacacaaagttcattaagaaatacatggagatctacgaacgaaagcgggaatactatatcggaccaggcaatgagaaaagcagaacagactacggcatctatactaccaggactgatgaggaagggaatttcatcgacgagaagaacatttttggcaaactgatcgggaagtgtagtgtgtaccccgaggaatatagagcaagctccgcctcatacaccgcccaggagttcaatctgctgaacgatctgaacaatctgaaaatcaacaatgagaagctgacagaatttcagaagaaagagattgtcgaaatcattaaggacgcttctagtgtgaacatgaggaaaatcattaagaaagtcatcgatgaggacattgaacagtacagcggagcacgaatcgataagaaaggcaaggaaatctaccacaccttcgagatctatcggaagctgaagaaagagctgaaaacaatcaatgtggatatcgactcttttactagagaggaactggataagaccatggacatcctgaccctgaacacagagagggaaagtattgtgaaggccttcgacgaacagaaatttgtctacgaggaaaatctgatcaagaaactgattgagtttcggaagaacaatcagagactgttcagcggctggcatagtttttcatacaaggctatgctgcagctgatcccagtgatgtacaaggagcccaaagaacagatgcagctgctgaccgaaatgaacgtgttcaaaagtaagaaagagaagtacgtcaactacaagtacatcccagagaacgaagtggtcaaggagatctataaccccgtggtcgtgaagagcattagaacaactgtgaaaattctgaatgcactgatcaagaaatacgggtatcctgaatccgtcgtgatcgagatgccaagggataagaactctgacgatgagaaggaaaagatcgacatgaaccagaagaaaaaccaggaggaatacgagaaaatcctgaacaagatctacgatgagaagggaatcgaaattaccaacaaggactacaagaaacagaagaaactggtgctgaagctgaaactgtggaacgagcaggaaggactgtgcctgtattccggcaagaaaatcgctattgaggatctgctgaatcaccccgagttctttgaaattgaccatatcattcctaagagcatctccctggacgattctcgcagtaacaaggtcctggtgtacaaaacagaaaattctatcaaggagaacgataccccctaccactatctgacacggattaacggaaagtggggctttgacgaatataaagctaatgtgctggagctgagaaggcgcggcaagatcgacgataagaaagtgaacaatctgctgtgcatggaggatatcactaagattgacgtcgtgaaagggttcattaaccgcaatctgaacgacaccagatacgcatccagggtggtgctgaacgaaatgcagtccttctttgagtctcgaaagtactgtaatactaaggtcaaagtgatccgaggctctctgacctatcagatgcggcaggatctgcacctgaagaaaaacagagaggaatcatacagccaccatgctgtggacgcaatgctgatcgcattctcccagaaggggtacgaggcctataggaagatccagaaagattgctacgactttgagacaggcgaaattctggacaaggaaaaatggaataagtacattgacgatgacgagtttgatgacatcctgtataaagagaggatgaacgaaatccgcaagaaaatcattgaggccgaggaaaaggtgaagtacaactacaagatcgataagaagtgcaatcgcgggctgtgtaaccagactatctacgggacccgagaaaaggacggaaaaatccacaagatttcaagctacaacatctatgatgacaaggagtgtaattccctgaagaaaatgattaacagtgggaaaggatcagatctgctgatgtacaacaatgatcctaagacatatcgcgacatgctgaaaatcctggaaacttactcctctgagaagaatccattcgtggcatataacaaagagacaggagactactttcggaaatattctaagaatcacaacggacccaaggtcgagaaggtgaaatactatagcggccagatcaactcctgcatcgatatttctcacaagtacggccatgccaaaaatagtaagaaagtcgtgctggtgtcactgaacccttatagaaccgacgtctactatgataatgacacaggcaagtactatctggtcggggtgaagtacaatcatatcaaatgtgtcggaaacaagtacgtgattgatagcgagacatataacgaactgctgaggaaggagggcgtgctgaacagcgatgagaacctggaggacctgaacagcaaaaacatcacttacaagttcagtctgtacaagaacgacatcatccagtacgagaagggcggggaatactatacagagcgctttctgagccgaatcaaagaacagaagaacctgattgagactaaacccatcaataagcctaacttccagcggaagaataagaaaggcgagtgggaaaataccagaaaccagatcgccctggctaagactaaatacgtggggaagctggtcaccgatgtgctgggaaactgttacatcgtgaacatggagaagttctccctggtcgtggacaaataagaattc

SEQ ID NO: 125 - DNA, 3474 bp, synthetic construct
  misc_feature 1..3474: note = source = /note="Description of Artificial Sequence: Synthetic polynucleotide"
  source 1..3474: mol_type = other DNA
accggtgccaccatgtacccatacgatgttccagattacgcttcgccgaagaaaaagcgcaaggtcgaagcgtccatgactaacggcaagattctggggctggacattggcatcgcaagcgtgggggtggggattattgaggcaaaaactggaaaggtggtgcatgccaattcccggctgttctctgccgctaacgctgagaacaatgcagaacggagagggtttaggggatctaggcgcctgaatcgacggaagaaacaccgcgtgaagcgagtccgggatctgttcgagaaatacggaatcgtcaccgactttcgcaacctgaatctgaacccttatgagctgcgagtgaagggcctgaccgaacagctgaaaaacgaggaactgttcgcagccctgagaacaatctctaagagaagggggattagttacctggacgatgccgaggacgatagtaccggatcaacagactatgctaagagcatcgatgagaatcgccgactgctgaaaaacaagacaccaggccagattcagctggagaggctggaaaagtacggccagctgcgcgggaatttcaccgtctatgacgagaacggggaagcccatcgcctgatcaatgtgtttagtacatcagattacgagaaagaagcacggaagatcctggagacacaggccgactacaacaagaaaatcacagctgagttcattgacgattatgtggaaatcctgacccagaaacgaaagtactatcacggccccgggaacgaaaagagccggactgactacggacggttccggaccgatgggaccacactggagaatattttcggaatcctgattggcaagtgcaacttttaccctgatgaatatcgagcaagcaaggccagctacaccgcacaggagtataatttcctgaacgacctgaacaatctgaaggtgagcaccgaaacagggaagctgtcaacagagcagaaagaaagcctggtggagtttgccaagaatactgctaccctgggacccgctaaactgctgaaggagatcgcaaaaattctggactgtaaggtggatgagatcaaaggatacagagaggacgataaaggcaagccagatctgcataccttcgagccctataggaaactgaagtttaatctggaaagcatcaacattgacgatctgtcccgcgaagtgatcgacaagctggctgatattctgactctgaacaccgagagagaaggaatcgaggacgcaattaagaggaatctgccaaaccagttcacagaggaacagatcagcgagatcatcaaggtgcggaagagccagtccactgctttcaataagggctggcactcttttagtgcaaaactgatgaacgagctgatccccgaactgtacgccacctccgacgagcagatgacaattctgactcggctggaaaaattcaaggtcaataagaaaagctccaaaaacacaaagactatcgacgagaaggaagtcactgatgagatctacaatcctgtggtcgccaagagcgtgagacagaccatcaaaatcattaacgctgcagtcaagaaatatggcgacttcgataagatcgtgattgaaatgccacgggataaaaatgctgacgatgagaagaagttcatcgacaagagaaataaggagaacaagaaggaaaaggacgatgccctgaaaagggccgcttacctgtataattctagtgacaagctgcccgatgaggtgttccacggcaacaagcagctggaaaccaaaatccgactgtggtatcagcagggggagcggtgcctgtatagtggaaagcccatctcaattcaggagctggtgcataactctaacaatttcgaaatcgatcacattctgcctctgtcactgagctttgacgatagtctggccaataaggtgctggtctacgcttggacaaaccaggagaaaggccagaaaaccccttatcaggtcatcgactccatggatgcagcctggtctttcagggagatgaaggactacgtgctgaaacagaagggactgggcaagaaaaagcgcgactatctgctgactaccgagaacatcgataagattgaagtgaagaagaagttcatcgagaggaatctggtggatactcgctacgcatctcgagtggtcctgaactctctgcagagtgccctgagagagctggggaaagacactaaggtgtctgtggtcaggggacagttcaccagtcagctgcggagaaaatggaagatcgataagagccgcgagacataccaccatcacgcagtggacgccctgatcattgctgcatcaagccagctgaaactgtgggagaagcaggacaatcccatgtttgtggattatggcaagaaccaggtggtcgacaaacagactggggagatcctgtccgtgtctgacgatgagtacaaggaactggtgttccagcccccttatcagggctttgtgaataccatctcctctaaagggttcgaggacgaaattctgtttagctaccaggtggattccaaatataaccggaaggtcagtgacgcaaccatctactcaacaagaaaagccaagattggcaaggataagaaagaggaaacctacgtgctgggaaaaatcaaggacatctactcccagaatggcttcgataccttcatcaagaagtacaacaaagataagactcagttcctgatgtatcagaaggactctctgacatgggagaacgtgatcgaagtcattctgagggactacccaacaactaagaaaagcgaggacggcaaaaatgatgtgaagtgcaacccctttgaggaatacaggcgcgagaatgggctgatctgtaagtattccaagaaagggaaaggaactcccatcaagagcctgaagtactatgacaagaaactggggaactgcatcgatattaccccagaggaatcacgcaataaggtcatcctgcagagcattaacccttggcgagccgacgtgtacttcaatccagagacactgaagtacgaactgatgggcctgaaatattcagatctgagctttgaaaagggcactgggaactaccatatcagccaggagaaatatgacgctatcaaagagaaggaaggaattggcaagaaatccgagttcaagtttacactgtaccgcaacgacctgatcctgatcaaggatatcgccagtggcgagcaggaaatctacagattcctgtcaagaactatgcccaatgtgaaccactacgtcgagctgaagccttacgacaaggaaaagttcgataacgtgcaggagctggtcgaagcactgggagaggcagataaagtgggacgatgtatcaaaggactgaataagccaaacatcagcatctacaaggtgagaaccgacgtcctgggaaacaaatatttcgtgaagaaaaagggcgacaaacccaagctggattttaagaacaacaagaagtaagaattc

SEQ ID NO: 126 - DNA, 3462 bp, synthetic construct
  misc_feature 1..3462: note = source = /note="Description of Artificial Sequence: Synthetic polynucleotide"
  source 1..3462: mol_type = other DNA
accggtgccaccatgtacccatacgatgttccagattacgcttcgccgaagaaaaagcgcaaggtcgaagcgtccatggccgaccgaatctctctggggctggacattggggtggcaagcgtggggttctcagtgctggacattgataagggaaaagtcattgagctgggcgccaggctgttctctgctactgtggccgctggcaaccaggatcgaagagacatgcgaggagccaggcgcctgctgaaccggaacaagcagcgacggcaggataccggaaagctgttcaagaaatttggcctgatcgacgattttgataagggcagcttctacgacaactttaatcagaacctgaatccttatgagctgagagtgaaaggcctgacagaacagctgactaaggaggaactggccgagtctctgtaccagatcgtgaaacatagggggattagttatgcactgaaggacgccgatgtggacgaaggcgggacagactactcagtcagcctgaaaatcaacagccaggagctggcagaaaagactccagcccagattcagctgcagagactgaatgattatggaaaggtgaggggccaggtggtcatcggcgacgatccagacaaccagaaggtgctgctgaatgtgttccccacatcagcttacgagaaagaagcaaagcagatcattgccactcagcagcagttctatcctgagagcctgaccgacaagttcaccgaggaatactgccagatcctgactcgcaagcgagattattttgtggggccaggaaacgagaaaagccggaccgactacgggatctacaagactgatggaagaaccctggacaatctgttcgaggaactgatcggccacgataagatctaccccgaggaactgcgggcatctgcagccagttataccgcccagctgtttaacgtgctgaatgacctgaacaatctgagaatcctgaactacgaggatgggaaactgacaaaggaggacaaggaaaagatcatcgctgaaattaagaacaacaccacaactatcaacatgctgaatgtgattaagaaagtcgccgggtgttccaaggacgatatcaaaggattccgagtgaatgagaaggataaacccgaaatcagctccatgcctgtgtaccgcaaaattcataaggacctgctgaaggccggcgtggatatctcagactggcccgtcgagttcatcgacgaactgagctttattctgacactgaacactgagaatggggaaattcgcaaacagctgaacaatcgactggcccctaagttcgattttctgaacgctgacctgatccagctgatcattgataataaggactcctttgagattaagactaacaacaagtggcacagattcagcgtgaaaaccatgaacaaactgatcccagagatgatggaaagacccgtggagcagatgaccctgctgaatgaaatgggactggtcaagaaagataagaaacgctttgagaacaataagtacctgccttacaaggaaatcgcaaaggacattttcaacccagtggcctccaaatctgtccgcgaggccctgaagatcgtgaatgctgtcctgaagaaatacggccacattgattatctggtggtcgaaatgcctcgggataaaaacctgaaggaggaacaggacaatatcaaggagttccagaacaaaaataagaaagctaaggacgctgcattcgaagcatttgtgaaatcagtcgggagcgagcagagagtgaaggaagccctgtctaaaaaccggaagctgcagatgaagatgagactgtggtatcagcagcaggagatcgatccatataatggaaagacaatcgatgccactgacctgattaacaatcctgataagttcgagattgaccatatcattccacagagtatctcattttacgacagtattaacaataagaccctgtgcttcgcctcaatgaaccaggtgaaaggacagaaaaccccctacgagtttatgctggaaggccacgggcagtcctatgacaagttcaaagctacagtgatggcaaacaagaattttggcaaggctaaaagggcaaactacctgttcgaggaaaatgtgagcgatatcgagactcggaagagattcctgtcccgcaacctggtggacacccgatattctagtcgggtggtgctgaacagcctgcaggatttctttcgggagaaatctgccgacaccaaggtgacagtcattcgcggcaagtttacctccaacatgcgaaaacattggcacatcgataagactagggagacattccaccatcacgccattgacgcttctatcattgccgctacaccatttctgcgcatgtggaagaaaggaggcactatcttccccgtgaaggtcggagaagaaagtatcgatattgagacaggcgaaattctggacgataagaattttgacaaagcaatgtacgaggaaccctatagtggcttcgtgtcagagatcatgaacgccgacgatcggatcaagttcagccaccaggtggataagaaaatgaataggaaggtgagcgacgccaccatctacagtactcgcaccgggaaactggctaaggataagaaagacgctgagtacatcgtggcaaaggtcaaagatatctacagcgtggacggattcaagaagttcaagaaagtctacgataaggacaaaaccaagtttctgctgtacaaatatgatcctaggacattctcaaagctggagcgcatcattagcgattgcccagacaaagtggaaaaggtccagacaaacggcaaagtgaaggctgtcgatatcagtccattcgagatgtacagaagggaccatgggatgatcaagaaatactcaaagaaaggaaacggccccgccatcaagcagctgaagtacctggataagaaactgggcagccacatcgacattacccccgcaaacgccaatggaaaacacgtgatcctgcagagtctgaagccttggagaaccgacgtctatctgaaccacgagacaggcgagtacgaaatcatggggattaagtatagcgatctgaagttcaacaagaatgaggggtacggaatcaagaaagacaagtatctggaaattaagaaagtggaggaagtctccgagaagtctgagttcatgtttagcctgtacaggaaggatcgcgtgaaagtccaggacatgaaaaccggcgagtccgtggaactgctgttctggagcaggaacttttccaataagaaatacgctgagctgaagcccatctcccaggcagaaaacgacaagaaactgcctgtgtatggcaaagggagactgatcaagaggctgattcccaaaaactgtaagatctggaaagtgaataccacaattctgggcgatccctactatctggagaaagaaagcgactcccctaaggatatcctggactaagaattc

SEQ ID NO: 127 - DNA, 4611 bp, synthetic construct
  misc_feature 1..4611: note = source = /note="Description of Artificial Sequence: Synthetic polynucleotide"
  source 1..4611: mol_type = other DNA
accggtgccaccatgtacccatacgatgttccagattacgcttcgccgaagaaaaagcgcaaggtcgaagcgtccatgaagaaaacactgggactggacctggggactaacagcattgggtgggccgtcatcaactcaaacatcgactcagaaggaaaagaaaagctggtggggatcagctcctgcggaagccggatcattcctatggacgctaccacactgggagatttcggaaagggcaacactaaaagtccagtggcagagcgaacccgactgcggggcattcggagactgctggaaaggtcactgctgaggcgcgagcgactgcaccgagtgctgtcagtcatggggttcctgccagagcattacgctagccagctggaccgctatggaaagtttctgccagaaaccgagcccaagctggcatggtacaaagacgatagcggcaggtatcagttcctgtttcagaagtccttccacgagatgctggaggactttcgacagcatcagccagaactggtggcaggagagaagaaaatcccttacgattggacaatctactatctgcggaagaaagcactgtctcaggagatcactaaggaggaactggcctggattctgctgaatttcaaccagaaacgcggctactatcagctgcgaggggaggaagagcaggaagagaacaataagagcgtggagtatcacgccctgaaagtggtgagcgtcgaggactctggagaaagaaagggcaaagatatctggtacaatgtgactctggagaacggatgggtctatcgacgggctagcaacattcccctggactggaccggcaaggtgaaagagttcgtggtcactaccgagctggacgatgccgggaacccaaagaaagataaggaaggaaatgtgaaaagatcctttagggcaccaaaggaggacgattgggggctgctgaaaactaggacccaggctcagatcgacgaatccggcaagaccgtgggaacttacatctacgagtctctgctgtgtatgcccaaccagaagatccggggaaaactggtgaggaccattgaacgcaagtactataaagacgagctgagacagatcctggtgaagcagagcgagttccacgccgctctgcaggatcataatctgctgctgtcctgtatcgaagagctgtaccctaacaatgaggcccacagaaggctgctgagcgccagcagcttcatctacttcctgatcgaggacattctgttttatcagcgcccactgaagtcccagaaagggctgatcgataactgcccctacgagtctcacatctacaaggataagaaagatggaagtctgcaccatgtgcctctgaagtgtgtcagcaaatcccatccactgttccaggaatttcgcctgtggcagttcctgtctaacctgcgaatctaccagagagagaggatgatggacggcagtctgaaactggacgtggatgtcacccgggagttcctgccctcagaagaggactacgtgaagctgtttgattggctgaatgagagaaaggaaatctctcagaaattcctgctggcttataaaccttttgggctgaagaaaaacgaacaggcaaattacagatggaactatgtggaggacaagagctacccctgcaacgagacacgggcagaaatcaagagcagactgtccaaagccggagtgcctgaagagtttctgactgaagagaaggaagaggccctgtggcacatcctgtattctattagtgataagaaagagctgactaaggctctgggcaccttcgcagccaaaaactgtctgaatgagtctttcgtggaagtctttgccaagatccccccttttgagtcaaactacgctgcatatagcctgaaggctattaggaaactgctggcactgatgcgcatggggaagtactggaatgaacaggccatcgacaggcagactcgcgatcgaatcgagaaaattctgaccggagagtatgacgaaacaatccggagcagagtgagggagaaggcaatgctgctgaccgatattagcagcttccggggcctgcctctgtggctggcctgttacatcgtgtatgaccgccactcagagagcaaggaactggtcaaatgggagacaccagccgacatcgatcatttcctgtccaagtttaaacagaacagcctgcggaaccccatcgtggaacaggtcattacagagtccctgcgcactgtgcgagacatttggaagcaggagggaaaaatcgatgagattcacgtggaactgggccgggagatgaagaaccctgcaaaagagcgcgcccgaattacagctcaggtgcaggaaaatgagaacactaatctgagaatcaaggctctgctggcagagttcatgaaccccgaatttgagattgaaaatgtgcatccatactcacccggccagcaggaaatcctgcggatctacgaggacggcgtgctgagcgggatcgctgagaaggatctgcctgacgatatcacagcaattctgaagaaattccgagaaaacgacgtgaagaaacggccaacaactagcgaagtcctgcggtacaaactgtggctggagcagcggtacagatccccatataccggaagagtgatccccctgggcaagctgttcacacctgcttacgagatcgaacacgtgattccccagagccggtattttgacgattccatctctaacaaagtgatctgcgaaagtgccgtcaataagctgaaagataactgtctgggctatgagttcatcaagaaacattccggggagatggtggaactggggaatggagagacagtgcccgtgttcagcgtggaagagtacgaacggttcgtcaaggagtcttacttcggcaacagtaagaaaatgaagaaactgctgctggaggacatcccagatagcttcattgagagacagctgaatgacagtcgatacatctcacgggtggtcacatctctgctgagtaacctggtgtgcgaagagggagagcaggatggcctgtccaagaatgtgatcgtctgtaccggcgggattacagacaggctgaagaaagattggggagtgcaggaagtctggaaccgcatcattctgcctcggttcctgagactgaatgagatcaccggacggacagactttacaagtacttcagtgaacggccacctgctgcctgccctgccactgtacctgcagaagggctttaataagaaaagaattgaccataggcaccatgccatggatgctatcgtgattgcctgcgctaaccggaatatcgtcaactacctgaacaattcctctgctagaaagaacagcgaaattagccgatatgacctgcagcggctgctgtgtgagaaggtgaaaaccgatgccaacggcaattacaagtggatcctgaggaaaccatgggagacattcacccaggatgtgtatgccgctctgacaaacatcgtggtcagctttaagcagaatctgcgcgtgattaatcgaaccacaaactactatcagcactacaacgaggcaggggaaaagcgcatgatccctcagaccaaaggcgacagatgggccattagaaagccaatgcataaagatactgtgtatggcgaagtcaatctgagaaaggagaaaaccctgccactgagggacgtggtcaagaaccccagtatcgtggtcgataaatcactgaagaacaagctgtacgagctgctgaagagccagtatgacctgaaggcaatcgccaaatacttcgagacacaccaggacgtgtgggcagatgtcaacctgaagaaaattaaggtgtactacttcactaaggagacaaacgaaagattctttgccactaggaagagcctggacccatcctttgatcagaagaaaatcgaagaggaagtgactgataccggcgtccagaagattctgctgcaccatctgcagcagaacaataacgaccctgatatggccttttccccagacggcatcgataggatgaaccagaatatgaccattctgaatgacgggaagtggcaccagcccatctacaaagtgcgcacatatgaaaaggcagataaattcgccgtcggcgagtctgggaacaaggccaagaaatttgtggaagcagccaaaggcaccaatctgttctttgccgtgtacgagagtgtccaggaggacgaagctatcgggaagcaggtctgcaaacggacattcgccactatccccctgaacgaagtgatcaagagaaagaaacagggcctgcccgctgcacctgaggacctgaacgggaatctgcccaagtttgtgctgagccctaacgatctggtctacctgcccaccgaggaagagaggaatagttcacgcatcattcagcctctggacagggagcgcatctataagatggtgagctcctctgggagtcagtgcttctttatcaaagtgttcgtcgccaattcaatttgggataagaacgaatacagcagcctgaacaagatggagagggctattacaaacgaaatgatcaaggagatttgtgtgcctatcaaaattgaccgcctgggcaatgtcagcctgatccagatttaagaattc

SEQ ID NO: 128 - DNA, 4458 bp, synthetic construct
  misc_feature 1..4458: note = source = /note="Description of Artificial Sequence: Synthetic polynucleotide"
  source 1..4458: mol_type = other DNA
accggtgccaccatgtacccatacgatgttccagattacgcttcgccgaagaaaaagcgcaaggtcgaagcgtccatgacaaagactattctgggactggatctggggactaacagcattggatgggcactgattaaccaggacttcgataacaaaaagggggagatcctgggcatgggcagccggatcattcctatgacacaggatattaaggacgagttcggaaaaggcaactctatcagtcagacagctgagcgaactcgactgcggggagtccggagactgatccacagaactctgctgaggcgcgagcggctgcatagagtgctgaatatcattggcttcctgccagaacactatgccaaccagattgactttgagaagaggttcggcaagttcaagcctgaatctgagccaaaaatcagtttcgatggaaatgacgtgttcctgtttgagaagagctaccaggaaatgctggtcgactttaaaatccaccagccacagctggtgagcaacggcaagaaaattccccatgactggacaatctactatctgagaaagaaagctctgtctaagaaaattgagaaggaggaactggcatggatcctgctgaacttcaatcagaaacggggatactatcagctgagaggcgaggaagaggaagagacaccaaataagctggtggagtttcatagcctgaaaattgtggaggtcaacgccgatgaaccccagaaaggaaagcctgagatctggtactcactggtgctggaaaacggctgggtctatcgacgggctagcaagactcccctgttcgattggaaagacaagattagggagtttatcgtgaccacagaaatcaacaatgatggaactgtcaaaaccgacaaggagggcaccgaaaagaggagcttccgcgcaccaaaacccgaggactggactctgcagaagaaaaagaccgagttcgagctgtcaaagagcgggaatgaagtgggagccttcatctacgaaagtatcctgcagaaacccaaccagaagattagaggcaaactgatttcaaccatcgagaggaaattttataaggaagagctgaaaaccatcctgaaaacacagctgttctttcacaaagaactgaaggatgagaaactgtacaatgcctgcatcgaagagctgtataagaacaatgaagctcaccggagcctgctgtccaacaaggggttcgagcatctgtttattaacgacatcctgttctaccagcgacctctgcggtctaaaaagagtcagatctcaaactgcccactggagaagcgcacatataaaaaggaggggattgaaatcactgagggcatcaaagtgatctccaaatctaatccaatctaccaggagttccggctgtggcagtggattagcaacctgtccctgtattgtatcgaacccaccgagacaaatgtgacttcaacctttctgaacagcattgaagattacgagaatctgttcgaatttctgaacaatcgcaaggaaatcgagcagaagcacctgctgaaatatctgctggagaaccaggggtttaaaggaaagctgctgacaaacgaactggagaagttccgctggaattttgtcgctgacaaaaagtacccctgtaatgagacaggcagcctgctgcatactcggctgagcaaagtgaagaacatttcccctgatttcctgaccaaggaaatcgagcaccagctgtggcatatcatctacagcgtgaccgacaagattgaatatgagcaggccctgaaaacctttgctcggaaaaacaatctggatgtggactccttctttgagcacttcaaaaagatccccccttttgagtctacctacggagcatatagtgaaaaggccatcaagaagctgctgccactgatcagactgggcaaatactggaactgggaggccattgatagtatctcaaaggacaggattagtaaaatcctgtcaggggaatacgatgagaacattaagaacagagtgagggagaaagcagtccacctgacctccgaaaacaatttccagggactgcaggagtggctggccaagtacatcgtctatgatcgccattctgagggcaatgacctggggaagtggactagcgtgtccgacctggagacatacctgaaggagttcaagcagcatagcctgcggaaccctattgtggagcaggtcatcacagaaactctgagagtggtcaaggatatttggatcaagcacgggaaaggaaccgaaaatttctttgacgaaatccatgtggagctgggccgggaaatgaagaacaattccgaggatcgcaaacgactgaccaacacaattactgaaaacgagaatacaaacctgagaatcaaggccctgctgatggaaatgatgaatgataacgacgtggagaacgtcaggccttactctccaagtcagcaggagattctgaagatctatgaggacggagctctgaatagcaacatcgagctggacgatgaaattgtgaagatctccaaaaaggcagagcccaccaaatctgaactgcagcgctacaagctgtggctggagcagaaataccgatccccttatactggccaggtcatcccactgaacaagctgttcacctctgaatatgagatcgaacacgtggtccctcagagtcgcttctttgacgatagcttcagcaacaaagtgatctgcgagtcagccgtcaacaagcggaaggataaccagctggggctgcagttcatcaagaaccatagcggagaaaaagtggagctgggcttcgggaaggtggtccaggtctttacagaagagcagtacctggattttgtgaaggagcactatagcaaaaatcgctccaagcataacaaactgctgctggaagagattcccgagaagatgatcgaaaggcagctgaatgacactcgctacatcagtaagttcgtgagctccattctgtccaacatcgtcagatctgagaaggacgatgacggcctgaatagcaaaaacattctgcctggaaatggcaagatcactaccgaactgaaaagggactgggggctgaatgatgtgtggaacgacctgattctgccaagattcgagaggatgaataccatcacaaacagcgatctgtttacaacttacaacgacaagtatcagaaacacctgcccaccgtgcctttcgagtactccaagggctttcagaaaaagcgcattgatcaccgacaccatgctatggacgcactggtcatcgcatgtgccacacgggatcatctgaatctgatgaacaatcagtctgccaagagtgaactgaaacgatacgacctgcagaacaagctgcggaaaaaggagccttacttcaaccagaaggagaacaaacagaaggaagccttcaaggattttatcaaaccatggggcactttcaccgaggacagcaagaatgctctggaaaaaatcattatctcctttaagcagaacctgagagtgatcaacaaggcaacaaactcatacgagagctataaggatgaggacgggaatctgaggatcggcaaggatgggaaaccagagaagggcctgatcaagcagaaggggctgaactgggcaatcagaaagcccctgcacaaagacaccgtgtcaggccagattaacctgagcaggatcaagctgcccaatgggaaaatcctgacagccactcgcaagaatctggataccagtttcgacctgaaaacaattgagaactcaatcaccgacacaggcattcagaaaatcctgaagaattacctgctgtccaaggaatctccagagctggccttctctcccgagggcctggaagagatgaacaatgagatcgaaaagtacaacaatgggaaatttcaccatcctattaacaaggctaggatctatgaactggggagcaaattcaatgtcggacagacaggcaacagaagggataagtttgtggaggccgctaaaggaactaatctgttctttgctatctaccaggacgagaataagaaccgctcttatgaaactattcccctgaacgaagtgatcgagcaccagaagtggcgagcaagtctgcctaaggaagagcaggagaaaattccactggtgcccgtcaacaagctgaaggggaccttcatcttttccctgtctcccaacgatctggtgtacgtcccttccaatgacgagctggaacgaagtgcttcaattgacttctctaagctgaaaaaggaacagatcaaccggctgtataaaatggtgtctagttcaggatcccagtgcttctttgtgaagagtgaggtcgcaacctcagtggtcaacaaaatggaatacagcagcctgaacaagatggagaagtctatcgataacctgatggtgaaggagatttgtatcaaactgaagattgacaggctgggcaacatcagcaaggcctaagaattc

SEQ ID NO: 129 - DNA, 4689 bp, synthetic construct
  misc_feature 1..4689: note = source = /note="Description of Artificial Sequence: Synthetic polynucleotide"
  source 1..4689: mol_type = other DNA
accggtgccaccatgtacccatacgatgttccagattacgcttcgccgaagaaaaagcgcaaggtcgaagcgtccatgaccaaaatcctggggctggacctggggactaatagcatcgggtgggcaatccgcgacacagaaaatgagggcatcaatcagatcctggacaagggcgcccgcattttcagcgagggagtgaagtccgagaatggcaaagaaatcagtagggcagctgaacgaaccgcttaccggagcgcaagaaagatcaaatatcggagaaaactgcggaagtacgagacactgaaggtgctgtcaattaacggaatgtgccccctgagcgtggaggaagtcgaacagtggaagaaatctggcttcaaggaatatcccctgaatcctgagtttctggattggctgcggaccaacgaggacaagaacatcaatccttacctgttcagagataaagctagcaagcagaaagtgacactgtttgaactgggaagagctctgtatcacatcgcacagaggcgcggcttcctgagtaacaggctggaccagtcagccgagggcgtctttgaggaacataatcctcagatccagaacctgattgaggacctggacagctccaacacaattctgaatgagctgaaggaatactatatcaatctggggatcattgacgagactgaaaagtccggcttcaagaaagacctggatgagggggaaaagaaactgaagtcactgtacaacagcctggtggccatcacaaagaaaaacgctaacgatatcgaaacttgcaagcaggagctgatcgctagactgaataagaaagaggacctgggcaaggtcaaagggaagatcaaagatatttctcaggcaatgctggacaggaactttaagactctgggacagtatttcttttcactgtacaacaaggagcgaatccggaaccagtataccagccgcgaggaacactacctggaggagttcatcattatctgtcagacccaggggatcgagggaattaacacaaatgagaagctgcctgagaagaagttcaccggcctggcaaaagatctgtatcgagccattttctttcagcggccactgaaatcccagaagggcctgatcgggaagtgctctttcgagaagaacaagtctcgctgtgccgtgagtcacccagactatgaggaatttcgaatgtggagctacctgaacacaatcaaaattggcactcagtccgagaaaaccctgcgcttcctgacactggaggaaaagctgaaactggtgcccaagttctaccgaaagagtgatttcaacttcgaggtgctggctaaggagctggtcgaaaaaggagcatcattcggctactacaagtctagtaagaaaaatgagttcttttactggttcaactataagcccaccgattcagtgagcgcctgcgtggtgagcgcttctctggagaacgcaatcggcaaggactggaagatcaagactttcgaatatcagactagaaacaccgagaagaatgaagtgaccaaatccgtcgattacaaggacctgtggcacctgctgtccgtggcaacatctgatacttacctgtatgactttgccatcgaaaagctgaaactggagcctaaaaacgcaaaggccttcagcaagacaaaactgaagaaagactttgccagtctgtcactggcagccatcgctaaaattctgccatatctgaagcagggcctgctgtactcccacgccgtgttcatggctaacatcgagaatattgtcgacgccgatatctggaaggatgaggaacagcagaagttcatccagtccaagattgtggagctggtcgacaattatatcgtggaaaagtctaaactggagctgatcaatgggctgctgaagatctacaacaccgaggataaggaaggacggaaagtgtactattcaaaggaggctgaaagcctgttcgaggcagacctgagaaagaaactggtccccttctacaaggctaacatcatcatcgaggaacacgagcaggaaatcattttccaggatctgtttcctatcctgatggaccagctgaagaaacaggagttcatcaaaattggcagactggataagcagattgaagccttcctggagggggaaaatgaggaaggacagatcttttgtaaccacacagataagctgaagaaactgtaccatccaagcgacatcgaggtgtttaagaaaaagactatcaaagatgagtgggggaatgaaaaggtggtcctgggatccccactgaccacatctatcaagaaccccatggcaatgagagccctgcaccagctgaggaaggtgctgaatacactgattgccaacgaccagatcgacgaggatactcggatccatattgagatggccagagaactgaacgatgctaataagcgaaaaggcatccaggacttccagaacgagaacaagaagtttcgggaggaagccatcaaggagatcaagaagctgtacctggaggaatgccacaaagacgtgaaccccaccgaggacgatatcctgaggtatcagctgtggctggaacagggaaagtgcgagatctacgaggaaggcaacaatatcagcatttgtgatatcattggcagcaatccctcctatgacatcgagcataccattcctcggagcatctcccaggataacagccagatgaacaagacactgtgtagcctgaagttcaacagatccatcaaaaagcagaagatgccagtggagctgtccaactacaatgacattctgcccaggatcgcacactggaaaaaggaggccgaggaactgactaggcagatcgaaaccatttctcgcagcatcaagagcgctgcaaccaaggtggccaaggataagaacatcagaaagaggcattacctgacactgaagcgagactatattctggggaaatacgagcggttcacttgggaggaacctaaagtgggctttaaaaactcccagatcccagacactgggatcattaccaagtacgctcaggcatatctgaaatcttacttcaaaagggtggagagtgtcaagggaggagcagtggctgagttccggaaactgtggggcatccaggaatcttttatcgatgagaactggtggaagcactataaggacaaagatagagacaaacatacccaccatacaatcgacgcaatcactattgcctgtatgcccaaggataaatacgacctgctggcacacgcctggaggctggaggatgaacaggacaaaaaggccgctaaggtgctgatcgagcaggccaaaccatggaaaaccttcaaggaggatatcgaaaagattgagactgaaatcctggtgagccattttacccccgacaacgtcaaaaagcagtcaaagagcatcatcaagaatcgcggcaaaaaggtgtacgtcctgaagaacgagctgcctgtgaacttcaagaacaagatcgaagggaaggattatttcaagctgaaatttgacagcaagattctgtacaaaatccccaaaaagaaagagaagcagaccgatacattctatgaggaactgcctaaaaactacctgaatggagtggaaggcaaggactacttcaaaatcaatactaccggcaagaccttctacaaaatcccaatttttaaccagggcgacacaatccgggggagcctgcaccaggagacaacttacggagccattaagctgccagatatcgacattgaaacaaagaaacccctgcatactgataagggaggcttcattctgaagaaagacatcaaaggcaatgagattgtgttctttgtggtccgcaaggaaatctctaaaattagtgagaacgatgtgcagaatatcgtcgacaacgtggtccggaagaaaattgagaatgctatcgcaaactccctgatcacttttaagatcgtgaagaaaaagaaagtggccgtcatcaaagagggggtcaccatttggatgagggagcccaacattgaaaaggggatcgagggaatccctattaagaaagtgcgcatcattaccaattctgtcaaaaaccctatcgagattaaggtgcacagtccactgtccaagtctcgccacaagcataaacagaaggtctacggccagaacgatgagaattatgccatggctctgtacgaactggacgggaagcgggagttcgaactgatcaacaattttaatctggccaagctgctgaaacagagtcagtcatactatccactgcataaagagaaggaaatcaagggaaagaaaattctggtgcccatcgagaagagaaacaacaaggatgtcatcctgaagaggggccagcaggtggtgttctacgacaaaaccgtggagaaccccaaggatatctctgaaatcattgactttcgcgagcgaatctacatcattgaagggctgaccatccagagacagaaagataagaaaacatccaaagtgaatgagtacggaatcattcagctgcgccacttcaaggaagctcgaaaaagtgaggaaatctcaaaggataacttcaaacctgacggcgagttcaagatcaacgagaataagccaactaggaaaatgaaccataatcagttcaccgcctttgtggaggggatcgacttcaaggtcctgcctagcggaaagtttcagaaaatttaagaattc

SEQ ID NO: 130 - DNA, 3621 bp, synthetic construct
  misc_feature 1..3621: note = source = /note="Description of Artificial Sequence: Synthetic polynucleotide"
  source 1..3621: mol_type = other DNA
accggtgccaccatgtacccatacgatgttccagattacgcttcgccgaagaaaaagcgcaaggtcgaagcgtccatgagcaagaaagtcagtagacgctatgaagaacaggcacaggagatttgtcagaggctggggagtagaccttattccatcgggctggacctgggagtgggatctatcggagtggcagtcgccgcttacgacccaattaagaaacagccctccgatctggtgttcgtcagctccaggatttttatcccttctaccggcgcagccgagcggagacagaagagaggacagaggaacagcctgcgccaccgagcaaatcgcctgaaattcctgtggaagctgctggctgaacgaaacctgatgctgtcatatagcgagcaggacgtgccagatcctgcacggctgagatttgaggacgctgtggtccgagcaaacccatacgagctgcggctgaagggcctgaatgaacagctgaccctgagcgagctggggtatgcactgtaccacatcgccaatcataggggatctagttcagtgcgcacattcctggatgaggaaaagagctccgacgataagaaactggaggaacagcaggctatgacagaacagctggcaaaagagaagggaatttccactttcatcgaagtgctgacagcctttaacactaatggcctgatcgggtacaggaactccgagtctgtgaagagtaagggcgtgccagtccccactcgcgacatcatttcaaatgagattgatgtgctgctgcagacccagaagcagttctatcaggaaatcctgtcagacgagtactgcgatcggattgtcagcgcaatcctgtttgaaaacgagaagatcgtgccagaagccggctgctgtccctatttccctgacgagaagaaactgcccagatgtcactttctgaatgaggaaaggcgcctgtgggaagccattaacaatgctaggatcaagatgcccatgcaggagggcgctgcaaaacgctaccagagtgcttcattcagcgacgagcagagacacattctgtttcatatcgcaaggagcgggactgatatcacccctaaactggtgcagaaggagttcccagccctgaaaacctccatcattgtgctgcagggaaaagagaaggctattcagaagatcgcaggcttccgatttcgacggctggaggaaaaatctttttggaagagactgagtgaggaacagaaggacgatttctttagcgcctggacaaacactcctgacgataaaagactgtccaagtacctgatgaaacacctgctgctgacagaaaatgaggtggtcgacgccctgaaaaccgtgagcctgattggagattatggcccaatcggcaagaccgcaacacagctgctgatgaaacatctggaggatggcctgacttacaccgaagccctggagcggggaatggaaaccggcgagttccaggaactgtcagtgtgggagcagcagagcctgctgccctactatgggcagatcctgacaggatctactcaggccctgatggggaagtattggcactctgcttttaaagaaaagagagacagtgagggattctttaagcctaacacaaatagcgatgaggaaaaatacggcaggattgccaacccagtggtccatcagactctgaacgaactgcgcaagctgatgaatgagctgattaccatcctgggagctaaacctcaggagatcacagtggaactggcacgagagctgaaggtcggagctgagaaaagagaggacatcattaagcagcagaccaaacaggaaaaggaggctgtgctggcatatagcaagtactgcgagcccaacaatctggacaaaaggtatattgaaaggttccgcctgctggaggatcaggcctttgtgtgcccttactgtctggagcacattagcgtcgcagatatcgcagctggaagggcagacgtggatcatatcttcccacgcgacgatacagctgacaactcctacgggaataaggtggtcgcacaccgacagtgtaacgatatcaagggaaagcggaccccctatgcagccttcagtaatacatcagcctggggccccatcatgcattacctggacgaaacccctgggatgtggcgcaaaagaaggaagtttgagacaaacgaggaagagtatgctaagtacctgcagtcaaaaggcttcgtgagcaggtttgaaagcgataactcctatatcgcaaaagctgcaaaggagtacctgcgctgcctgttcaatccaaacaatgtgactgccgtcgggtccctgaagggaatggagacatctatcctgcggaaggcctggaatctgcagggaattgacgatctgctgggcagccggcactggagtaaggacgccgataccagccccacaatgcgcaaaaaccgggacgacaatcggcaccatggcctggacgccatcgtggctctgtattgttccagatctctggtccagatgattaacaccatgtccgagcagggcaagcgagcagtggaaatcgaggctatgattcctatcccagggtacgcatccgaaccaaatctgtctttcgaagcccagcgggagctgtttagaaagaaaatcctggagttcatggacctgcacgcctttgtgagtatgaaaaccgacaacgatgcaaatggcgccctgctgaaagatactgtgtattcaattctgggagcagacacccagggagaggatctggtgttcgtggtcaagaaaaagattaaggacatcggcgtgaaaatcggggattatgaagaggtcgcatctgccattcgaggccggatcaccgacaaacagccaaagtggtatcccatggaaatgaaagataagatcgagcagctgcagtctaagaacgaagccgctctgcagaaatacaaggagagtctggtgcaggcagccgctgtcctggaagagagtaataggaagctgattgagtcaggcaaaaagcccatccagctgagtgaaaaaacaatttcaaaaaaggccctggagctggtgggcgggtactattacctgattagcaacaacaagcgcacaaagactttcgtggtcaaggaaccttcaaacgaggtgaaagggttcgcatttgacactggaagcaatctgtgcctggacttttatcacgatgcccagggaaagctgtgtggcgagatcattagaaaaatccaggctatgaacccttcctataagccagcatacatgaaacaggggtattctctgtacgtgagactgtaccagggcgacgtgtgcgagctgagggcaagcgatctgactgaagcagagtccaacctggccaagaccacacatgtccgcctgcccaatgctaaacctgggcgaaccttcgtgatcattatcacctttacagagatggggtctggatatcagatctacttcagcaacctggccaagtccaaaaagggacaggacactagttttaccctgactaccatcaagaattatgatgtgcggaaagtccagctgtctagtgccgggctggtgagatacgtcagccctctgctggtggacaaaatcgagaaggatgaagtcgctctgtgtggagagtaagaattc

SEQ ID NO: 131 - DNA, 3588 bp, synthetic construct
  misc_feature 1..3588: note = source = /note="Description of Artificial Sequence: Synthetic polynucleotide"
  source 1..3588: mol_type = other DNA
accggtgccaccatgtacccatacgatgttccagattacgcttcgccgaagaaaaagcgcaaggtcgaagcgtccatggcaagacctgcatttcgggcacctcggagagaacacgtcaacggctggacccctgacccacatcggattagcaaaccctttttcatcctggtgagctggcacctgctgtcccgggtggtcattgacagctcctctggatgcttcccaggcaccagccgggaccacaccgacaagtttgccgagtgggaatgtgctgtgcagccctacaggctgagtttcgacctggggaccaactcaatcggatggggcctgctgaatctggatcgccagggaaaaccaagggagatccgagcactggggtcccgcatcttcagcgacggacgggatccccaggacaaggcttctctggctgtggcacggagactggccagacagatgaggcgccgacgggacagatatctgactagaaggaccaggctgatgggagctctggtgcgcttcggcctgatgccagcagaccctgcagctaggaagcgcctggaagtggccgtcgatccatacctggcacgagagcgggccacaagagaaaggctggagcccttcgaaatcgggagggccctgtttcacctgaaccagcgccgaggatataaacccgtgcgcaccgccacaaagcctgatgaggaagccggcaaggtgaaagaggctgtcgaaaggctggaggcagcaatcgctgcagccggagcacctactctgggagcttggttcgcatggcgaaaaacacgaggagaaactctgcgagcacgactggctgggaagggaaaagaggctgcatacccattctatcccgcacggagaatgctggaggccgaatttgacactctgtgggcagagcaggccaggcaccatccagatctgctgaccgccgaagctcgcgagatcctgcggcacagaatttttcatcagcggcccctgaagccacctccagtgggaagatgcactctgtaccctgacgatgggagagctcctagggcactgccaagcgctcagaggctgcgcctgttccaggagctggccagcctgagagtgatccacctggacctgtccgaacgccctctgaccccagctgagcgagatcggattgtggcatttgtccagggcagaccccctaaagccggaaggaagcctggcaaagtgcagaagagcgtcccattcgaaaagctgagggggctgctggagctgccaccaggcactgggttttctctggagagtgacaaacggcctgaactgctgggcgacgagacaggcgccagaatcgcaccagcattcggacctggatggacagctctgcctctggaggaacaggacgccctggtggaactgctgctgacagaggcagaaccagagagggcaattgcagctctgactgcacgatgggctctggacgaggcaactgcagcaaagctggctggagcaaccctgccagattttcacggacgatatggcaggcgcgcagtggctgaactgctgcctgtcctggaacgcgagacacgaggcgacccagatgggagagtgaggcccatccggctggacgaggcagtgaaactgctgagaggcgggaaggatcactcagacttcagccgggaaggagctctgctggacgcactgccctactatggagccgtgctggagagacatgtcgcttttgggacaggaaaccccgcagatcctgaggaaaagcgggtgggaagagtcgccaatcccactgtgcacatcgctctgaaccagctgcggcatctggtgaatgcaattctggccaggcacggccgccctgaggaaatcgtgattgagctggcacgggacctgaaaaggtctgccgaagatcgacggagagaggacaagcggcaggccgataaccagaaaagaaatgaggaacgcaagcgactgatcctgagtctgggagagcgcccaaccccacgaaacctgctgaagctgcggctgtgggaggaacagggcccagtggaaaataggcgctgcccctactctggggagacaattagtatgagaatgctgctgagcgagcaggtggacatcgatcacattctgccattcagcgtgtccctggacgattccgctgcaaacaaggtggtctgtctgcgggaggccaacagaatcaagcggaatagatctccctgggaggccttcggccatgacagtgagagatgggcagggattctggcacgagcagaagctctgcccaagaacaaaaggtggcgctttgctcctgacgcactggagaaactggaaggagagggaggcctgcgagcacgacacctgaatgatacaaggcatctgagtcgcctggccgtggagtatctgcggtgcgtctgtcctaaggtgcgggtgagcccaggccgactgactgcactgctgcgacggagatggggcatcgacgccattctggcagaagcagatggacctccaccagaagtgcccgcagagacactggacccttccccagctgagaagaaccgagcagaccaccggcaccatgccctggatgctgtggtcatcggctgtattgatcgctcaatggtgcagcgagtccagctggccgctgcaagcgcagaaagagaggccgctgcaagggaggacaatatcaggcgcgtgctggagggattcaaagaggaaccttgggatggctttagagctgaactggagcgacgggcacggaccatcgtggtgagccacagaccagaacatgggattgggggagccctgcataaggagacagcttacgggcctgtggaccctccagaggaaggattcaacctggtggtcaggaaaccaatcgacggcctgtcaaaggatgagattaatagcgtgcgggacccccggctgagaagggcactgatcgatcgcctggccattcgccgacgggatgctaacgaccctgctaccgcactggccaaagcagctgaggatctggcagcacagccagcctcccgcggcatcagaagggtgcgggtcctgaagaaagaatctaaccccattagggtggagcacggcgggaatccaagtggaccccgctcaggaggcccttttcataagctgctgctggcaggagaggtgcaccatgtggacgtcgcactgcgagcagatggccgccgatgggtgggacactgggtcacactgttcgaggcacatgggggacggggagcagacggagctgcagccccacctagactgggcgatggggaaagatttctgatgaggctgcacaagggagactgcctgaaactggagcataagggcagagtgagggtcatgcaggtggtcaaactggaacctagttcaaatagcgtggtcgtggtcgagccacaccaggtgaaaaccgacagatccaaacatgtcaagatctcttgtgatcagctgcgcgctcgaggagcacggagagtgaccgtcgatccactgggacgggtgagagtccacgccccaggagctagggtgggaatcggaggggacgccggacgaaccgctatggaacccgcagaggatattagctaagaattc

SEQ ID NO: 132 - DNA, 3234 bp, synthetic construct
  misc_feature 1..3234: note = source = /note="Description of Artificial Sequence: Synthetic polynucleotide"
  source 1..3234: mol_type = other DNA
accggtgccaccatgtacccatacgatgttccagattacgcttcgccgaagaaaaagcgcaaggtcgaagcgtccatgggagagaatatgattgacgagagtctgaccttcggcattgacctggggattgggagttgtgggtgggcagtgctgaggcggccaagcgccttcggacggaagggcgtgatcgagggaatgggctcctggtgctttgacgtccccgagacatctaaagaacggactcctaccaaccagatccggagatccaatagactgctgaggcgcgtgatccgacggagaaggaaccggatggccgctattcgccgactgctgcacgcagcaggcctgctgccatcaaccgacagcgatgccctgaagcggcccggacatgatccttgggaactgagggcacgaggcctggacaagccactgaaacccgtggagttcgctgtggtcctgggccacatcgcaaagcggagagggtttaaatccgctgcaaagagaaaagccacaaacattagctccgacgataagaaaatgctgacagccctggaggctactcgagaacggctggggagatacaggaccgtgggagaaatgttcgccagggaccctgattttgcttctaggcgccgaaatcgcgagggcaagtatgataggaccacagctcgcgacgatctggagcacgaagtgcacgccctgttcgcagctcagcggagactgggacagggatttgccagtccagaactggaggaggccttcaccgcttcagcatttcatcagaggcccatgcaggacagcgagcgcctggtgggattctgcccttttgagcgaaccgaaaagcgggcagccaaactgacaccctctttcgagcgctttcgactgctggcccggctgctgaacctgagaatcactaccccagacggagagcggcccctgacagtggatgaaattgctctggtcacccgggacctgggcaagaccgcaaaactgagtatcaagcgggtgagaactctgattggactggaggacaatcagaggttcacaactatccgccccgaggacgaagatcgagacattgtggctcggacaggcggggcaatgacagggactgccaccctgaggaaggcactgggagaggccctgtggactgatatgcaggagcgccctgaacagctggacgctatcgtgcaggtcctgagcttctttgaggccaacgaaacaatcactgagaagctgagggaaattggcctgactctggccgtgctggacgtcctgctgaccgcactggatgccggagtgttcgccaagtttaaaggcgctgcacacatcagcaccaaagccgctaggaatctgctgccacatctggagcagggcaggcgctacgatgaggcctgcacaatggcagggtatgaccacgcagcctcccgcctgtctcaccatggccagatcgtggcaaagacacagttcaacgccctggtcactgagatcggcgaatccattgccaatccaatcgctcggaaggcactgatcgaggggctgaaacagatttgggccatgagaaaccactgggggctgcccggaagtatccatgtggagctggcccgggatgtcggcaactcaattgaaaagcgacgggagattgaaaagcacatcgagaaaaatactgccctgagggctcgcgagagaagggaggtgcatgatctgctggacctggaagatgtcaatggcgacaccctgctgcgataccggctgtggaaggagcagggaggcaaatgcctgtatacagggaaggccatccacattcggcagatcgctgcaactgacaactccgtgcaggtcgatcatattctgccttggagccggttcggcgacgatagttttaacaacaagaccctgtgtctggcctctgctaatcagcagaagaaaaggtcaacaccatacgagtggctgagcggccagactggggatgcatggaacgccttcgtgcagcgcatcgagacaaataaggaactgagagggtttaagaaaaggaactatctgctgaagaatgctaaagaggcagaggaaaaattcagaagcaggaacctgaatgacaccagatacgccgctaggctgttcgcagaggccgtgaagctgctgtatgcctttggggagagacaggaaaaagggggaaaccgccgagtgtttactcggcctggagcactgaccgcagcactgagacaggcttggggagtggagagcctgaagaaacaggatgggaagcgcatcaatgacgatcgacaccatgccctggatgctctgaccgtggctgcagtcgacgaggccgaaattcagaggctgacaaaatcattccacgagtgggaacagcagggcctggggcggcctctgcggagagtggagccaccttgggagagcttccgggcagacgtcgaggctacctaccctgaagtgtttgtcgcacggccagagaggcgccgagcaagaggagaaggccatgccgctaccatccggcaggtgaaggagagagaatgcacaccaattgtgtttgagagaaaggctgtctctagtctgaaagaggcagacctggaacgaatcaaagatggcgagcgcaacgaagcaattgtggaggccatcaggagctggattgccactggacgcccagctgatgcaccaccacgctccccccgaggcgacatcattaccaagatcaggctggccaccaccatcaaggcagccgtgcctgtccgcggagggaccgcaggaaggggagaaatggtgcgcgcagatgtgttcagcaagccaaaccggagagggaaagacgagtggtatctggtgcccgtgtatccacaccagatcatgaacaggaaggcttggcccaaacctccaatgcgctcaattgtggccaataaggatgaggacgaatggaccgaagtgggacctgaacaccagttccggtttagcctgtaccctagatccaatatcgagatcattaggccatctggagaagtgatcgaaggatatttcgtcggcctgcatcgcaacactggcgctctgaccatcagtgcacacaatgatcccaagagtatccattcaggcattgggaccaagacactgctggccatttccaaataccaggtggacagattcggcagaaagtctccagtgcgcaaagaggtccgaacttggcacggggaagcctgtatctctcccaccccccctggataagaattc

SEQ ID NO: 133 - DNA, 3504 bp, synthetic construct
  misc_feature 1..3504: note = source = /note="Description of Artificial Sequence: Synthetic polynucleotide"
  source 1..3504: mol_type = other DNA
accggtgccaccatgtacccatacgatgttccagattacgcttcgccgaagaaaaagcgcaaggtcgaagcgtccatgagagagaacgggagtgacgaaaggcggaggaatatggacgaaaaaatggattacaggattgggctggacatcggcatcgcatcagtggggtgggccgtcctgcagaacaattcagacgatgagcctgtgaggattgtcgacctgggagtgcgcattttcgataccgcagagatcccaaagacaggcgaaagcctggcaggaccccggagagcagctcgaaccacaaggcgccgactgcggagaaggaaacaccgcctggaccgaatcaagtggctgttcgagaaccaggggctgatcaatattgacgattttctgaagagatacaacatggccggactgccagatgtgtaccagctgcggtatgaggctctggacagaaaactgaccgatgaggaactggcccaggtgctgctgcacatcgctaagcatcggggcttcagaagcaccaggaaagccgagacagcagccaaggaaaacggggcagtgctgaaggccacagacgagaatcagaaacgaatgcaggaaaagggatacaggacagtgggcgagatgatctacctggacgaggccttccggactggctgctcttggagtgagaaagggtacatcctgaccccccgcaacaaggctgaaaattatcagcacacaatgctgcgggcaatgctggtggaggaagtcaaggagattttcagctcccagcgccgactgggcaacgaaaaagccactgaggaactggaggaaaagtacctggagatcatgacctcccagcgctcttttgacctggggcctggaatgcagccagatgggaagccctccccttatgcaatggagggcttctctgacagagtggggaaatgtacttttctgggggatcagggagagctgaggggcgctaaggggacctacacagccgaatatttcgtggctctgcagaaaatcaaccacacaaagctggtcaatcaggacggcgagacaaggaatttcactgaggaagagcggagagccctgactctgctgctgtttacccagaaagaggtgaagtacgctgcagtccgcaagaaactgggcctgcctgaggacatcctgttctacaacctgaactacaagaaggccgctactaaagaagagcagcagaaggagaaccagaataccgaaaaagccaagtttatcgggatgccatactatcacgattacaagaaatgcctggaagagagagtgaagtatctgaccgagaacgaagtcagggacctgtttgatgagatcggaatgattctgacttgttacaaaaatgacgattcccgcaccgaacgactggccaagctgggactggtgcccatcgagatggaaggcctgctggcttatactcctaccaaattccagcatctgtctatgaaggcaatgcggaacatcattccctttctggagaaagggatgacctacgacaaggcttgcgaagaggcaggatatgacttcaaagccgatagcaaggggactaaacagaagctgctgaccggagagaacgtgaatcagacaatcaacgaaattactaatcctgtggtcaaacgctcagtgagccagacagtgaaggtcattaacgccatcattcggacttacggcagtccacaggctatcaatattgagctggcaagagaaatgtcaaagacctttgaagagaggcgcaaaatcaagggggacatggagaaacggcagaagaacaatgaagatgtgaagaaacagattcaggagctgggaaaactgtctcctacaggccaggacatcctgaagtacagactgtggcaggagcagcaggggatttgtatgtatagtggaaaaaccatcccactggaagagctgttcaagcccggctacgacatcgatcacattctgccctattcaattacattcgacgatagctttaggaacaaagtgctggtcacatcccaggagaacagacagaagggcaataggactccttacgagtatatggggaacgacgaacagcgctggaatgagtttgaaaccagggtgaaaactaccatccgcgattacaagaaacagcagaagctgctgaagaaacatttctctgaagaggaaaggagtgagtttaaagaacggaacctgacagacactaagtacatcacaaccgtgatctacaacatgatcagacagaatctggagatggcccccctgaaccgccctgaaaagaaaaagcaggtgcgggctgtcaatggcgcaattaccgcctacctgcgaaaacggtgggggctgccacagaagaatcgggagacagacacacaccatgctatggatgcagtggtcatcgcctgctgtaccgacggcatgatccagaaaattagtagatacacaaaggtgagagagaggtgctattcaaagggaacagagttcgtcgatgcagagactggcgaaatctttagacccgaggactacagcagggccgagtgggatgaaattttcggcgtgcacatcccaaagccctgggagacatttcgcgccgaactggacgtccgaatgggggacgatccaaagggattcctggacactcatagcgatgtggctctggagctggattatcccgagtacatctacgaaaacctgcggcctatcttcgtgagcagaatgccaaatcacaaggtcaccggagcagcccatgctgacacaattcggtccccaagacactttaaagatgagggcatcgtgctgactaagaccgcactgaccgacctgaaactggacaaggatggggagatcgacggatactataacccccagtccgatctgctgctgtacgaagcactgaaaaagcagctgctgctgtatggcaatgatgccaaaaaggccttcgctcaggactttcataaacccaaggccgatggaactgagggccctgtggtcaggaaggtgaagatccagaaaaagcagaccatgggagtgttcgtcgactctggcaacgggattgccgagaatggcgggatggtgcgcatcgatgtgttccgagtcaacggcaagtactattttgtgcccgtctacaccgctgacgtggtcaaaaaggtgctgcctaatagggccagtacagctcacaagccatacggcgagtggaaagtgatggaggacaaggatttcctgtttagtctgtattcacgcgacctgatccatatcaagtctaaaaaggatatccctattaagatggtgaacggaggcatggaggggatcaaggaaacctacgcatactatattggagccgacatcagcgctgcaaatatccagggcattgcccacgattccaggtataaattccgcggactgggcattcagtctctggacgtgctggagaagtgtcagatcgatgtgctgggacatgtcagcgtggtccgatccgaaaagcggatgggctttagctaagaattc

SEQ ID NO: 134 - DNA, 3243 bp, synthetic construct; identical to SEQ ID NO: 85
  misc_feature 1..3243: note = source = /note="Description of Artificial Sequence: Synthetic polynucleotide"
  source 1..3243: mol_type = other DNA

SEQ ID NO: 135 - DNA, 3243 bp, synthetic construct; identical to SEQ ID NO: 85
  misc_feature 1..3243: note = source = /note="Description of Artificial Sequence: Synthetic polynucleotide"
  source 1..3243: mol_type = other DNA

SEQ ID NO: 136 - DNA, 3891 bp, synthetic construct
  misc_feature 1..3891: note = source = /note="Description of Artificial Sequence: Synthetic polynucleotide"
  source 1..3891: mol_type = other DNA
accggtgccaccatgtacccatacgatgttccagattacgcttcgccgaagaaaaagcgcaaggtcgaagcgtccatgaacaatagcatcaaatctaaacctgaagtgaccatcgggctggacctgggagtgggaagcgtggggtgggcaatcgtggataacgaaacaaacatcattcaccatctgggctccaggctgttttctcaggccaagactgctgaggatcggagatctttccgcggggtgaggcgcctgatccgacggagaaaatacaagctgaaacgattcgtcaatctgatttggaagtacaacagctatttcggcttcaagaacaaagaggacatcctgaacaattatcaggagcagcagaagctgcacaataccgtgctgaacctgaaatcagaggcactgaatgccaagatcgatcctaaagcactgagctggattctgcacgactacctgaagaacagaggccatttttatgaggacaatagggatttcaacgtgtacccaacaaaggagctggccaagtacttcgataagtacgggtactacaagggaatcattgacagcaaggaggacaatgataacaaactggaggaagagctgacaaagtacaaattctccaataagcactggctggaagaggtgaagaaagtcctgtctaaccagactggcctgccagaaaagtttaaagaagagtatgagtcactgttcagctacgtgagaaattattcagagggcccagggagcatcaactctgtcagtccctacgggatctaccatctggacgaaaaagagggaaaggtggtccagaagtacaacaacatctgggataagacaatcggaaagtgcaacatcttccctgacgagtatagagctcccaagaacagtcctatcgcaatgattttcaatgaaatcaacgagctgtccacaatcaggtcatacagcatctacctgactggctggttcattaatcaggagttcaagaaagcctacctgaacaagctgctggatctgctgatcaaaaccaacggagagaagccaattgacgcaaggcagttcaagaaactgcgcgaagagacaatcgccgaaagcattggcaaagagacactgaaggatgtggagaatgaagagaaactggaaaaggaggaccacaagtggaaactgaagggactgaagctgaataccaacggcaaaatccagtacaacgatctgagctccctggctaagtttgtgcacaaactgaagcagcatctgaaactggatttcctgctggaggaccagtatgcaacactggacaagatcaatttcctgcagtccctgtttgtgtacctgggcaagcacctgagatattccaatagggtcgattctgccaacctgaaggaattttccgactctaacaaactgttcgagcgcatcctgcagaaacagaaggatgggctgttcaagctgtttgaacagactgacaaagacgatgagaagatcctggcccagacacatagtctgtcaactaaggccatgctgctggctattacccggatgacaaatctggacaacgatgaggacaaccagaaaaacaatgacaagggctggaattttgaggccatcaaaaacttcgatcagaagtttatcgacatcaccaagaaaaacaacaacctgagcctgaaacagaataagcgctacctggacgatcgattcatcaacgatgctattctgtcccctggggtgaagcgaatcctgcgggaggcaaccaaggtctttaatgccattctgaaacagttctctgaagagtacgacgtgacaaaggtggtcatcgaactggctcgcgagctgagcgaagagaaggaactggagaacacaaagaactacaagaaactgatcaagaaaaacggcgacaagattagtgagggcctgaaagcactggggatctcagaagatgagatcaaagacattctgaagagtcccactaaatcatacaagtttctgctgtggctgcagcaggaccacatcgatccttatagcctgaaggagatcgccttcgacgatatttttaccaaaacagaaaagttcgagatcgaccatatcattccctacagcatttccttcgacgattctagttcaaacaagctgctggtgctggctgaaagtaatcaggcaaagtcaaaccagactccttatgagttcatcagctccggaaacgcaggcattaagtgggaagattacgaggcctattgccgcaagttcaaggatggggactctagtctgctggacagcacccagcggtccaagaaattcgccaaaatgatgaaaaccgatacctcaagcaagtacgacatcggatttctggctcgaaatctgaacgatactcggtacgcaaccattgtgttccgggacgccctggaggactatgctaataaccacctggtcgaggacaaacccatgtttaaggtggtctgtatcaatgggtccgtgacctctttcctgcggaagaactttgacgattcctcttacgccaagaaagatagagacaagaatatccaccatgctgtggatgcaagtatcatctcaattttcagcaacgagacaaagactctgttcaaccagctgactcagtttgctgactataaactgttcaagaacaccgatggcagctggaagaaaatcgaccctaagacaggggtggtcactgaagtgaccgacgagaattggaagcagattagggtgcgcaaccaggtgagcgaaatcgccaaagtcattgagaagtacatccaggatagcaacatcgaaagaaaggctaggtattcccgcaaaatcgagaataagactaacatttccctgtttaatgacaccgtgtactctgccaagaaagtcggctatgaggatcagatcaaaagaaagaacctgaaaaccctggacattcacgaatctgctaaagagaataagaacagtaaagtgaagcggcagtttgtctacagaaagctggtgaatgtcagcctgctgaataacgataagctggcagacctgttcgccgaaaaagaggatatcctgatgtatagggccaatccatgggtcatcaacctggctgagcagattttcaatgaatacactgagaacaagaaaatcaagtcccagaacgtgtttgaaaaatatatgctggacctgaccaaagagttccccgagaagttcagcgagtttctggtgaagtccatgctgagaaacaagaccgccatcatctacgacgataagaaaaacattgtccatcgaatcaaacggctgaagatgctgagttcagaactgaaagagaataagctgtctaacgtgatcattaggtctaagaatcagagtgggaccaaactgtcataccaggatacaatcaacagcctggccctgatgattatgcgcagcatcgaccctactgctaagaaacagtatattcgagtgccactgaataccctgaacctgcacctgggagatcatgactttgatctgcacaatatggatgcttacctgaagaaaccaaaattcgtgaagtatctgaaagcaaacgaaatcggcgacgagtacaagccctggagggtcctgacatctggcactctgctgatccataagaaggataagaaactgatgtacatcagctccttccagaatctgaacgacgtgatcgaaattaagaatctgatcgaaaccgagtataaagagaacgacgattctgatagtaagaaaaagaaaaaggcaaaccgctttctgatgaccctgagcacaatcctgaatgactacattctgctggacgccaaggataacttcgacatcctggggctgtctaaaaatcggatcgatgagattctgaacagtaagctgggactggacaagattgtgaaataagaattc

SEQ ID NO: 137 - DNA, 3093 bp, synthetic construct
  misc_feature 1..3093: note = source = /note="Description of Artificial Sequence: Synthetic polynucleotide"
  source 1..3093: mol_type = other DNA
accggtgccaccatgtacccatacgatgttccagattacgcttcgccgaagaaaaagcgcaaggtcgaagcgtccatgaggattctggggtttgacattggcattaacagcatcgggtgggcttttgtggagaacgacgaactgaaggactgcggagtgcggatcttcacaaaggccgagaacccaaaaaataaggaaagcctggcactgccccggagaaatgcacgcagctccaggcgccgactgaaacggagaaaggcccggctgatcgctattaagagaatcctggccaaagagctgaagctgaactacaaggactatgtcgcagctgatggagagctgccaaaggcctacgaaggatccctggcatctgtgtacgagctgcggtataaggccctgacacagaacctggaaactaaagatctggccagagtgatcctgcacattgctaagcatagggggtacatgaacaagaacgagaagaaatcaaacgacgctaagaaaggaaagatcctgagcgctctgaaaaacaatgcactgaagctggagaactaccagagcgtgggcgaatacttctacaaggagttctttcagaaatacaagaaaaacacaaagaacttcatcaagatccgcaacactaaggataattacaacaattgcgtgctgtctagtgacctggaaaaagagctgaagctgatcctggaaaaacagaaggagttcggctacaactactctgaagatttcatcaacgagattctgaaggtcgccttctttcagcggcccctgaaggacttcagtcacctggtgggggcctgcactttctttgaggaagagaaaagggcctgtaagaacagctactctgcctgggagtttgtggctctgaccaagatcattaacgagatcaagagcctggagaagatcagcggcgaaattgtgccaacccagacaatcaacgaggtcctgaatctgatcctggacaaggggtctatcacctacaagaaattcagaagttgtatcaatctgcatgagagtatcagcttcaagagcctgaagtatgataaagaaaacgccgagaatgctaaactgatcgacttccgcaagctggtggagtttaagaaagccctgggagtccacagcctgtcccggcaggaactggatcagatctccactcatatcaccctgattaaggacaacgtgaagctgaaaaccgtcctggagaaatacaacctgagtaatgaacagatcaacaatctgctggaaattgagttcaacgattatatcaacctgagcttcaaggccctgggaatgattctgccactgatgcgcgagggcaaacgatacgacgaggcctgcgagatcgccaatctgaaacctaagaccgtggacgagaagaaagatttcctgccagcattttgtgattccattttcgcccacgagctgtctaaccccgtggtcaatagggctatcagcgaataccgcaaggtgctgaacgcactgctgaagaaatatggaaaggtccacaaaattcatctggagctggctcgcgacgtgggcctgtccaagaaagcacgagagaagatcgaaaaagagcagaaggaaaaccaggccgtgaatgcatgggccctgaaggaatgcgagaatattggcctgaaggccagcgcaaagaacatcctgaaactgaagctgtggaaagaacagaaggagatctgtatctactccggaaataagatctctattgagcacctgaaagatgaaaaggccctggaggtggaccatatctacccctattctaggagtttcgacgattcttttatcaacaaagtgctggtgttcaccaaggaaaatcaggagaaactgaacaagacacctttcgaggcctttggcaagaatattgaaaaatggagcaagatccagaccctggctcagaacctgccatacaagaaaaagaataagattctggacgagaacttcaaagataagcagcaggaggactttatctctcgaaatctgaacgacacccggtatatcgctacactgattgcaaaatacacaaaggagtatctgaacttcctgctgctgagcgaaaatgagaacgccaatctgaagagtggcgaaaaagggtcaaagatccacgtgcagactattagcgggatgctgacctccgtcctgaggcacacatgggggtttgacaaaaaggatcgcaacaatcatctgcaccatgcactggatgccatcattgtggcctacagtacaaattcaatcattaaggctttcagcgatttccggaaaaaccaggagctgctgaaggccagattctacgctaaagaactgacttccgataactataaacatcaggtcaagttctttgagcctttcaagagttttagagaaaaaatcctgtcaaagatcgacgagattttcgtgtccaaaccacctcgaaagcgagctaggcgcgcactgcacaaggatacctttcattctgagaacaagatcattgacaagtgcagctacaactccaaggaaggcctgcagattgccctgagctgtggaagagtgaggaaaatcggcactaagtatgtcgagaatgataccatcgtgagggtcgacattttcaaaaagcagaacaagttttacgctatcccaatctacgcaatggattttgccctggggatcctgcccaataagatcgtgattactggaaaagataagaacaataaccccaaacagtggcagaccattgacgaatcatacgagttctgctttagcctgtataagaatgacctgatcctgctgcagaaaaagaacatgcaggaacctgagttcgcctactataacgatttttcaatcagcacatcaagcatttgtgtggagaaacacgacaacaagttcgaaaatctgactagcaaccagaagctgctgttttccaatgcaaaagagggctctgtgaaggtcgaaagtctggggatccagaacctgaaagtgttcgagaagtacatcattacccccctgggagataaaattaaggctgactttcagcctcgagaaaacatcagcctgaaaaccagtaaaaagtatggcctgaggtaagaattc

SEQ ID NO: 138 - DNA, 4104 bp, Homo sapiens
  source 1..4104: mol_type = unassigned DNA
  CDS 1..4104
atggacaagaagtacagcatcggcctggacatcggcaccaactctgtgggctgggccgtgatcaccgacgagtacaaggtgcccagcaagaaattcaaggtgctgggcaacaccgaccggcacagcatcaagaagaacctgatcggagccctgctgttcgacagcggcgaaacagccgaggccacccggctgaagagaaccgccagaagaagatacaccagacggaagaaccggatctgctatctgcaagagatcttcagcaacgagatggccaaggtggacgacagcttcttccacagactggaagagtccttcctggtggaagaggataagaagcacgagcggcaccccatcttcggcaacatcgtggacgaggtggcctaccacgagaagtaccccaccatctaccacctgagaaagaaactggtggacagcaccgacaaggccgacctgcggctgatctatctggccctggcccacatgatcaagttccggggccacttcctgatcgagggcgacctgaaccccgacaacagcgacgtggacaagctgttcatccagctggtgcagacctacaaccagctgttcgaggaaaaccccatcaacgccagcggcgtggacgccaaggccatcctgtctgccagactgagcaagagcagacggctggaaaatctgatcgcccagctgcccggcgagaagaagaatggcctgttcggcaacctgattgccctgagcctgggcctgacccccaacttcaagagcaacttcgacctggccgaggatgccaaactgcagctgagcaaggacacctacgacgacgacctggacaacctgctggcccagatcggcgaccagtacgccgacctgtttctggccgccaagaacctgtccgacgccatcctgctgagcgacatcctgagagtgaacaccgagatcaccaaggcccccctgagcgcctctatgatcaagagatacgacgagcaccaccaggacctgaccctgctgaaagctctcgtgcggcagcagctgcctgagaagtacaaagagattttcttcgaccagagcaagaacggctacgccggctacattgacggcggagccagccaggaagagttctacaagttcatcaagcccatcctggaaaagatggacggcaccgaggaactgctcgtgaagctgaacagagaggacctgctgcggaagcagcggaccttcgacaacggcagcatcccccaccagatccacctgggagagctgcacgccattctgcggcggcaggaagatttttacccattcctgaaggacaaccgggaaaagatcgagaagatcctgaccttccgcatcccctactacgtgggccctctggccaggggaaacagcagattcgcctggatgaccagaaagagcgaggaaaccatcaccccctggaacttcgaggaagtggtggacaagggcgcttccgcccagagcttcatcgagcggatgaccaacttcgataagaacctgcccaacgagaaggtgctgcccaagcacagcctgctgtacgagtacttcaccgtgtataacgagctgaccaaagtgaaatacgtgaccgagggaatgagaaagcccgccttcctgagcggcgagcagaaaaaggccatcgtggacctgctgttcaagaccaaccggaaagtgaccgtgaagcagctgaaagaggactacttcaagaaaatcgagtgcttcgactccgtggaaatctccggcgtggaagatcggttcaacgcctccctgggcacataccacgatctgctgaaaattatcaaggacaaggacttcctggacaatgaggaaaacgaggacattctggaagatatcgtgctgaccctgacactgtttgaggacagagagatgatcgaggaacggctgaaaacctatgcccacctgttcgacgacaaagtgatgaagcagctgaagcggcggagatacaccggctggggcaggctgagccggaagctgatcaacggcatccgggacaagcagtccggcaagacaatcctggatttcctgaagtccgacggcttcgccaacagaaacttcatgcagctgatccacgacgacagcctgacctttaaagaggacatccagaaagcccaggtgtccggccagggcgatagcctgcacgagcacattgccaatctggccggcagccccgccattaagaagggcatcctgcagacagtgaaggtggtggacgagctcgtgaaagtgatgggccggcacaagcccgagaacatcgtgatcgccatggccagagagaaccagaccacccagaagggacagaagaacagccgcgagagaatgaagcggatcgaagagggcatcaaagagctgggcagccagatcctgaaagaacaccccgtggaaaacacccagctgcagaacgagaagctgtacctgtactacctgcagaatgggcgggatatgtacgtggaccaggaactggacatcaaccggctgtccgactacgatgtggacgccatcgtgcctcagagctttctgaaggacgactccatcgacgccaaggtgctgaccagaagcgacaaggcccggggcaagagcgacaacgtgccctccgaagaggtcgtgaagaagatgaagaactactggcggcagctgctgaacgccaagctgattacccagagaaagttcgacaatctgaccaaggccgagagaggcggcctgagcgaactggataaggccggcttcatcaagagacagctggtggaaacccggcagatcacaaagcacgtggcacagatcctggactcccggatgaacactaagtacgacgagaatgacaagctgatccgggaagtgaaagtgatcaccctgaagtccaagctggtgtccgatttccggaaggatttccagttttacaaagtgcgcgagatcaacaactaccaccacgcccacgccgcctacctgaacgccgtcgtgggaaccgccctgatcaaaaagtaccctaagctggaaagcgagttcgtgtacggcgactacaaggtgtacgacgtgcggaagatgatcgccaagagcgagcaggaaatcggcaaggctaccgccaagtacttcttctacagcaacatcatgaactttttcaagaccgagattaccctggccaacggcgagatccggaagcggcctctgatcgagacaaacggcgaaaccggggagatcgtgtgggataagggccgggattttgccaccgtgcggaaagtgctgagcatgccccaagtgaatatcgtgaaaaagaccgaggtgcagacaggcggcttcagcaaagagtctatcctgcccaagaggaacagcgataagctgatcgccagaaagaaggactgggaccctaagaagtacggcggcttcgacagccccaccgtggcctattctgtgctggtggtggccaaagtggaaaagggcaagtccaagaaactgaagagtgtgaaagagctgctggggatcaccatcatggaaagaagcagcttcgagaagaatcccatcgactttctggaagccaagggctacaaagaagtgaaaaaggacctgatcatcaagctgcctaagtactccctgttcgagctggaaaacggccggaagagaatgctggcctctgccggcgaactgcagaagggaaacgaactggccctgccctccaaatatgtgaacttcctgtacctggccagccactatgagaagctgaagggctcccccgaggataatgagcagaaacagctgtttgtggaacagcacaagcactacctggacgagatcatcgagcagatcagcgagttctccaagagagtgatcctggccgacgctaatctggacaaagtgctgtccgcctacaacaagcaccgggataagcccatcagagagcaggccgagaatatcatccacctgtttaccctgaccaatctgggagcccctgccgccttcaagtactttgacaccaccatcgaccggaagaggtacaccagcaccaaagaggtgctggacgccaccctgatccaccagagcatcaccggcctgtacgagacacggatcgacctgtctcagctgggaggcgac

SEQ ID NO: 139 - protein, 1368 aa, Homo sapiens
MDKKYSIGLDIGTNSVGWAVITDEYKVPSKKFKVLGNTDRHSIKKNLIGALLFDSGETAEATRLKRTARRRYTRRKNRICYLQEIFSNEMAKVDDSFFHRLEESFLVEEDKKHERHPIFGNIVDEVAYHEKYPTIYHLRKKLVDSTDKADLRLIYLALAHMIKFRGHFLIEGDLNPDNSDVDKLFIQLVQTYNQLFEENPINASGVDAKAILSARLSKSRRLENLIAQLPGEKKNGLFGNLIALSLGLTPNFKSNFDLAEDAKLQLSKDTYDDDLDNLLAQIGDQYADLFLAAKNLSDAILLSDILRVNTEITKAPLSASMIKRYDEHHQDLTLLKALVRQQLPEKYKEIFFDQSKNGYAGYIDGGASQEEFYKFIKPILEKMDGTEELLVKLNREDLLRKQRTFDNGSIPHQIHLGELHAILRRQEDFYPFLKDNREKIEKILTFRIPYYVGPLARGNSRFAWMTRKSEETITPWNFEEVVDKGASAQSFIERMTNFDKNLPNEKVLPKHSLLYEYFTVYNELTKVKYVTEGMRKPAFLSGEQKKAIVDLLFKTNRKVTVKQLKEDYFKKIECFDSVEISGVEDRFNASLGTYHDLLKIIKDKDFLDNEENEDILEDIVLTLTLFEDREMIEERLKTYAHLFDDKVMKQLKRRRYTGWGRLSRKLINGIRDKQSGKTILDFLKSDGFANRNFMQLIHDDSLTFKEDIQKAQVSGQGDSLHEHIANLAGSPAIKKGILQTVKVVDELVKVMGRHKPENIVIAMARENQTTQKGQKNSRERMKRIEEGIKELGSQILKEHPVENTQLQNEKLYLYYLQNGRDMYVDQELDINRLSDYDVDAIVPQSFLKDDSIDAKVLTRSDKARGKSDNVPSEEVVKKMKNYWRQLLNAKLITQRKFDNLTKAERGGLSELDKAGFIKRQLVETRQITKHVAQILDSRMNTKYDENDKLIREVKVITLKSKLVSDFRKDFQFYKVREINNYHHAHAAYLNAVVGTALIKKYPKLESEFVYGDYKVYDVRKMIAKSEQEIGKATAKYFFYSNIMNFFKTEITLANGEIRKRPLIETNGETGEIVWDKGRDFATVRKVLSMPQVNIVKKTEVQTGGFSKESILPKRNSDKLIARKKDWDPKKYGGFDSPTVAYSVLVVAKVEKGKSKKLKSVKELLGITIMERSSFEKNPIDFLEAKGYKEVKKDLIIKLPKYSLFELENGRKRMLASAGELQKGNELALPSKYVNFLYLASHYEKLKGSPEDNEQKQLFVEQHKHYLDEIIEQISEFSKRVILADANLDKVLSAYNKHRDKPIREQAENIIHLFTLTNLGAPAAFKYFDTTIDRKRYTSTKEVLDATLIHQSITGLYETRIDLSQLGGD

SEQ ID NO: 140 - RNA, 155 nt, unidentified; identical to SEQ ID NO: 102
  source 1..155: mol_type = unassigned RNA

SEQ ID NO: 141 - RNA, 107 nt, Treponema denticola; identical to SEQ ID NO: 103
  source 1..107: mol_type = unassigned RNA

SEQ ID NO: 142 - RNA, 99 nt, Filifactor alocis; identical to SEQ ID NO: 104
  source 1..99: mol_type = unassigned RNA

SEQ ID NO: 143 - RNA, 91 nt, Staphylococcus pseudintermedius; identical to SEQ ID NO: 105
  source 1..91: mol_type = unassigned RNA

SEQ ID NO: 144 - RNA, 94 nt, Lactobacillus johnsonii; identical to SEQ ID NO: 106
  source 1..94: mol_type = unassigned RNA

SEQ ID NO: 145 - RNA, 78 nt, Eubacterium ventriosum; identical to SEQ ID NO: 107
  source 1..78: mol_type = unassigned RNA

SEQ ID NO: 146 - RNA, 84 nt, unidentified; identical to SEQ ID NO: 108
  source 1..84: mol_type = unassigned RNA

SEQ ID NO: 147 - RNA, 85 nt, Lactobacillus farciminis; identical to SEQ ID NO: 109
  source 1..85: mol_type = unassigned RNA

SEQ ID NO: 148 - RNA, 100 nt, Bacteroides coprophilus; identical to SEQ ID NO: 110
  source 1..100: mol_type = unassigned RNA

SEQ ID NO: 149 - RNA, 102 nt, unidentified; identical to SEQ ID NO: 111
  source 1..102: mol_type = unassigned RNA

SEQ ID NO: 150 - RNA, 90 nt, Flavobacterium columnare; identical to SEQ ID NO: 112
  source 1..90: mol_type = unassigned RNA

SEQ ID NO: 151 - RNA, 78 nt, unidentified; identical to SEQ ID NO: 113
  source 1..78: mol_type = unassigned RNA

SEQ ID NO: 152 - RNA, 85 nt, Azospirillum sp.; identical to SEQ ID NO: 114
  source 1..85: mol_type = unassigned RNA

SEQ ID NO: 153 - RNA, 126 nt, unidentified; identical to SEQ ID NO: 115
  source 1..126: mol_type = unassigned RNA

SEQ ID NO: 154 - RNA, 82 nt, Roseburia intestinalis; identical to SEQ ID NO: 116
  source 1..82: mol_type = unassigned RNA

SEQ ID NO: 155 - RNA, 83 nt, Staphylococcus aureus; identical to SEQ ID NO: 117
  source 1..83: mol_type = unassigned RNA

SEQ ID NO: 156 - RNA, 94 nt, Mycoplasma gallisepticum; identical to SEQ ID NO: 118
  source 1..94: mol_type = unassigned RNA

SEQ ID NO: 157 - RNA, 117 nt, Campylobacter lari
  source 1..117: mol_type = unassigned RNA
gttttagtctctgaaaagagactaaaataagtggtttttggtcatccacgcagggttacaatccctttaaaaccattaaaattcaaataaactaggttgtatcaacttagttttttt

SEQ ID NO: 158 - RNA, 119 nt, synthetic construct
  misc_feature 1..119: note = source = /note="Description of Artificial Sequence: Synthetic polynucleotide"
  source 1..119: mol_type = other RNA
nnnnnnnnnnnnnnnnnnnnactggggttcaggaaactgaacctcagtaagcattggctcgtttccaatgttgattgctccgccggtgctccttatttttaagggcgccggcttttttt

SEQ ID NO: 159 - protein, 1084 aa, Corynebacterium diphtheriae
MKYHVGIDVGTFSVGLAAIEVDDAGMPIKTLSLVSHIHDSGLDPDEIKSAVTRLASSGIARRTRRLYRRKRRRLQQLDKFIQRQGWPVIELEDYSDPLYPWKVRAELAASYIADEKERGEKLSVALRHIARHRGWRNPYAKVSSLYLPDGPSDAFKAIREEIKRASGQPVPETATVGQMVTLCELGTLKLRGEGGVLSARLQQSDYAREIQEICRMQEIGQELYRKIIDVVFAAESPKGSASSRVGKDPLQPGKNRALKASDAFQRYRIAALIGNLRVRVDGEKRILSVEEKNLVFDHLVNLTPKKEPEWVTIAEILGIDRGQLIGTATMTDDGERAGARPPTHDTNRSIVNSRIAPLVDWWKTASALEQHAMVKALSNAEVDDFDSPEGAKVQAFFADLDDDVHAKLDSLHLPVGRAAYSEDTLVRLTRRMLSDGVDLYTARLQEFGIEPSWTPPTPRIGEPVGNPAVDRVLKTVSRWLESATKTWGAPERVIIEHVREGFVTEKRAREMDGDMRRRAARNAKLFQEMQEKLNVQGKPSRADLWRYQSVQRQNCQCAYCGSPITFSNSEMDHIVPRAGQGSTNTRENLVAVCHRCNQSKGNTPFAIWAKNTSIEGVSVKEAVERTRHWVTDTGMRSTDFKKFTKAVVERFQRATMDEEIDARSMESVAWMANELRSRVAQHFASHGTTVRVYRGSLTAEARRASGISGKLKFFDGVGKSRLDRRHHAIDAAVIAFTSDYVAETLAVRSNLKQSQAHRQEAPQWREFTGKDAEHRAAWRVWCQKMEKLSALLTEDLRDDRVVVMSNVRLRLGNGSAHKETIGKLSKVKLSSQLSVSDIDKASSEALWCALTREPGFDPKEGLPANPERHIRVNGTHVYAGDNIGLFPVSAGSIALRGGYAELGSSFHHARVYKITSGKKPAFAMLRVYTIDLLPYRNQDLFSVELKPQTMSMRQAEKKLRDALATGNAEYLGWLVVDDELVVDTSKIATDQVKAVEAELGTIRRWRVDGFFSPSKLRLRPLQMSKEGIKKESAPELSKIIDRPGWLPAVNKLFSDGNVTVVRRDSLGRVRLESTAHLPVTWKVQ

SEQ ID NO: 160 - DNA, 3336 bp, synthetic construct
  misc_feature 1..3336: note = source = /note="Description of Artificial Sequence: Synthetic polynucleotide"
  source 1..3336: mol_type = other DNA
accggtgccaccatgtacccatacgatgttccagattacgcttcgccgaagaaaaagcgcaaggtcgaagcgtccatgaagtaccatgtcggaatcgatgtcggaaccttttctgtggggctggctgctattgaagtggatgacgctggaatgcctattaagaccctgagtctggtgtcacacattcatgactcaggactggatcctgacgagatcaagagcgctgtgaccaggctggcaagctccggaatcgcccggagaacaaggcgcctgtaccgacggaagagaaggcgcctgcagcagctggataagttcatccagaggcagggctggccagtgatcgagctggaagattacagcgaccccctgtatccttggaaggtgcgcgccgaactggccgcttcttatattgctgacgagaaggaacggggggagaaactgagtgtggctctgagacacatcgcaaggcatcgcggatggaggaacccttacgccaaggtgtctagtctgtatctgccagatggcccctcagacgccttcaaggctattagggaggaaatcaaacgcgctagcggccagcctgtgccagagactgcaaccgtcgggcagatggtgaccctgtgcgaactgggcacactgaagctgcgaggagagggaggagtgctgagtgcacggctgcagcagtcagattacgcccgcgagatccaggaaatttgtcgaatgcaggagatcggccaggaactgtatcgcaagatcattgacgtggtgttcgcagccgagtccccaaagggctctgcctcaagccgggtggggaaagatcctctgcagccaggaaagaacagagcactgaaagccagcgacgcttttcagcgataccggattgctgcactgatcggcaatctgagagtcagggtggatggggagaagaggattctgagcgtggaggagaagaacctggtgttcgaccacctggtgaatctgactccaaagaaagagcccgaatgggtgaccatcgccgaaattctgggcatcgatcgcgggcagctgatcggaacagctactatgaccgacgatggagagcgagcaggagcccgaccccctacacacgatactaacagaagtattgtgaacagccggatcgcaccactggtcgactggtggaaaacagctagcgcactggagcagcacgccatggtgaaggcactgtccaacgccgaagtcgacgattttgattctcccgagggagcaaaagtgcaggcattctttgccgatctggacgatgacgtccacgccaagctggacagcctgcatctgcctgtgggacgagcagcttactccgaggacactctggtcagactgacccgacggatgctgagtgatggggtggacctgtataccgcccggctgcaggagttcggaattgaacctagctggaccccacccacaccaagaatcggagagcctgtcggcaatccagccgtcgaccgggtgctgaaaacagtgagcagatggctggaatccgcaacaaagacttggggcgccccagagagggtcatcattgagcacgtgcgcgaaggcttcgtcactgagaaacgcgctcgagaaatggatggggacatgagaaggcgcgcagcccggaacgccaagctgtttcaggagatgcaggaaaagctgaatgtgcagggcaaacccagtcgagccgatctgtggagataccagtcagtgcagagacagaactgccagtgtgcctattgcgggtccccaattaccttttctaatagtgaaatggaccacatcgtgcccagagcagggcagggatccaccaacacaagggagaatctggtcgccgtgtgccatcgctgtaaccagtctaagggcaatacacccttcgctatttgggcaaaaaacacttctatcgaaggggtcagtgtgaaggaggccgtggaacggaccagacattgggtcactgataccggcatgagaagcactgacttcaagaagttcaccaaggctgtggtcgagcggtttcagagagcaacaatggatgaggaaatcgacgccagaagcatggaatccgtcgcctggatggctaatgagctgaggagccgcgtggctcagcacttcgcatcccatggaaccacagtcagggtgtaccgaggcagcctgacagcagaggctcgacgggcatctgggatcagtggaaagctgaaattctttgatggcgtggggaagtccaggctggatagaaggcaccatgctattgacgctgcagtgatcgcattcacctctgactatgtggccgaaacactggctgtccgctcaaacctgaaacagagccaggcccaccgacaggaggctcctcagtggagagagttcaccggcaaggatgcagagcatcgagcagcttggagagtgtggtgccagaagatggaaaaactgagcgccctgctgaccgaggacctgcgagatgaccgggtggtcgtgatgtctaacgtgcgactgcggctgggaaatggcagtgcccacaaggaaaccattggcaaactgtcaaaggtgaaactgtcctctcagctgtcagtcagcgatatcgacaaagcaagttcagaggccctgtggtgtgctctgaccagagagcccggattcgatcctaaggaaggcctgcccgctaaccctgagagacacatcagggtgaatgggacacatgtctacgccggggacaatattggactgtttccagtgtcagcaggaagcatcgcactgaggggaggatacgcagagctgggcagctccttccaccatgctcgcgtgtataaaattacttccggcaagaaacccgcatttgccatgctgagggtgtacaccatcgatctgctgccttatcgcaaccaggacctgtttagcgtggaactgaagccacagacaatgtccatgaggcaggctgagaagaaactgcgcgacgctctggcaactgggaatgcagaatatctgggatggctggtcgtggatgacgagctggtcgtggatacatctaagattgccactgaccaggtcaaagcagtggaggccgaactggggactatccgccgatggcgggtggatggattcttttccccctctaaactgagactgaggcctctgcagatgtccaaggaggggatcaagaaagagtccgctcccgaactgtctaaaatcattgacagaccaggatggctgcccgccgtgaacaagctgttctctgatggaaatgtcaccgtcgtgcggagagactctctgggacgcgtgcgactggagagtacagcccacctgcctgtcacttggaaggtgcagtaagaattc

SEQ ID NO: 161 - RNA, 175 nt, synthetic construct
  misc_feature 1..175: note = source = /note="Description of Artificial Sequence: Synthetic polynucleotide"
  source 1..175: mol_type = other RNA
nnnnnnnnnnnnnnnnnnnngtttcagtgctataggaaactataggaaatcaccttcgggtgagctgaaatcccctaaagctaagattgaatccggccactatctattagtagatatccggatattctgatataaaacctcattctttgattagaccaaaggatgaggttttttt

SEQ ID NO: 162 - protein, 1422 aa, Sutterella wadsworthensis
MTQSERRFSCSIGIDMGAKYTGVFYALFDREELPTNLNSKAMTLVMPETGPRYVQAQRTAVRHRLRGQKRYTLARKLAFLVVDDMIKKQEKRLTDEEWKRGREALSGLLKRRGYSRPNADGEDLTPLENVRADVFAAHPAFSTYFSEVRSLAEQWEEFTANISNVEKFLGDPNIPADKEFIEFAVAEGLIDKTEKKAYQSALSTLRANANVLTGLRQMGHKPRSEYFKAIEADLKKDSRLAKINEAFGGAERLARLLGNLSNLQLRAERWYFNAPDIMKDRGWEPDRFKKTLVRAFKFFHPAKDQNKQHLELIKQIENSEDIIETLCTLDPNRTIPPYEDQNNRRPPLDQTLLLSPEKLTRQYGEIWKTWSARLTSAEPTLAPAAEILERSTDRKSRVAVNGHEPLPTLAYQLSYALQRAFDRSKALDPYALRALAAGSKSNKLTSARTALENCIGGQNVKTFLDCARRYYREADDAKVGLWFDNADGLLERSDLHPPMKKKILPLLVANILQTDETTGQKFLDEIWRKQIKGRETVASRCARIETVRKSFGGGFNIAYNTAQYREVNKLPRNAQDKELLTIRDRVAETADFIAANLGLSDEQKRKFANPFSLAQFYTLIETEVSGFSATTLAVHLENAWRMTIKDAVINGETVRAAQCSRLPAETARPFDGLVRRLVDRQAWEIAKRVSTDIQSKVDFSNGIVDVSIFVEENKFEFSASVADLKKNKRVKDKMLSEAEKLETRWLIKNERIKKASRGTCPYTGDRLAEGGEIDHILPRSLIKDARGIVFNAEPNLIYASSRGNQLKKNQRYSLSDLKANYRNEIFKTSNIAAITAEIEDVVTKLQQTHRLKFFDLLNEHEQDCVRHALFLDDGSEARDAVLELLATQRRTRVNGTQIWMIKNLANKIREELQNWCKTTNNRLHFQAAATNVSDAKNLRLKLAQNQPDFEKPDIQPIASHSIDALCSFAVGSADAERDQNGFDYLDGKTVLGLYPQSCEVIHLQAKPQEEKSHFDSVAIFKEGIYAEQFLPIFTLNEKIWIGYETLNAKGERCGAIEVSGKQPKELLEMLAPFFNKPVGDLSAHATYRILKKPAYEFLAKAALQPLSAEEKRLAALLDALRYCTSRKSLMSLFMAANGKSLKKREDVLKPKLFQLKVELKGEKSFKLNGSLTLPVKQDWLRICDSPELADAFGKPCSADELTSKLARIWKRPVMRDLAHAPVRREFSLPAIDNPSGGFRIRRTNLFGNELYQVHAINAKKYRGFASAGSNVDWSKGILFNELQHENLTECGGRFITSADVTPMSEWRKVVAEDNLSIWIAPGTEGRRYVRVETTFIQASHWFEQSVENWAITSPLSLPASFKVDKPAEFQKAVGTELSELLGQPRSEIFIENVGNAKHIRFWYIVVSSNKKMNESYNNVSKS

SEQ ID NO: 163 - DNA, 4350 bp, synthetic construct; identical to SEQ ID NO: 119
  misc_feature 1..4350: note = source = /note="Description of Artificial Sequence: Synthetic polynucleotide"
  source 1..4350: mol_type = other DNA

SEQ ID NO: 164 - RNA, 112 nt, synthetic construct
  misc_feature 1..112: note = source = /note="Description of Artificial Sequence: Synthetic polynucleotide"
  source 1..112: mol_type = other RNA
nnnnnnnnnnnnnnnnnnnngtttcagtggtgaaaaccctgaaatcaacaaaattaaagattgaatcgtttttctatgctcgtcttaatagcgagcatataacgattttttt

SEQ ID NO: 165 - protein, 1372 aa, Legionella pneumophila
MESSQILSPIGIDLGGKFTGVCLSHLEAFAELPNHANTKYSVILIDHNNFQLSQAQRRATRHRVRNKKRNQFVKRVALQLFQHILSRDLNAKEETALCHYLNNRGYTYVDTDLDEYIKDETTINLLKELLPSESEHNFIDWFLQKMQSSEFRKILVSKVEEKKDDKELKNAVKNIKNFITGFEKNSVEGHRHRKVYFENIKSDITKDNQLDSIKKKIPSVCLSNLLGHLSNLQWKNLHRYLAKNPKQFDEQTFGNEFLRMLKNFRHLKGSQESLAVRNLIQQLEQSQDYISILEKTPPEITIPPYEARTNTGMEKDQSLLLNPEKLNNLYPNWRNLIPGIIDAHPFLEKDLEHTKLRDRKRIISPSKQDEKRDSYILQRYLDLNKKIDKFKIKKQLSFLGQGKQLPANLIETQKEMETHFNSSLVSVLIQIASAYNKEREDAAQGIWFDNAFSLCELSNINPPRKQKILPLLVGAILSEDFINNKDKWAKFKIFWNTHKIGRTSLKSKCKEIEEARKNSGNAFKIDYEEALNHPEHSNNKALIKIIQTIPDIIQAIQSHLGHNDSQALIYHNPFSLSQLYTILETKRDGFHKNCVAVTCENYWRSQKTEIDPEISYASRLPADSVRPFDGVLARMMQRLAYEIAMAKWEQIKHIPDNSSLLIPIYLEQNRFEFEESFKKIKGSSSDKTLEQAIEKQNIQWEEKFQRIINASMNICPYKGASIGGQGEIDHIYPRSLSKKHFGVIFNSEVNLIYCSSQGNREKKEEHYLLEHLSPLYLKHQFGTDNVSDIKNFISQNVANIKKYISFHLLTPEQQKAARHALFLDYDDEAFKTITKFLMSQQKARVNGTQKFLGKQIMEFLSTLADSKQLQLEFSIKQITAEEVHDHRELLSKQEPKLVKSRQQSFPSHAIDATLTMSIGLKEFPQFSQELDNSWFINHLMPDEVHLNPVRSKEKYNKPNISSTPLFKDSLYAERFIPVWVKGETFAIGFSEKDLFEIKPSNKEKLFTLLKTYSTKNPGESLQELQAKSKAKWLYFPINKTLALEFLHHYFHKEIVTPDDTTVCHFINSLRYYTKKESITVKILKEPMPVLSVKFESSKKNVLGSFKHTIALPATKDWERLFNHPNFLALKANPAPNPKEFNEFIRKYFLSDNNPNSDIPNNGHNIKPQKHKAVRKVFSLPVIPGNAGTMMRIRRKDNKGQPLYQLQTIDDTPSMGIQINEDRLVKQEVLMDAYKTRNLSTIDGINNSEGQAYATFDNWLTLPVSTFKPEIIKLEMKPHSKTRRYIRITQSLADFIKTIDEALMIKPSDSIDDPLNMPNEIVCKNKLFGNELKPRDGKMKIVSTGKIVTYEFESDSTPQWIQTLYVTQLKKQP

SEQ ID NO: 166 - DNA, 4200 bp, synthetic construct
  misc_feature 1..4200: note = source = /note="Description of Artificial Sequence: Synthetic polynucleotide"
  source 1..4200: mol_type = other DNA
accggtgccaccatgtacccatacgatgttccagattacgcttcgccgaagaaaaagcgcaaggtcgaagcgtccatggagtcctctcagatcctgtcacctatcggcatcgacctgggcggaaagtttactggagtctgcctgtcacacctggaagcatttgctgagctgcctaaccacgcaaatacaaagtactcagtgatcctgattgatcataacaatttccagctgagccaggcacagcggagagccactagacacagggtgcgcaacaagaaaagaaatcagttcgtgaagagggtcgccctgcagctgtttcagcacatcctgtcccgggacctgaacgccaaggaggaaaccgctctgtgccattacctgaacaatagaggctacacctatgtggacacagatctggacgagtatatcaaagatgaaaccacaattaacctgctgaaggagctgctgccaagcgagtccgaacataatttcattgactggtttctgcagaagatgcagagctccgagttccggaagatcctggtgagcaaagtcgaggaaaagaaagacgataaagaactgaagaacgccgtgaagaacatcaagaacttcatcaccggattcgagaaaaatagcgtggaaggccaccgacatcggaaggtctactttgagaacatcaagtccgatattacaaaagacaatcagctggattctatcaagaaaaagattcctagcgtgtgtctgtccaacctgctgggccacctgtccaacctgcagtggaagaatctgcataggtatctggccaaaaatccaaagcagttcgacgagcagaccttcgggaacgaatttctgcggatgctgaagaattttcgacacctgaaaggatctcaggagagtctggctgtgcgcaacctgatccagcagctggaacagtctcaggattacatcagtatcctggagaaaaccccccctgaaatcaccattccaccctatgaggcccggacaaacactggcatggaaaaagaccagagcctgctgctgaaccccgagaagctgaacaatctgtacccaaactggagaaatctgatccccgggatcattgacgcccaccctttcctggagaaggatctggaacatacaaagctgagagacaggaaacgcatcatttctcccagtaaacaggacgagaagcgggatagctacatcctgcagagatatctggacctgaacaaaaagatcgataagttcaagatcaagaagcagctgagctttctgggacagggcaaacagctgcctgctaacctgatcgagacacagaaggagatggaaactcacttcaattctagtctggtgtctgtcctgatccagattgctagtgcatacaacaaggagagggaagatgccgctcaggggatctggttcgacaatgccttttcactgtgcgagctgagcaacatcaatcctccacgcaaacagaagattctgcccctgctggtgggagcaatcctgagcgaggacttcattaacaacaaggataagtgggccaaattcaagatcttttggaacacccacaagattgggcgaacatcactgaaaagcaagtgtaaagagatcgaggaagcccggaagaacagtggaaacgcttttaaaatcgactacgaggaagctctgaatcacccagagcattcaaacaacaaggccctgatcaagatcattcagaccattcccgatatcattcaggccatccagtcacacctgggacataacgacagccaggctctgatctaccacaatcctttctcactgagccagctgtatactatcctggagacaaagagggatggctttcataaaaactgcgtggccgtcacttgtgaaaattactggcggagccagaaaaccgagatcgacccagaaatttcctatgcatctaggctgccagcagacagtgtgcgccccttcgatggcgtcctggcacgaatgatgcagcggctggcctacgagatcgccatggctaagtgggaacagatcaaacacattcctgataactcaagcctgctgatcccaatctacctggagcagaatcggttcgaatttgaggagagcttcaagaagatcaaggggtcctctagtgacaaaaccctggagcaggccatcgaaaagcagaacattcagtgggaggaaaagttccagagaatcattaacgcaagtatgaatatctgcccttacaagggcgcctcaattggcgggcagggggagatcgaccacatctacccaaggtccctgtctaaaaagcatttcggcgtgatctttaactccgaagtcaatctgatctactgttcaagccaggggaatcgcgagaaaaaggaggaacactacctgctggaacatctgtctccactgtatctgaaacaccagttcggcactgacaacgtgtccgatatcaagaattttatttctcagaacgtcgctaatatcaaaaagtacatttccttccacctgctgaccccagagcagcagaaggcagcacggcacgccctgtttctggattatgacgatgaagcattcaaaaccattacaaagtttctgatgtctcagcagaaggccagagtgaacggcacacagaaattcctggggaagcagatcatggagtttctgtccactctggcagattctaaacagctgcagctggagttcagcatcaagcagattaccgccgaggaagtgcacgaccatagagagctgctgtctaagcaggaacccaaactggtcaagagtaggcagcagagtttcccttcacacgctatcgacgcaactctgaccatgtctattgggctgaaggagttcccacagtttagtcaggaactggataactcatggtttatcaatcacctgatgccagacgaggtgcatctgaaccccgtccggagcaaggaaaagtacaacaaacctaacatctcctctactccactgttcaaggattccctgtatgctgagcggttcatccccgtgtgggtcaagggagaaaccttcgcaatcggctttagcgagaaggacctgttcgagatcaagccctccaacaaggagaaactgtttacactgctgaaaacctacagtactaaaaatcctggcgagtcactgcaggaactgcaggctaagagcaaagcaaagtggctgtacttcccaatcaacaaaaccctggccctggagttcctgcaccattattttcacaaggaaatcgtgacacccgacgatactaccgtctgccatttcatcaactcactgagatactacactaaaaaggagagcatcaccgtgaaaattctgaaggaacccatgcctgtgctgtccgtcaagttcgagagttcaaaaaagaacgtgctgggatcttttaaacacacaatcgccctgcctgctactaaggattgggagaggctgttcaaccatccaaattttctggcactgaaggccaacccagctcccaatcctaaagagttcaatgagttcatccgcaagtacttcctgagcgacaacaatcccaactccgatatccctaacaatggccacaatatcaagccccagaaacataaggccgtgcgaaaggtctttagcctgccagtgatccccgggaacgctggaaccatgatgcgcattaggcgcaaagacaataagggacagccactgtatcagctgcagacaatcgacgatactcccagcatgggcatccagattaacgaggatcgcctggtgaaacaggaagtcctgatggacgcctacaagacacgaaatctgagcactatcgatgggattaacaattccgagggacaggcatatgccacattcgacaactggctgaccctgcccgtgagcaccttcaagcctgagatcatcaagctggaaatgaagcctcactctaaaacccgacggtacatcagaattacacagagtctggccgacttcatcaaaactattgatgaggctctgatgatcaagcccagtgactcaattgacgatcctctgaacatgccaaatgagatcgtgtgtaaaaacaagctgttcgggaatgaactgaagcctagggatggaaaaatgaagatcgtgagcactggcaagattgtcacctacgagtttgaaagcgactccaccccccagtggatccagaccctgtatgtgacacagctgaaaaagcagccttaagaattc

SEQ ID NO: 167 - RNA, 127 nt, synthetic construct
  misc_feature 1..127: note = source = /note="Description of Artificial Sequence: Synthetic polynucleotide"
  source 1..127: mol_type = other RNA
nnnnnnnnnnnnnnnnnnnngtttgagagttggaaacaacgagttcaaataagaattcatcaaaatcgtcccttttgggaccgctcattgtggagcatcaaggcttaacatggttaagccttttttt

SEQ ID NO: 168 - protein, 1395 aa, Treponema denticola
MKKEIKDYFLGLDVGTGSVGWAVTDTDYKLLKANRKDLWGMRCFETAETAEVRRLHRGARRRIERRKKRIKLLQELFSQEIAKTDEGFFQRMKESPFYAEDKTILQENTLFNDKDFADKTYHKAYPTINHLIKAWIENKVKPDPRLLYLACHNIIKKRGHFLFEGDFDSENQFDTSIQALFEYLREDMEVDIDADSQKVKEILKDSSLKNSEKQSRLNKILGLKPSDKQKKAITNLISGNKINFADLYDNPDLKDAEKNSISFSKDDFDALSDDLASILGDSFELLLKAKAVYNCSVLSKVIGDEQYLSFAKVKIYEKHKTDLTKLKNVIKKHFPKDYKKVFGYNKNEKNNNNYSGYVGVCKTKSKKLIINNSVNQEDFYKFLKTILSAKSEIKEVNDILTEIETGTFLPKQISKSNAEIPYQLRKMELEKILSNAEKHFSFLKQKDEKGLSHSEKIIMLLTFKIPYYIGPINDNHKKFFPDRCWVVKKEKSPSGKTTPWNFFDHIDKEKTAEAFITSRTNFCTYLVGESVLPKSSLLYSEYTVLNEINNLQIIIDGKNICDIKLKQKIYEDLFKKYKKITQKQISTFIKHEGICNKTDEVIILGIDKECTSSLKSYIELKNIFGKQVDEISTKNMLEEIIRWATIYDEGEGKTILKTKIKAEYGKYCSDEQIKKILNLKFSGWGRLSRKFLETVTSEMPGFSEPVNIITAMRETQNNLMELLSSEFTFTENIKKINSGFEDAEKQFSYDGLVKPLFLSPSVKKMLWQTLKLVKEISHITQAPPKKIFIEMAKGAELEPARTKTRLKILQDLYNNCKNDADAFSSEIKDLSGKIENEDNLRLRSDKLYLYYTQLGKCMYCGKPIEIGHVFDTSNYDIDHIYPQSKIKDDSISNRVLVCSSCNKNKEDKYPLKSEIQSKQRGFWNFLQRNNFISLEKLNRLTRATPISDDETAKFIARQLVETRQATKVAAKVLEKMFPETKIVYSKAETVSMFRNKFDIVKCREINDFHHAHDAYLNIVVGNVYNTKFTNNPWNFIKEKRDNPKIADTYNYYKVFDYDVKRNNITAWEKGKTIITVKDMLKRNTPIYTRQAACKKGELFNQTIMKKGLGQHPLKKEGPFSNISKYGGYNKVSAAYYTLIEYEEKGNKIRSLETIPLYLVKDIQKDQDVLKSYLTDLLGKKEFKILVPKIKINSLLKINGFPCHITGKTNDSFLLRPAVQFCCSNNEVLYFKKIIRFSEIRSQREKIGKTISPYEDLSFRSYIKENLWKKTKNDEIGEKEFYDLLQKKNLEIYDMLLTKHKDTIYKKRPNSATIDILVKGKEKFKSLIIENQFEVILEILKLFSATRNVSDLQHIGGSKYSGVAKIGNKISSLDNCILIYQSITGIFEKRIDLLKV

SEQ ID NO: 169 - DNA, 4269 bp, synthetic construct; identical to SEQ ID NO: 120
  misc_feature 1..4269: note = source = /note="Description of Artificial Sequence: Synthetic polynucleotide"
  source 1..4269: mol_type = other DNA

SEQ ID NO: 170 - RNA, 119 nt, synthetic construct
  misc_feature 1..119: note = source = /note="Description of Artificial Sequence: Synthetic polynucleotide"
  source 1..119: mol_type = other RNA
nnnnnnnnnnnnnnnnnnnngtttgagagtaggaaactacacggttcaaataaagaatttttctaatcgcccaatgggcccatattgatatggatgaaactcgcttagcgagttttttt

SEQ ID NO: 171 - protein, 1365 aa, Filifactor alocis
MTKEYYLGLDVGTNSVGWAVTDSQYNLCKFKKKDMWGIRLFESANTAKDRRLQRGNRRRLERKKQRIDLLQEIFSPEICKIDPTFFIRLNESRLHLEDKSNDFKYPLFIEKDYSDIEYYKEFPTIFHLRKHLIESEEKQDIRLIYLALHNIIKTRGHFLIDGDLQSAKQLRPILDTFLLSLQEEQNLSVSLSENQKDEYEEILKNRSIAKSEKVKKLKNLFEISDELEKEEKKAQSAVIENFCKFIVGNKGDVCKFLRVSKEELEIDSFSFSEGKYEDDIVKNLEEKVPEKVYLFEQMKAMYDWNILVDILETEEYISFAKVKQYEKHKTNLRLLRDIILKYCTKDEYNRMFNDEKEAGSYTAYVGKLKKNNKKYWIEKKRNPEEFYKSLGKLLDKIEPLKEDLEVLTMMIEECKNHTLLPIQKNKDNGVIPHQVHEVELKKILENAKKYYSFLTETDKDGYSVVQKIESIFRFRIPYYVGPLSTRHQEKGSNVWMVRKPGREDRIYPWNMEEIIDFEKSNENFITRMTNKCTYLIGEDVLPKHSLLYSKYMVLNELNNVKVRGKKLPTSLKQKVFEDLFENKSKVTGKNLLEYLQIQDKDIQIDDLSGFDKDFKTSLKSYLDFKKQIFGEEIEKESIQNMIEDIIKWITIYGNDKEMLKRVIRANYSNQLTEEQMKKITGFQYSGWGNFSKMFLKGISGSDVSTGETFDIITAMWETDNNLMQILSKKFTFMDNVEDFNSGKVGKIDKITYDSTVKEMFLSPENKRAVWQTIQVAEEIKKVMGCEPKKIFIEMARGGEKVKKRTKSRKAQLLELYAACEEDCRELIKEIEDRDERDFNSMKLFLYYTQFGKCMYSGDDIDINELIRGNSKWDRDHIYPQSKIKDDSIDNLVLVNKTYNAKKSNELLSEDIQKKMHSFWLSLLNKKLITKSKYDRLTRKGDFTDEELSGFIARQLVETRQSTKAIADIFKQIYSSEVVYVKSSLVSDFRKKPLNYLKSRRVNDYHHAKDAYLNIVVGNVYNKKFTSNPIQWMKKNRDTNYSLNKVFEHDVVINGEVIWEKCTYHEDTNTYDGGTLDRIRKIVERDNILYTEYAYCEKGELFNATIQNKNGNSTVSLKKGLDVKKYGGYFSANTSYFSLIEFEDKKGDRARHIIGVPIYIANMLEHSPSAFLEYCEQKGYQNVRILVEKIKKNSLLIINGYPLRIRGENEVDTSFKRAIQLKLDQKNYELVRNIEKFLEKYVEKKGNYPIDENRDHITHEKMNQLYEVLLSKMKKFNKKGMADPSDRIEKSKPKFIKLEDLIDKINVINKMLNLLRCDNDTKADLSLIELPKNAGSFVVKKNTIGKSKIILVNQSVTGLYENRREL

SEQ ID NO: 172 - DNA, 4179 bp, synthetic construct; identical to SEQ ID NO: 121
  misc_feature 1..4179: note = source = /note="Description of Artificial Sequence: Synthetic polynucleotide"
  source 1..4179: mol_type = other DNA

SEQ ID NO: 173 - RNA, 111 nt, synthetic construct
  misc_feature 1..111: note = source = /note="Description of Artificial Sequence: Synthetic polynucleotide"
  source 1..111: mol_type = other RNA
nnnnnnnnnnnnnnnnnnnngttttagcactagaaatagttaagttaaaacaagcttaaagcgtcaatgtaatattttattaacaccctactgtgtcagtggggttttttt

SEQ ID NO: 174 - protein, 1334 aa, Staphylococcus pseudintermedius
MGRKPYILSLDIGTGSVGYACMDKGFNVLKYHDKDALGVYLFDGALTAQERRQFRTSRRRKNRRIKRLGLLQELLAPLVQNPNFYQFQRQFAWKNDNMDFKNKSLSEVLSFLGYESKKYPTIYHLQEALLLKDEKFDPELIYMALYHLVKYRGHFLFDHLKIENLTNNDNMHDFVELIETYENLNNIKLNLDYEKTKVIYEILKDNEMTKNDRAKRVKNMEKKLEQFSIMLLGLKFNEGKLFNHADNAEELKGANQSHTFADNYEENLTPFLTVEQSEFIERANKIYLSLTLQDILKGKKSMAMSKVAAYDKFRNELKQVKDIVYKADSTRTQFKKIFVSSKKSLKQYDATPNDQTFSSLCLFDQYLIRPKKQYSLLIKELKKIIPQDSELYFEAENDTLLKVLNTTDNASIPMQINLYEAETILRNQQKYHAEITDEMIEKVLSLIQFRIPYYVGPLVNDHTASKFGWMERKSNESIKPWNFDEVVDRSKSATQFIRRMTNKCSYLINEDVLPKNSLLYQEMEVLNELNATQIRLQTDPKNRKYRMMPQIKLFAVEHIFKKYKTVSHSKFLEIMLNSNHRENFMNHGEKLSIFGTQDDKKFASKLSSYQDMTKIFGDIEGKRAQIEEIIQWITIFEDKKILVQKLKECYPELTSKQINQLKKLNYSGWGRLSEKLLTHAYQGHSIIELLRHSDENFMEILTNDVYGFQNFIKEENQVQSNKIQHQDIANLTTSPALKKGIWSTIKLVRELTSIFGEPEKIIMEFATEDQQKGKKQKSRKQLWDDNIKKNKLKSVDEYKYIIDVANKLNNEQLQQEKLWLYLSQNGKCMYSGQSIDLDALLSPNATKHYEVDHIFPRSFIKDDSIDNKVLVIKKMNQTKGDQVPLQFIQQPYERIAYWKSLNKAGLISDSKLHKLMKPEFTAMDKEGFIQRQLVETRQISVHVRDFLKEEYPNTKVIPMKAKMVSEFRKKFDIPKIRQMNDAHHAIDAYLNGVVYHGAQLAYPNVDLFDFNFKWEKVREKWKALGEFNTKQKSRELFFFKKLEKMEVSQGERLISKIKLDMNHFKINYSRKLANIPQQFYNQTAVSPKTAELKYESNKSNEVVYKGLTPYQTYVVAIKSVNKKGKEKMEYQMIDHYVFDFYKFQNGNEKELALYLAQRENKDEVLDAQIVYSLNKGDLLYINNHPCYFVSRKEVINAKQFELTVEQQLSLYNVMNNKETNVEKLLIEYDFIAEKVINEYHHYLNSKLKEKRVRTFFSESNQTHEDFIKALDELFKVVTASATRSDKIGSRKNSMTHRAFLGKGKDVKIAYTSISGLKTTKPKSLFKLAESRNEL

SEQ ID NO: 175 - DNA, 4086 bp, synthetic construct; identical to SEQ ID NO: 122
  misc_feature 1..4086: note = source = /note="Description of Artificial Sequence: Synthetic polynucleotide"
  source 1..4086: mol_type = other DNA

SEQ ID NO: 176 - RNA, 114 nt, synthetic construct
  misc_feature 1..114: note = source = /note="Description of Artificial Sequence: Synthetic polynucleotide"
  source 1..114: mol_type = other RNA
nnnnnnnnnnnnnnnnnnnngttttagatggtgaaaaccagatttaaaatcaagcaatgcatcttttgatgcaaagtttcaatatttgtcccacgttatcgagggacttttttt

SEQ ID NO: 177 - protein, 1375 aa, Lactobacillus johnsonii
MTKIKDDYIVGLDIGTDSCGWVAMNSNNDILKLQGKTAIGSRLFEGGKSAAERRLFRTTHRRIKRRRWRLKLLEEFFDPYMAEVDPYFFARLKESGLSPLDKRKTVSSIVFPTSAEDKKFYDDYPTIYHLRYKLMTEDEKFDLREVYLAIHHIIKYRGNFLYNTSVKDFKASKIDVKSSIEKLNELYENLGLDLNVEFNISNTAEIEKVLKDKQIFKRDKVKKIAELFAIKTDNKEQSKRIKDISKQVANAVLGYKTRFDTIALKEISKDELSDWNFKLSDIDADSKFEALMGNLDENEQAILLTIKELFNEVTLNGIVEDGNTLSESMINKYNDHRDDLKLLKEVIENHIDRKKAKELALAYDLYVNNRHGQLLQAKKKLGKIKPRSKEDFYKVVNKNLDDSRASKEIKKKIELDSFMPKQRTNANGVIPYQLQQLELDKIIENQSKYYPFLKEINPVSSHLKEAPYKLDELIRFRVPYYVGPLISPNESTKDIQTKKNQNFAWMIRKEEGRITPWNFDQKVDRIESANKFIKRMTTKDTYLFGEDVLPANSLLYQKFTVLNELNNIRINGKRISVDLKQEIYENLFKKHTTVTVKKLENYLKENHNLVKVEIKGLADEKKFNSGLTTYNRFKNLNIFDNQIDDLKYRNDFEKIIEWSTIFEDKSIYKEKLRSIDWLNEKQINALSNIRLQGWGRLSKKLLAQLHDHNGQTIIEQLWDSQNNFMQIVTQADFKDAIAKANQNLLVATSVEDILNNAYTSPANKKAIRQVIKVVDDIVKAASGKVPKQIAIEFTRDADENPKRSQTRGSKLQKVYKDLSTELASKTIAEELNEAIKDKKLVQDKYYLYFMQLGRDAYTGEPINIDEIQKYDIDHILPQSFIKDDALDNRVLVSRAVNNGKSDNVPVKLFGNEMAANLGMTIRKMWEEWKNIGLISKTKYNNLLTDPDHINKYKSAGFIRRQLVETSQIIKLVSTILQSRYPNTEIITVKAKYNHYLREKFDLYKSREVNDYHHAIDAYLSAICGNLLYQNYPNLRPFFVYGQYKKFSSDPDKEKAIFNKTRKFSFISQLLKNKSENSKEIAKKLKRAYQFKYMLVSRETETRDQEMFKMTVYPRFSHDTVKAPRNLIPKKMGMSPDIYGGYTNNSDAYMVIVRIDKKKGTEYKILGIPTRELVNLKKAEKEDHYKSYLKEILTPRILYNKNGKRDKKITSFEIVKSKIPYKQVIQDGDKKFMLGSSTYVYNAKQLTLSTESMKAITNNFDKDSDENDALIKAYDEILDKVDKYLPLFDINKFREKLHSGREKFIKLSLEDKKDTILKVLEGLHDNAVMTKIPTIGLSTPLGFMQFPNGVILSENAKLIYQSPTGLFKKSVKISDL

SEQ ID NO: 178 - DNA, 4209 bp, synthetic construct; identical to SEQ ID NO: 123
  misc_feature 1..4209: note = source = /note="Description of Artificial Sequence: Synthetic polynucleotide"
  source 1..4209: mol_type = other DNA

SEQ ID NO: 179 - RNA, 178 nt, synthetic construct
  misc_feature 1..178: note = source = /note="Description of Artificial Sequence: Synthetic polynucleotide"
  source 1..178: mol_type = other RNA
nnnnnnnnnnnnnnnnnnnngttgtagctcccattctcgaaagagaaccgttgctacaataaggccgtctgaaaagatgtgccgcaacgctctgccccttaaagcttctgctttaaggggcatcgtttatttcggttaaaaatgccgtctgaaaccggtttttaggtttcagacggca

SEQ ID NO: 180 - protein, 1082 aa, Neisseria cinerea
MAAFKPNPMNYILGLDIGIASVGWAIVEIDEEENPIRLIDLGVRVFERAEVPKTGDSLAAARRLARSVRRLTRRRAHRLLRARRLLKREGVLQAADFDENGLIKSLPNTPWQLRAAALDRKLTPLEWSAVLLHLIKHRGYLSQRKNEGETADKELGALLKGVADNTHALQTGDFRTPAELALNKFEKESGHIRNQRGDYSHTFNRKDLQAELNLLFEKQKEFGNPHVSDGLKEGIETLLMTQRPALSGDAVQKMLGHCTFEPTEPKAAKNTYTAERFVWLTKLNNLRILEQGSERPLTDTERATLMDEPYRKSKLTYAQARKLLDLDDTAFFKGLRYGKDNAEASTLMEMKAYHAISRALEKEGLKDKKSPLNLSPELQDEIGTAFSLFKTDEDITGRLKDRVQPEILEALLKHISFDKFVQISLKALRRIVPLMEQGNRYDEACTEIYGDHYGKKNTEEKIYLPPIPADEIRNPVVLRALSQARKVINGVVRRYGSPARIHIETAREVGKSFKDRKEIEKRQEENRKDREKSAAKFREYFPNFVGEPKSKDILKLRLYEQQHGKCLYSGKEINLGRLNEKGYVEIDHALPFSRTWDDSFNNKVLALGSENQNKGNQTPYEYFNGKDNSREWQEFKARVETSRFPRSKKQRILLQKFDEDGFKERNLNDTRYINRFLCQFVADHMLLTGKGKRRVFASNGQITNLLRGFWGLRKVRAENDRHHALDAVVVACSTIAMQQKITRFVRYKEMNAFDGKTIDKETGEVLHQKAHFPQPWEFFAQEVMIRVFGKPDGKPEFEEADTPEKLRTLLAEKLSSRPEAVHKYVTPLFISRAPNRKMSGQGHMETVKSAKRLDEGISVLRVPLTQLKLKDLEKMVNREREPKLYEALKARLEAHKDDPAKAFAEPFYKYDKAGNRTQQVKAVRVEQVQKTGVWVHNHNGIADNATIVRVDVFEKGGKYYLVPIYSWQVAKGILPDRAVVQGKDEEDWTVMDDSFEFKFVLYANDLIKLTAKKNEFLGYFVSLNRATGAIDIRTHDTDSTKGKNGIFQSVGVKTALSFQKYQIDELGKEIRPCRLKKRPPVR

SEQ ID NO: 181 - DNA, 3330 bp, synthetic construct
  misc_feature 1..3330: note = source = /note="Description of Artificial Sequence: Synthetic polynucleotide"
  source 1..3330: mol_type = other DNA
accggtgccaccatgtacccatacgatgttccagattacgcttcgccgaagaaaaagcgcaaggtcgaagcgtccatggctgccttcaaacctaatcctatgaactacatcctgggcctggacattggaatcgcttctgtcgggtgggctatcgtggaaatcgacgaggaagagaaccctatcagactgattgatctgggagtcagagtgtttgaaagggcagaggtgccaaagaccggcgactccctggccgctgcacggagactggctcggtctgtcaggcgcctgacacgacggagagcacacaggctgctgcgagctaggcgcctgctgaagagagagggcgtgctgcaggccgctgacttcgatgaaaacggcctgatcaagagcctgcccaatactccttggcagctgagagcagccgctctggacaggaagctgaccccactggagtggtctgccgtgctgctgcacctgatcaagcatcgcggctacctgagtcagcgaaaaaatgaaggggagacagcagataaggagctgggagcactgctgaaaggagtggccgacaacactcatgctctgcagaccggcgattttaggacacccgctgagctggcactgaataagttcgaaaaagagagtggacacattcgaaaccagcggggcgactattcacataccttcaaccgcaaggatctgcaggccgagctgaatctgctgtttgaaaagcagaaagagttcgggaatccccacgtgtccgacgggctgaaagaaggaatcgagacactgctgatgactcagaggcctgcactgtctggcgatgccgtgcagaagatgctggggcattgcacctttgaaccaacagagcccaaggcagccaaaaacacctacacagccgagaggttcgtgtggctgacaaagctgaacaatctgcgcatcctggaacagggcagtgagcggcccctgactgacaccgaaagagccacactgatggatgagccttacaggaagtctaaactgacttatgcccaggctcgcaagctgctggacctggacgatactgccttctttaagggcctgaggtacgggaaagataatgcagaagccagcaccctgatggagatgaaggcctatcacgctatctcccgcgccctggaaaaagagggcctgaaggacaagaaatctcccctgaacctgagtcctgaactgcaggatgagattgggaccgcttttagcctgttcaagactgacgaggatatcaccggacgcctgaaagaccgagtgcagcccgaaattctggaggcactgctgaagcacatcagttttgataaattcgtgcagatttcactgaaggccctgcgacggatcgtccctctgatggagcagggcaatcggtacgacgaggcctgcaccgagatctacggagatcattatggcaagaaaaacacagaagagaaaatctatctgccccctattcctgccgacgagatccggaatccagtggtcctgagagctctgtcacaggcaagaaaagtgatcaacggagtggtcagaaggtacggcagccctgctaggatccacattgaaaccgcacgcgaagtgggaaagtcctttaaagaccgcaaggaaatcgagaagcgacaggaagagaatagaaaagatagggaaaagtctgctgcaaaattcagggagtactttccaaacttcgtgggcgaacccaagagtaaagacatcctgaagctgcgcctgtacgagcagcagcacgggaagtgtctgtatagcggaaaagaaattaacctgggccggctgaatgaaaagggctatgtggagatcgatcatgcactgcccttttccagaacatgggacgattctttcaacaataaggtcctggctctggggagcgagaaccagaacaagggaaatcagactccttacgaatatttcaacgggaaggacaatagccgagaatggcaggagtttaaagcccgcgtggagacaagccggttcccacgaagcaagaaacagcggattctgctgcagaagtttgacgaagatggattcaaagagagaaacctgaatgacacccggtacatcaacagatttctgtgccagttcgtggctgatcacatgctgctgaccggaaagggcaaacgccgagtctttgcaagcaacggccagatcacaaatctgctgaggggcttctgggggctgcggaaggtgagagccgagaatgaccgccaccatgcactggatgccgtggtcgtggcttgttccactattgcaatgcagcagaagatcaccaggtttgtgcgctataaagagatgaacgccttcgacggaaagacaattgataaagaaactggcgaggtgctgcaccagaaggcacattttcctcagccatgggagttcttcgcccaggaagtgatgatccgggtctttgggaagcctgacggaaaaccagagttcgaagaggccgataccccagaaaagctgcggacactgctggctgaaaaactgagctccagacccgaggcagtgcacaagtacgtcacccccctgttcattagcagggcccctaatcgcaaaatgtccgggcagggacatatggagactgtgaaatcagctaagcggctggacgaaggcatcagcgtgctgagagtcccactgacccagctgaagctgaaagatctggagaagatggtgaaccgggaaagagagcccaagctgtatgaagctctgaaagcaagactggaggcccacaaggacgatccagctaaagcatttgccgagcccttctacaaatatgacaaggccggcaatcggacacagcaggtgaaggctgtcagagtggagcaggtccagaaaactggggtctgggtgcacaaccataatggaattgccgacaacgctacaatcgtccgggtggatgtgttcgagaaaggcgggaagtactatctggtgcctatctactcctggcaggtcgccaagggaatcctgccagatagagctgtcgtgcagggcaaagacgaagaggattggactgtgatggacgattctttcgagtttaagttcgtcctgtacgcaaacgacctgatcaagctgacagccaagaaaaatgaatttctggggtatttcgtgtcactgaacagggcaactggagccatcgatattcgcacacatgacactgatagcaccaagggaaaaaacggcatctttcagtctgtgggcgtcaagaccgccctgagtttccagaaatatcagattgacgaactggggaaggagatccgaccctgtcggctgaagaaacgaccacccgtgcggtaagaattc

SEQ ID NO: 182 - RNA, 145 nt, synthetic construct
  misc_feature 1..145: note = source = /note="Description of Artificial Sequence: Synthetic polynucleotide"
  source 1..145: mol_type = other RNA
nnnnnnnnnnnnnnnnnnnngctgcggattgcgggaaatcgcttttcgcaagcaaattgaccccttgtgcgggctcggcatcccaaggtcagctgccggttattatcgaaaaggcccaccgcaagcagcgcgtgggccttttttt

SEQ ID NO: 183 - protein, 1037 aa, Parvibaculum lavamentivorans
MERIFGFDIGTTSIGFSVIDYSSTQSAGNIQRLGVRIFPEARDPDGTPLNQQRRQKRMMRRQLRRRRIRRKALNETLHEAGFLPAYGSADWPVVMADEPYELRRRGLEEGLSAYEFGRAIYHLAQHRHFKGRELEESDTPDPDVDDEKEAANERAATLKALKNEQTTLGAWLARRPPSDRKRGIHAHRNVVAEEFERLWEVQSKFHPALKSEEMRARISDTIFAQRPVFWRKNTLGECRFMPGEPLCPKGSWLSQQRRMLEKLNNLAIAGGNARPLDAEERDAILSKLQQQASMSWPGVRSALKALYKQRGEPGAEKSLKFNLELGGESKLLGNALEAKLADMFGPDWPAHPRKQEIRHAVHERLWAADYGETPDKKRVIILSEKDRKAHREAAANSFVADFGITGEQAAQLQALKLPTGWEPYSIPALNLFLAELEKGERFGALVNGPDWEGWRRTNFPHRNQPTGEILDKLPSPASKEERERISQLRNPTVVRTQNELRKVVNNLIGLYGKPDRIRIEVGRDVGKSKREREEIQSGIRRNEKQRKKATEDLIKNGIANPSRDDVEKWILWKEGQERCPYTGDQIGFNALFREGRYEVEHIWPRSRSFDNSPRNKTLCRKDVNIEKGNRMPFEAFGHDEDRWSAIQIRLQGMVSAKGGTGMSPGKVKRFLAKTMPEDFAARQLNDTRYAAKQILAQLKRLWPDMGPEAPVKVEAVTGQVTAQLRKLWTLNNILADDGEKTRADHRHHAIDALTVACTHPGMTNKLSRYWQLRDDPRAEKPALTPPWDTIRADAEKAVSEIVVSHRVRKKVSGPLHKETTYGDTGTDIKTKSGTYRQFVTRKKIESLSKGELDEIRDPRIKEIVAAHVAGRGGDPKKAFPPYPCVSPGGPEIRKVRLTSKQQLNLMAQTGNGYADLGSNHHIAIYRLPDGKADFEIVSLFDASRRLAQRNPIVQRTRADGASFVMSLAAGEAIMIPEGSKKGIWIVQGVWASGQVVLERDTDADHSTTTRPMPNPILKDDAKKVSIDPIGRVRPSND

SEQ ID NO: 184 - DNA, 3195 bp, synthetic construct
  misc_feature 1..3195: note = source = /note="Description of Artificial Sequence: Synthetic polynucleotide"
  source 1..3195: mol_type = other DNA
accggtgccaccatgtacccatacgatgttccagattacgcttcgccgaagaaaaagcgcaaggtcgaagcgtccatggagaggattttcggctttgacatcggcacaacaagtatcggattcagcgtgattgattacagtagcacccagtccgcaggcaacatccagaggctgggcgtgcgcattttccctgaggcaagggacccagatgggacccccctgaaccagcagcggagacagaaacgcatgatgaggcgccagctgcgacggagaaggattcgccgaaaggcactgaatgagacactgcacgaagccggctttctgccagcttacgggtctgcagattggcccgtggtcatggccgacgagccttatgaactgcggagaaggggactggaggaaggcctgagtgcttacgagttcggacgggcaatctatcatctggcccagcaccggcattttaaaggcagagaactggaggaatccgatacacccgaccctgatgtggacgatgagaaggaagccgctaacgagagagcagccactctgaaggccctgaaaaatgaacagaccacactgggagcatggctggcccgccgacccccttctgaccgcaagcgaggaatccacgcccataggaacgtggtcgctgaggagttcgagcgcctgtgggaagtgcagtccaagtttcaccccgctctgaaatctgaggaaatgcgggcaagaatcagtgatacaattttcgcccagaggcctgtgttttggcgcaagaacactctgggagagtgcagattcatgcctggcgaaccactgtgtcccaaggggtcctggctgtctcagcagcggagaatgctggagaaactgaacaatctggctatcgcaggcgggaatgctaggccactggatgcagaggaacgcgacgccattctgagtaagctgcagcagcaggccagcatgtcctggccaggcgtgcggtcagctctgaaggcactgtacaaacagagaggcgagcccggggctgaaaagagcctgaaattcaacctggagctgggaggcgaatccaagctgctgggaaatgccctggaggctaaactggcagatatgtttggccctgactggccagctcacccccgaaagcaggagatccggcacgcagtgcatgaacggctgtgggctgcagattacggcgagacacccgacaagaaaagagtcatcattctgtccgagaaggatcgaaaagctcatcgggaagccgctgcaaactctttcgtggcagactttggaattactggcgagcaggcagctcagctgcaggccctgaagctgccaaccggctgggaaccttatagcatcccagcactgaacctgttcctggccgagctggaaaagggggagaggtttggagccctggtgaatggacctgattgggaaggctggaggcgcacaaacttcccccaccgcaatcagcctactggggagatcctggacaagctgccaagtcccgcctcaaaagaggaaagggaacgcattagccagctgcgcaacccaaccgtggtccgaacacagaatgagctgagaaaggtggtcaacaatctgatcgggctgtatggaaaacccgatcgaatccggattgaagtgggccgggacgtcgggaagtccaaaagagaaagggaggaaatccagtctggcattcgacggaacgagaagcagagaaagaaagccactgaagatctgatcaaaaacggaattgctaatcctagccgggacgatgtggagaagtggatcctgtggaaagagggccaggaaagatgcccatacaccggcgaccagattggcttcaatgccctgtttagagaaggcagatatgaggtggaacacatctggcctcgctctcgaagttttgataacagcccaaggaataagacactgtgtcgcaaagacgtgaacatcgagaagggaaataggatgcctttcgaggcatttggccatgacgaagatcggtggagcgccatccagattagactgcagggcatggtgtcagccaaagggggaactgggatgagccccggaaaggtcaaacgcttcctggctaagaccatgcctgaggattttgcagcccggcagctgaacgacacaagatacgctgcaaagcagatcctggcccagctgaaaaggctgtggccagacatgggacctgaggctccagtgaaggtcgaagcagtgactggacaggtcaccgcccagctgcgcaaactgtggactctgaacaatattctggctgacgatggggagaaaaccagagcagatcacaggcaccatgccatcgacgctctgacagtggcctgcactcatcctggaatgaccaacaagctgagcaggtattggcagctgcgcgacgatccacgagcagagaagccagctctgactccaccctgggataccatccgcgccgacgctgagaaagccgtgtctgaaattgtggtcagtcaccgggtgagaaagaaagtcagcggcccactgcataaggagactacctacggcgatacagggactgacattaagaccaaatccggcacatatagacagttcgtgaccaggaagaaaatcgagtcactgagcaagggggagctggatgaaattcgcgacccccgaatcaaagaaattgtggcagctcacgtcgcaggacgaggaggcgaccccaagaaggccttccctccatacccctgtgtgtctcccggaggccctgagatccggaaggtcagactgaccagtaaacagcagctgaacctgatggcccagacagggaatggatacgctgacctgggctccaaccaccatatcgcaatctaccggctgcccgatgggaaggccgacttcgagattgtgtcactgtttgatgctagcagaaggctggcacagagaaatccaatcgtgcagaggacacgagcagacggagccagcttcgtcatgtccctggcagccggagaggccatcatgattcccgaaggctcaaagaaagggatctggattgtgcagggagtctgggcaagcggacaggtggtcctggagagggacaccgatgctgaccactctacaactacccgccctatgccaaaccccatcctgaaggacgatgccaagaaagtgagtatcgatcctattggccgagtccggccatcaaatgactaagaattc

SEQ ID NO: 185 - RNA, 103 nt, synthetic construct
  misc_feature 1..103: note = source = /note="Description of Artificial Sequence: Synthetic polynucleotide"
  source 1..103: mol_type = other RNA
nnnnnnnnnnnnnnnnnnnngttttagtactctggaaacagaatctactaaaacaaggcaaaatgccgtgtttatctcgtcaacttgttggcgagattttttt

SEQ ID NO: 186 - protein, 1053 aa, Staphylococcus aureus
MKRNYILGLDIGITSVGYGIIDYETRDVIDAGVRLFKEANVENNEGRRSKRGARRLKRRRRHRIQRVKKLLFDYNLLTDHSELSGINPYEARVKGLSQKLSEEEFSAALLHLAKRRGVHNVNEVEEDTGNELSTKEQISRNSKALEEKYVAELQLERLKKDGEVRGSINRFKTSDYVKEAKQLLKVQKAYHQLDQSFIDTYIDLLETRRTYYEGPGEGSPFGWKDIKEWYEMLMGHCTYFPEELRSVKYAYNADLYNALNDLNNLVITRDENEKLEYYEKFQIIENVFKQKKKPTLKQIAKEILVNEEDIKGYRVTSTGKPEFTNLKVYHDIKDITARKEIIENAELLDQIAKILTIYQSSEDIQEELTNLNSELTQEEIEQISNLKGYTGTHNLSLKAINLILDELWHTNDNQIAIFNRLKLVPKKVDLSQQKEIPTTLVDDFILSPVVKRSFIQSIKVINAIIKKYGLPNDIIIELAREKNSKDAQKMINEMQKRNRQTNERIEEIIRTTGKENAKYLIEKIKLHDMQEGKCLYSLEAIPLEDLLNNPFNYEVDHIIPRSVSFDNSFNNKVLVKQEENSKKGNRTPFQYLSSSDSKISYETFKKHILNLAKGKGRISKTKKEYLLEERDINRFSVQKDFINRNLVDTRYATRGLMNLLRSYFRVNNLDVKVKSINGGFTSFLRRKWKFKKERNKGYKHHAEDALIIANADFIFKEWKKLDKAKKVMENQMFEEKQAESMPEIETEQEYKEIFITPHQIKHIKDFKDYKYSHRVDKKPNRELINDTLYSTRKDDKGNTLIVNNLNGLYDKDNDKLKKLINKSPEKLLMYHHDPQTYQKLKLIMEQYGDEKNPLYKYYEETGNYLTKYSKKDNGPVIKKIKYYGNKLNAHLDITDDYPNSRNKVVKLSLKPYRFDVYLDNGVYKFVTVKNLDVIKKENYYEVNSKCYEEAKKLKKISNQAEFIASFYNNDLIKINGELYRVIGVNNDLLNRIEVNMIDITYREYLENMNDKRPPRIIKTIASKTQSIKKYSTDILGNLYEVKSKKHPQIIKKG

SEQ ID NO: 187 - DNA, 3243 bp, synthetic construct; identical to SEQ ID NO: 85
  misc_feature 1..3243: note = source = /note="Description of Artificial Sequence: Synthetic polynucleotide"
  source 1..3243: mol_type = other DNA

SEQ ID NO: 188 - RNA, 114 nt, synthetic construct
  misc_feature 1..114: note = source = /note="Description of Artificial Sequence: Synthetic polynucleotide"
  source 1..114: mol_type = other RNA
nnnnnnnnnnnnnnnnnnnngttttagcactgtacaagaaattgtcgtgctaaaataaggcgctgttaatgcagctgccgcatccgccagagcatttatgctctggcttttttt

SEQ ID NO: 189 - protein, 1269 aa, Mycoplasma gallisepticum
MNNSIKSKPEVTIGLDLGVGSVGWAIVDNETNIIHHLGSRLFSQAKTAEDRRSFRGVRRLIRRRKYKLKRFVNLIWKYNSYFGFKNKEDILNNYQEQQKLHNTVLNLKSEALNAKIDPKALSWILHDYLKNRGHFYEDNRDFNVYPTKELAKYFDKYGYYKGIIDSKEDNDNKLEEELTKYKFSNKHWLEEVKKVLSNQTGLPEKFKEEYESLFSYVRNYSEGPGSINSVSPYGIYHLDEKEGKVVQKYNNIWDKTIGKCNIFPDEYRAPKNSPIAMIFNEINELSTIRSYSIYLTGWFINQEFKKAYLNKLLDLLIKTNGEKPIDARQFKKLREETIAESIGKETLKDVENEEKLEKEDHKWKLKGLKLNTNGKIQYNDLSSLAKFVHKLKQHLKLDFLLEDQYATLDKINFLQSLFVYLGKHLRYSNRVDSANLKEFSDSNKLFERILQKQKDGLFKLFEQTDKDDEKILAQTHSLSTKAMLLAITRMTNLDNDEDNQKNNDKGWNFEAIKNFDQKFIDITKKNNNLSLKQNKRYLDDRFINDAILSPGVKRILREATKVFNAILKQFSEEYDVTKVVIELARELSEEKELENTKNYKKLIKKNGDKISEGLKALGISEDEIKDILKSPTKSYKFLLWLQQDHIDPYSLKEIAFDDIFTKTEKFEIDHIIPYSISFDDSSSNKLLVLAESNQAKSNQTPYEFISSGNAGIKWEDYEAYCRKFKDGDSSLLDSTQRSKKFAKMMKTDTSSKYDIGFLARNLNDTRYATIVFRDALEDYANNHLVEDKPMFKVVCINGSVTSFLRKNFDDSSYAKKDRDKNIHHAVDASIISIFSNETKTLFNQLTQFADYKLFKNTDGSWKKIDPKTGVVTEVTDENWKQIRVRNQVSEIAKVIEKYIQDSNIERKARYSRKIENKTNISLFNDTVYSAKKVGYEDQIKRKNLKTLDIHESAKENKNSKVKRQFVYRKLVNVSLLNNDKLADLFAEKEDILMYRANPWVINLAEQIFNEYTENKKIKSQNVFEKYMLDLTKEFPEKFSEFLVKSMLRNKTAIIYDDKKNIVHRIKRLKMLSSELKENKLSNVIIRSKNQSGTKLSYQDTINSLALMIMRSIDPTAKKQYIRVPLNTLNLHLGDHDFDLHNMDAYLKKPKFVKYLKANEIGDEYKPWRVLTSGTLLIHKKDKKLMYISSFQNLNDVIEIKNLIETEYKENDDSDSKKKKKANRFLMTLSTILNDYILLDAKDNFDILGLSKNRIDEILNSKLGLDKIVK

SEQ ID NO: 190 - DNA, 3891 bp, synthetic construct; identical to SEQ ID NO: 136
  misc_feature 1..3891: note = source = /note="Description of Artificial Sequence: Synthetic polynucleotide"
  source 1..3891: mol_type = other DNA

SEQ ID NO: 191 - RNA, 137 nt, synthetic construct
  misc_feature 1..137: note = source = /note="Description of Artificial Sequence: Synthetic polynucleotide"
  source 1..137: mol_type = other RNA
nnnnnnnnnnnnnnnnnnnngttttagtctctgaaaagagactaaaataagtggtttttggtcatccacgcagggttacaatccctttaaaaccattaaaattcaaataaactaggttgtatcaacttagttttttt

SEQ ID NO: 192 - protein, 1003 aa, Campylobacter lari
MRILGFDIGINSIGWAFVENDELKDCGVRIFTKAENPKNKESLALPRRNARSSRRRLKRRKARLIAIKRILAKELKLNYKDYVAADGELPKAYEGSLASVYELRYKALTQNLETKDLARVILHIAKHRGYMNKNEKKSNDAKKGKILSALKNNALKLENYQSVGEYFYKEFFQKYKKNTKNFIKIRNTKDNYNNCVLSSDLEKELKLILEKQKEFGYNYSEDFINEILKVAFFQRPLKDFSHLVGACTFFEEEKRACKNSYSAWEFVALTKIINEIKSLEKISGEIVPTQTINEVLNLILDKGSITYKKFRSCINLHESISFKSLKYDKENAENAKLIDFRKLVEFKKALGVHSLSRQELDQISTHITLIKDNVKLKTVLEKYNLSNEQINNLLEIEFNDYINLSFKALGMILPLMREGKRYDEACEIANLKPKTVDEKKDFLPAFCDSIFAHELSNPVVNRAISEYRKVLNALLKKYGKVHKIHLELARDVGLSKKAREKIEKEQKENQAVNAWALKECENIGLKASAKNILKLKLWKEQKEICIYSGNKISIEHLKDEKALEVDHIYPYSRSFDDSFINKVLVFTKENQEKLNKTPFEAFGKNIEKWSKIQTLAQNLPYKKKNKILDENFKDKQQEDFISRNLNDTRYIATLIAKYTKEYLNFLLLSENENANLKSGEKGSKIHVQTISGMLTSVLRHTWGFDKKDRNNHLHHALDAIIVAYSTNSIIKAFSDFRKNQELLKARFYAKELTSDNYKHQVKFFEPFKSFREKILSKIDEIFVSKPPRKRARRALHKDTFHSENKIIDKCSYNSKEGLQIALSCGRVRKIGTKYVENDTIVRVDIFKKQNKFYAIPIYAMDFALGILPNKIVITGKDKNNNPKQWQTIDESYEFCFSLYKNDLILLQKKNMQEPEFAYYNDFSISTSSICVEKHDNKFENLTSNQKLLFSNAKEGSVKVESLGIQNLKVFEKYIITPLGDKIKADFQPRENISLKTSKKYGLR

SEQ ID NO: 193 - DNA, 3093 bp, synthetic construct; identical to SEQ ID NO: 137
  misc_feature 1..3093: note = source = /note="Description of Artificial Sequence: Synthetic polynucleotide"
  source 1..3093: mol_type = other DNA

SEQ ID NO: 194 - RNA, 103 nt, synthetic construct
  misc_feature 1..103: note = source = /note="Description of Artificial Sequence: Synthetic polynucleotide"
  source 1..103: mol_type = other RNA
nnnnnnnnnnnnnnnnnnnngttttagagctagaaatagcaagttaaaataaggctagtccgttatcaacttgaaaaagtggcaccgagtcggtgcttttttt

SEQ ID NO: 195 - protein, 1368 aa, Streptococcus pyogenes [sequence omitted]

SEQ ID NO: 196 - DNA, 4218 bp, synthetic construct
  misc_feature 1..4218: note = source = /note="Description of Artificial Sequence: Synthetic polynucleotide"
  source 1..4218: mol_type = other DNA
accggtgccaccatgtacccatacgatgttccagattacgcttcgccgaagaaaaagcgcaaggtcgaagcgtccgacaagaagtacagcatcggcctggacatcggcaccaactctgtgggctgggccgtgatcaccgacgagtacaaggtgcccagcaagaaattcaaggtgctgggcaacaccgaccggcacagcatcaagaagaacctgatcggagccctgctgttcgacagcggcgaaacagccgaggccacccggctgaagagaaccgccagaagaagatacaccagacggaagaaccggatctgctatctgcaagagatcttcagcaacgagatggccaaggtggacgacagcttcttccacagactggaagagtccttcctggtggaagaggataagaagcacgagcggcaccccatcttcggcaacatcgtggacgaggtggcctaccacgagaagtaccccaccatctaccacctgagaaagaaactggtggacagcaccgacaaggccgacctgcggctgatctatctggccctggcccacatgatcaagttccggggccacttcctgatcgagggcgacctgaaccccgacaacagcgacgtggacaagctgttcatccagctggtgcagacctacaaccagctgttcgaggaaaaccccatcaacgccagcggcgtggacgccaaggccatcctgtctgccagactgagcaagagcagacggctggaaaatctgatcgcccagctgcccggcgagaagaagaatggcctgttcggcaacctgattgccctgagcctgggcctgacccccaacttcaagagcaacttcgacctggccgaggatgccaaactgcagctgagcaaggacacctacgacgacgacctggacaacctgctggcccagatcggcgaccagtacgccgacctgtttctggccgccaagaacctgtccgacgccatcctgctgagcgacatcctgagagtgaacaccgagatcaccaaggcccccctgagcgcctctatgatcaagagatacgacgagcaccaccaggacctgaccctgctgaaagctctcgtgcggcagcagctgcctgagaagtacaaagagattttcttcgaccagagcaagaacggctacgccggctacattgacggcggagccagccaggaagagttctacaagttcatcaagcccatcctggaaaagatggacggcaccgaggaactgctcgtgaagctgaacagagaggacctgctgcggaagcagcggaccttcgacaacggcagcatcccccaccagatccacctgggagagctgcacgccattctgcggcggcaggaagatttttacccattcctgaaggacaaccgggaaaagatcgagaagatcctgaccttccgcatcccctactacgtgggccctctggccaggggaaacagcagattcgcctggatgaccagaaagagcgaggaaaccatcaccccctggaacttcgaggaagtggtggacaagggcgcttccgcccagagcttcatcgagcggatgaccaacttcgataagaacctgcccaacgagaaggtgctgcccaagcacagcctgctgtacgagtacttcaccgtgtataacgagctgaccaaagtgaaatacgtgaccgagggaatgagaaagcccgccttcctgagcggcgagcagaaaaaggccatcgtggacctgctgttcaagaccaaccggaaagtgaccgtgaagcagctgaaagaggactacttcaagaaaatcgagtgcttcgactccgtggaaatctccggcgtggaagatcggttcaacgcctccctgggcacataccacgatctgctgaaaattatcaaggacaaggacttcctggacaatgaggaaaacgaggacattctggaagatatcgtgctgaccctgacactgtttgaggacagagagatgatcgaggaacggctgaaaacctatgcccacctgttcgacgacaaagtgatgaagcagctgaagcggcggagatacaccggctggggcaggctgagccggaagctgatcaacggcatccgggacaagcagtccggcaagacaatcctggatttcctgaagtccgacggcttcgccaacagaaacttcatgcagctgatccacgacgacagcctgacctttaaagaggacatccagaaagcccaggtgtccggccagggcgatagcctgcacgagcacattgccaatctggccggcagccccgccattaagaagggcatcctgcagacagtgaaggtggtggacgagctcgtgaaagtgatgggccggcacaagcccgagaacatcgtgatcgaaatggccagagagaaccagaccacccagaagggacagaagaacagccgcgagagaatgaagcggatcgaagagggcatcaaagagctgggcagccagatcctgaaagaacaccccgtggaaaacacccagctgcagaacgagaagctgtacctgtactacctgcagaatgggcgggatatgtacgtggaccaggaactggacatcaaccggctgtccgactacgatgtggaccatatcgtgcctcagagctttctgaaggacgactccatcgacaacaaggtgctgaccagaagcgacaagaaccggggcaagagcgacaacgtgccctccgaagaggtcgtgaagaagatgaagaactactggcggcagctgctgaacgccaagctgattacccagagaaagttcgacaatctgaccaaggccgagagaggcggcctgagcgaactggataaggccggcttcatcaagagacagctggtggaaacccggcagatcacaaagcacgtggcacagatcctggactcccggatgaacactaagtacgacgagaatgacaagctgatccgggaagtgaaagtgatcaccctgaagtccaagctggtgtccgatttccggaaggatttccagttttacaaagtgcgcgagatcaacaactaccaccacgcccacgacgcctacctgaacgccgtcgtgggaaccgccctgatcaaaaagtaccctaagctggaaagcgagttcgtgtacggcgactacaaggtgtacgacgtgcggaagatgatcgccaagagcgagcaggaaatcggcaaggctaccgccaagtacttcttctacagcaacatcatgaactttttcaagaccgagattaccctggccaacggcgagatccggaagcggcctctgatcgagacaaacggcgaaaccggggagatcgtgtgggataagggccgggattttgccaccgtgcggaaagtgctgagcatgccccaagtgaatatcgtgaaaaagaccgaggtgcagacaggcggcttcagcaaagagtctatcctgcccaagaggaacagcgataagctgatcgccagaaagaaggactgggaccctaagaagtacggcggcttcgacagccccaccgtggcctattctgtgctggtggtggccaaagtggaaaagggcaagtccaagaaactgaagagtgtgaaagagctgctggggatcaccatcatggaaagaagcagcttcgagaagaatcccatcgactttctggaagccaagggctacaaagaagtgaaaaaggacctgatcatcaagctgcctaagtactccctgttcgagctggaaaacggccggaagagaatgctggcctctgccggcgaactgcagaagggaaacgaactggccctgccctccaaatatgtgaacttcctgtacctggccagccactatgagaagctgaagggctcccccgaggataatgagcagaaacagctgtttgtggaacagcacaagcactacctggacgagatcatcgagcagatcagcgagttctccaagagagtgatcctggccgacgctaatctggacaaagtgctgtccgcctacaacaagcaccgggataagcccatcagagagcaggccgagaatatcatccacctgtttaccctgaccaatctgggagcccctgccgccttcaagtactttgacaccaccatcgaccggaagaggtacaccagcaccaaagaggtgctggacgccaccctgatccaccagagcatcaccggcctgtacgagacacggatcgacctgtctcagctgggaggcgacagccccaagaagaagagaaaggtggaggccagctaagaattc

SEQ ID NO: 197 - RNA, 116 nt, synthetic construct
  misc_feature 1..116: note = source = /note="Description of Artificial Sequence: Synthetic polynucleotide"
  source 1..116: mol_type = other RNA
nnnnnnnnnnnnnnnnnnnngtttttgtactctcaagatttagaaacttgcagaagctacaaagataaggcttcatgccgaaatcaacaccctgtcattttatggcagggtgtttt

SEQ ID NO: 198 - protein, 1120 aa, Streptococcus thermophilus
MSDLVLGLDIGIGSVGVGILNKVTGEIIHKNSRIFPAAQAENNLVRRTNRQGRRLARRKKHRRVRLNRLFEESGLITDFTKISINLNPYQLRVKGLTDELSNEELFIALKNMVKHRGISYLDDASDDGNSSVGDYAQIVKENSKQLETKTPGQIQLERYQTYGQLRGDFTVEKDGKKHRLINVFPTSAYRSEALRILQTQQEFNPQITDEFINRYLEILTGKRKYYHGPGNEKSRTDYGRYRTSGETLDNIFGILIGKCTFYPDEFRAAKASYTAQEFNLLNDLNNLTVPTETKKLSKEQKNQIINYVKNEKAMGPAKLFKYIAKLLSCDVADIKGYRIDKSGKAEIHTFEAYRKMKTLETLDIEQMDRETLDKLAYVLTLNTEREGIQEALEHEFADGSFSQKQVDELVQFRKANSSIFGKGWHNFSVKLMMELIPELYETSEEQMTILTRLGKQKTTSSSNKTKYIDEKLLTEEIYNPVVAKSVRQAIKIVNAAIKEYGDFDNIVIEMARETNEDDEKKAIQKIQKANKDEKDAAMLKAANQYNGKAELPHSVFHGHKQLATKIRLWHQQGERCLYTGKTISIHDLINNSNQFEVDHILPLSITFDDSLANKVLVYATANQEKGQRTPYQALDSMDDAWSFRELKAFVRESKTLSNKKKEYLLTEEDISKFDVRKKFIERNLVDTRYASRVVLNALQEHFRAHKIDTKVSVVRGQFTSQLRRHWGIEKTRDTYHHHAVDALIIAASSQLNLWKKQKNTLVSYSEDQLLDIETGELISDDEYKESVFKAPYQHFVDTLKSKEFEDSILFSYQVDSKFNRKISDATIYATRQAKVGKDKADETYVLGKIKDIYTQDGYDAFMKIYKKDKSKFLMYRHDPQTFEKVIEPILENYPNKQINEKGKEVPCNPFLKYKEEHGYIRKYSKKGNGPEIKSLKYYDSKLGNHIDITPKDSNNKVVLQSVSPWRADVYFNKTTGKYEILGLKYADLQFEKGTGTYKISQEKYNDIKKKEGVDSDSEFKFTLYKNDLLLVKDTETKEQQLFRFLSRTMPKQKHYVELKPYDKQKFEGGEALIKVLGNVANSGQCKKGLGKSNISIYKVRTDVLGNQHIIKNEGDKPKLM

SEQ ID NO: 199 - DNA, 3477 bp, synthetic construct
  misc_feature 1..3477: note = source = /note="Description of Artificial Sequence: Synthetic polynucleotide"
  source 1..3477: mol_type = other DNA
accggtgccaccatgtacccatacgatgttccagattacgcttcgccgaagaaaaagcgcaaggtcgaagcgtcctccgacctggtacttggactggatattggtatcggttcggtgggagtcggaatcctcaacaaggtcacgggggagatcattcacaagaactcgcggatcttccccgcagctcaggctgagaacaacttggtgcggagaacgaataggcagggcaggcgactggcgaggaggaagaaacacaggagagtccgattgaaccggctgttcgaggagtccggtttgatcaccgactttacgaaaatctcgattaaccttaatccctatcagcttcgggtgaaaggcctgacagacgaactttcgaatgaggaacttttcatcgcgctgaaaaacatggtcaagcacagagggatttcctacctcgatgacgcctcggatgacggaaattcctcagtaggagattatgcacagatcgtgaaagagaactcaaagcaactggaaacaaagacaccggggcagatccaacttgaaagataccagacatacggacagctcagaggagattttacggtggagaaggacggtaaaaagcacagactcattaacgtatttcccacgtcggcgtacagatccgaagcgctccgcatccttcagactcaacaggagttcaacccgcaaattactgatgagttcatcaaccgctatttggaaatcttgaccggaaagcgcaagtattatcatgggccgggtaatgagaaatccagaacagattacggccgatacagaacttcgggggaaaccttggataacatctttggtattttgattggaaagtgcaccttttacccggacgagtttcgagcggccaaggcgtcatacacagcacaagagtttaatctcttgaatgatttgaacaacttgacggtccccacggagacaaagaagctctccaaagagcaaaagaaccaaatcatcaactacgtcaagaacgagaaggctatggggccagcgaagctgttcaagtatatcgctaaacttctcagctgtgatgtggcggacatcaaagggtaccgaatcgacaagtcgggaaaagcggaaattcacacgtttgaagcatatcgaaagatgaaaacgttggaaacactggacattgagcagatggaccgggaaacgctcgacaaactggcatacgtgctcacgttgaatactgaacgagagggaatccaagaggcccttgaacatgagttcgccgatggatcgttcagccagaagcaggtcgacgaacttgtgcaattccgcaaggcgaatagctccatcttcgggaagggatggcacaacttttcggtcaaactcatgatggagttgatcccagaactttatgagacttcggaggagcaaatgacgatcttgacgcgcttggggaaacagaaaacgacaagctcatcgaacaaaactaagtacattgatgagaaattgctgacggaagaaatctataatccggtagtagcgaaatcggtaagacaagcgatcaaaatcgtgaacgcggcgatcaaggaatatggtgactttgataacatcgtaattgaaatggctagagagacgaacgaagatgacgagaaaaaggcaatccagaagatccagaaggccaacaaggatgaaaaagatgcagcgatgcttaaagcggccaaccaatacaatggaaaggcggagctgccccattcagtgtttcacggtcataaacagttggcgaccaagatccgactctggcatcagcagggtgagcggtgtctctacaccggaaagactatctccatccatgacttgattaacaattcgaaccagtttgaagtggatcatattctgcccctgtcaatcacctttgacgactcgcttgcgaacaaggtgctcgtgtacgcaacggcaaatcaggagaaaggccagcggactccgtatcaggcgctcgactcaatggacgatgcgtggtcattccgggagctgaaggcgttcgtacgcgagagcaagacactgagcaacaaaaagaaagagtatctgctgacagaggaggacatctcgaaattcgatgtcaggaagaagttcatcgagcggaatcttgtcgacactcgctacgcttccagagtagtactgaacgcgctccaggaacactttagagcgcacaaaattgacacgaaggtgtcagtggtgagagggcagttcacatcccaactccgccgacattggggcatcgaaaagacgcgggacacatatcaccatcatgcggtggacgcgctgattattgccgcttcgtcccagttgaatctctggaaaaagcagaagaacacgctggtgtcgtattcggaggatcagcttttggacatcgaaaccggggagctgatttccgacgatgaatacaaagaatcggtgtttaaggcaccatatcagcatttcgtggacacgctgaagagcaaagagtttgaggacagcatcctcttttcgtaccaagtggactcgaagtttaatcgcaagatttcagacgccacaatctacgcgacgaggcaggcgaaggtgggcaaagataaagcagatgaaacctacgtccttggtaaaatcaaggacatctacactcaggacgggtacgatgcgttcatgaaaatctacaagaaggataagtcgaagtttctcatgtaccgccacgatccacagactttcgaaaaagtcattgagcctattttggagaactaccctaacaagcaaatcaacgagaaagggaaagaagtcccgtgcaacccctttctgaagtacaaggaagagcacggttatatccgcaaatactcgaagaaaggaaatgggcctgagattaagtcgcttaagtattacgactcaaagttgggtaaccacatcgacattaccccgaaagactccaacaacaaagtcgtgttgcagtccgtctcgccctggcgagcagatgtgtattttaataagacgaccggcaaatatgagatccttggactcaaatacgcagaccttcaattcgaaaaggggacgggcacttataagatttcacaagagaagtacaacgacatcaagaaaaaggaaggggtcgattcagattcggagttcaaattcaccctctacaaaaacgacctcctgcttgtgaaggacacagaaacgaaggagcagcagctctttcggttcctctcacgcacgatgcccaaacaaaaacattacgtcgaacttaaaccttacgataagcaaaagtttgaagggggagaggcactgatcaaagtattgggtaacgtagccaatagcggacagtgtaagaaagggctgggaaagtccaatatctcgatctataaagtacgaacagatgtattgggaaaccagcatatcatcaaaaatgagggggataaacccaaactcgatttcagccccaagaagaagagaaaggtggaggccagctaagaattc

SEQ ID NO: 200 - DNA, 27 bp, synthetic construct
  misc_feature 1..27: note = source = /note="Description of Artificial Sequence: Synthetic oligonucleotide"
  source 1..27: mol_type = other DNA
gcccgggtggaactggtagccatgaat

SEQ ID NO: 201 - DNA, 26 bp, synthetic construct
  misc_feature 1..26: note = source = /note="Description of Artificial Sequence: Synthetic oligonucleotide"
  source 1..26: mol_type = other DNA
gttgaagatgaagcccagagcggagt

SEQ ID NO: 202 - DNA, 27 bp, synthetic construct
  misc_feature 1..27: note = source = /note="Description of Artificial Sequence: Synthetic oligonucleotide"
  source 1..27: mol_type = other DNA
gcttccgacgaggtggccatcaaggat

SEQ ID NO: 203 - DNA, 27 bp, synthetic construct
  misc_feature 1..27: note = source = /note="Description of Artificial Sequence: Synthetic oligonucleotide"
  source 1..27: mol_type = other DNA
gcaccatctctccgtggtaccccgggt

SEQ ID NO: 204 - DNA, 26 bp, synthetic construct
  misc_feature 1..26: note = source = /note="Description of Artificial Sequence: Synthetic oligonucleotide"
  source 1..26: mol_type = other DNA
ggtggaactggtagccatgaatgaga

SEQ ID NO: 205 - DNA, 27 bp, synthetic construct
  misc_feature 1..27: note = source = /note="Description of Artificial Sequence: Synthetic oligonucleotide"
  source 1..27: mol_type = other DNA
gccatgaatgagaccgacccaaagagc

SEQ ID NO: 206 - DNA, 27 bp, synthetic construct
  misc_feature 1..27: note = source = /note="Description of Artificial Sequence: Synthetic oligonucleotide"
  source 1..27: mol_type = other DNA
gcatcctcgtgggcacttccgacgagg

SEQ ID NO: 207 - DNA, 27 bp, synthetic construct
  misc_feature 1..27: note = source = /note="Description of Artificial Sequence: Synthetic oligonucleotide"
  source 1..27: mol_type = other DNA
gcagagcggagtgctgttctcccaagt

SEQ ID NO: 208 - DNA, 26 bp, synthetic construct
  misc_feature 1..26: note = source = /note="Description of Artificial Sequence: Synthetic oligonucleotide"
  source 1..26: mol_type = other DNA
ggtcggtctcattcatggctaccagt

SEQ ID NO: 209 - DNA, 26 bp, synthetic construct
  misc_feature 1..26: note = source = /note="Description of Artificial Sequence: Synthetic oligonucleotide"
  source 1..26: mol_type = other DNA
gcaataaaaggtgctattgctatagt

SEQ ID NO: 210 - DNA, 26 bp, synthetic construct
  misc_feature 1..26: note = source = /note="Description of Artificial Sequence: Synthetic oligonucleotide"
  source 1..26: mol_type = other DNA
gtactcaaccaagtcattctgagaat

SEQ ID NO: 211 - DNA, 26 bp, synthetic construct
  misc_feature 1..26: note = source = /note="Description of Artificial Sequence: Synthetic oligonucleotide"
  source 1..26: mol_type = other DNA
nnnnnnngtactcaaccaagtcattc

SEQ ID NO: 212 - protein, 1121 aa, Streptococcus thermophilus
MSDLVLGLDIGIGSVGVGILNKVTGEIIHKNSRIFPAAQAENNLVRRTNRQGRRLARRKKHRRVRLNRLFEESGLITDFTKISINLNPYQLRVKGLTDELSNEELFIALKNMVKHRGISYLDDASDDGNSSVGDYAQIVKENSKQLETKTPGQIQLERYQTYGQLRGDFTVEKDGKKHRLINVFPTSAYRSEALRILQTQQEFNPQITDEFINRYLEILTGKRKYYHGPGNEKSRTDYGRYRTSGETLDNIFGILIGKCTFYPDEFRAAKASYTAQEFNLLNDLNNLTVPTETKKLSKEQKNQIINYVKNEKAMGPAKLFKYIAKLLSCDVADIKGYRIDKSGKAEIHTFEAYRKMKTLETLDIEQMDRETLDKLAYVLTLNTEREGIQEALEHEFADGSFSQKQVDELVQFRKANSSIFGKGWHNFSVKLMMELIPELYETSEEQMTILTRLGKQKTTSSSNKTKYIDEKLLTEEIYNPVVAKSVRQAIKIVNAAIKEYGDFDNIVIEMARETNEDDEKKAIQKIQKANKDEKDAAMLKAANQYNGKAELPHSVFHGHKQLATKIRLWHQQGERCLYTGKTISIHDLINNSNQFEVDHILPLSITFDDSLANKVLVYATANQEKGQRTPYQALDSMDDAWSFRELKAFVRESKTLSNKKKEYLLTEEDISKFDVRKKFIERNLVDTRYASRVVLNALQEHFRAHKIDTKVSVVRGQFTSQLRRHWGIEKTRDTYHHHAVDALIIAASSQLNLWKKQKNTLVSYSEDQLLDIETGELISDDEYKESVFKAPYQHFVDTLKSKEFEDSILFSYQVDSKFNRKISDATIYATRQAKVGKDKADETYVLGKIKDIYTQDGYDAFMKIYKKDKSKFLMYRHDPQTFEKVIEPILENYPNKQINEKGKEVPCNPFLKYKEEHGYIRKYSKKGNGPEIKSLKYYDSKLGNHIDITPKDSNNKVVLQSVSPWRADVYFNKTTGKYEILGLKYADLQFEKGTGTYKISQEKYNDIKKKEGVDSDSEFKFTLYKNDLLLVKDTETKEQQLFRFLSRTMPKQKHYVELKPYDKQKFEGGEALIKVLGNVANSGQCKKGLGKSNISIYKVRTDVLGNQHIIKNEGDKPKLDF

SEQ ID NO: 213 - DNA, 20 bp, unidentified
  source 1..20: mol_type = unassigned DNA
aaaagggaataagggcgaca

SEQ ID NO: 214 - DNA, 27 bp, Sutterella wadsworthensis
  source 1..27: mol_type = unassigned DNA
nggnnnncattctgagaatagtgtatg

SEQ ID NO: 215 - DNA, 20 bp, Sutterella wadsworthensis
  source 1..20: mol_type = unassigned DNA
gcgaccgagttgctcttgcc

SEQ ID NO: 216 - DNA, 27 bp, Legionella pneumophila
  source 1..27: mol_type = unassigned DNA
nggnnnncattctgagaatagtgtatg

SEQ ID NO: 217 - DNA, 20 bp, Legionella pneumophila
  source 1..20: mol_type = unassigned DNA
gcgaccgagttgctcttgcc

SEQ ID NO: 218 - DNA, 27 bp, Filifactor alocis
  source 1..27: mol_type = unassigned DNA
nnnaagcttgagtactcaccagtcaca

SEQ ID NO: 219 - DNA, 20 bp, Filifactor alocis
  source 1..20: mol_type = unassigned DNA
ctcttcctttttcaatatta

SEQ ID NO: 220 - DNA, 27 bp, Lactobacillus johnsonii
  source 1..27: mol_type = unassigned DNA
nnaaanntaaatgcttcaataatattg

SEQ ID NO: 221 - DNA, 20 bp, Lactobacillus johnsonii
  source 1..20: mol_type = unassigned DNA
aaagggaataagggcgacac

SEQ ID NO: 222 - DNA, 27 bp, Parvibaculum lavamentivorans
  source 1..27: mol_type = unassigned DNA
nnncatnaaaggaagagtatgagtatt

SEQ ID NO: 223 - DNA, 20 bp, Staphylococcus aureus
  source 1..20: mol_type = unassigned DNA
ctattctcagaatgacttgg

SEQ ID NO: 224 - DNA, 27 bp, Mycoplasma gallisepticum
  source 1..27: mol_type = unassigned DNA
nnganggagtcacagaaaagcatctta

SEQ ID NO: 225 - DNA, 20 bp, Mycoplasma gallisepticum
  source 1..20: mol_type = unassigned DNA
gtttctgggtgagcaaaaac

SEQ ID NO: 226 - DNA, 27 bp, Campylobacter lari
  source 1..27: mol_type = unassigned DNA
nngggnagaaggcaaaatgccgcaaaa

SEQ ID NO: 227 - DNA, 20 bp, Campylobacter lari
  source 1..20: mol_type = unassigned DNA
ggtattatcccgtattgacg

SEQ ID NO: 228 - DNA, 20 bp, unidentified
  misc_feature 1..20: note = source = /note="Description of Unknown: SpCas9 oligonucleotide"
  source 1..20: mol_type = unassigned DNA
gggactcaaccaagtcattc